European Patent Application EP 4 748 224 A2, published May 27, 2026. Title: Optimized plant CRISPR/Cpf1 systems. Applicant: KWS SAAT SE & Co. KGaA. Application EP. The sequence listing filed with the application follows.

SEQUENCE LISTING (158 sequences)

SEQ ID NO: 1 - DNA, 1413 bp, Brachypodium distachyon
  source 1..1413: mol_type = genomic DNA
ggagaagaactcgagagggaattgcagatcatgaggcagatggctatttttgtgtcacatatgcgcaaaaagagaggctatatttgtgtccctaggttcttcgttgtattgcagtttccatatcaatctgacttggtcgcatgagaaattgatggttaaataatttgaatctctcatgtagtatcaactattagatattattttcaccaaatatatttccatcggagaagaagaggctacagaggaagcagaagagaggggtgggagaatttttacacttttgtacacccacttaaacagcaaaatccgtatgaaaacaggcccaccaaaacaatgccacgataacaatccgtagaaacaaaagcttcatttaacagcggcgcaacaaagcacgcttatccatggtagttgtagtccgtatgcgatccaaagatcacgattcacgcgtgacggacggacgacgcgtgccacaccacaactaacggcatccatggtagttgtagtccgtatgcgatccaaagatcacgattcacgcgtgacggacggacgacgcgcgccacaccacaactaacagcgtgagccagcgtccaaactccggatggcaacggggacgaaacccgtcgggtagtcactgcccaaacccgtccccgcaaccttcatcccaaacccgtccccgtttccggtcgcgggtttcagttttctaccagacccgtccccatcgggtttttcatccccgtcgggaaatccgaacccgccagcatttcagcaccaagccaaagttgcagcagcaacatgaataaaaaacaacccgtttcaacaccaagataaaacaaaacattataatttagacaacatttcacacgtataacaataacatatagttctcacatataacaacaccatttcacacataaaacaacaccatttgggataaaaatatgggctatatcaggccatttttatgggccatattgagttttcgtgggtttcacaggtaccggatttgtagaatgctgaaccgggtttgaaccgtaaaatccgcgggtattgaatttgacccaatcccgtcgtcccctggtggggtaaaaacaccatcttgagtccaaacggccaccaaccaaactccgacggcaacaaacaaacggcgttgctttgctcctcggtatctccgtgaccgctcaatctcccggctgtttccccggaattgcgtggactctctcatccacacgcaaaccgcctctccctcctctctcgtcctatccgccccggtgccgtagcctcacgggactcttcttcctcccttgctataaaatccccgccccctcccgtctcctctccacacatccaaactctcaatcgcaccgagaaaaatctcctagcgatcgaagcgaagcctctcccgatcctctcaag

SEQ ID NO: 2 - DNA, 981 bp, Zea mays
  source 1..981: mol_type = genomic DNA
tgcagcgtgacccggtcgtgcccctctctagagataatgagcattgcatgtctaagttataaaaaattaccacatattttttttgtcacacttgtttgaagtgcagtttatctatctttatacatatatttaaactttactctacgaataatataatctatagtactacaataatatcagtgttttagagaatcatataaatgaacagttagacatggtctaaaggacaattgagtattttgacaacaggactctacagttttatctttttagtgtgcatgtgttctcctttttttttgcaaatagcttcacctatataatacttcatccattttattagtacatccatttagggtttagggttaatggtttttatagactaatttttttagtacatctattttattctattttagcctctaaattaagaaaactaaaactctattttagtttttttatttaataatttagatataaaatagaataaaataaagtgactaaaaattaaacaaataccctttaagaaattaaaaaaactaaggaaacatttttcttgtttcgagtagataatgccagcctgttaaacgccgtcgatcgacgagtctaacggacaccaaccagcgaaccagcagcgtcgcgtcgggccaagcgaagcagacggcacggcatctctgtcgctgcctctggacccctctcgagagttccgctccaccgttggacttgctccgctgtcggcatccagaaattgcgtggcggagcggcagacgtgagccggcacggcaggcggcctcctcctcctctcacggcaccggcagctacgggggattcctttcccaccgctccttcgctttcccttcctcgcccgccgtaataaatagacaccccctccacaccctctttccccaacctcgtgttgttcggagcgcacacacacacaaccagatctcccccaaatccacccgtcggcacctccgcttcaag

SEQ ID NO: 3 - DNA, 1247 bp, Oryza sativa
  source 1..1247: mol_type = genomic DNA
tagctagcatactcgaggtcattcatatgcttgagaagagagtcgggatagtccaaaataaaacaaaggtaagattacctggtcaaaagtgaaaacatcagttaaaaggtggtataagtaaaatatcggtaataaaaggtggcccaaagtgaaatttactcttttctactattataaaaattgaggatgttttgtcggtactttgatacgtcatttttgtatgaattggtttttaagtttattcgcgatttggaaatgcatatctgtatttgagtcggtttttaagttcgttgcttttgtaaatacagagggatttgtataagaaatatctttaaaaaacccatatgctaatttgacataatttttgagaaaaatatatattcaggcgaattccacaatgaacaataataagattaaaatagcttgcccccgttgcagcgatgggtattttttctagtaaaataaaagataaacttagactcaaaacatttacaaaaacaacccctaaagtcctaaagcccaaagtgctatgcacgatccatagcaagcccagcccaacccaacccaacccaacccaccccagtgcagccaactggcaaatagtctccacccccggcactatcaccgtgagttgtccgcaccaccgcacgactcgcagccaaaaaaaaaaaaagaaagaaaaaaaagaaaaagaaaaacagcagctgggtccgggtcgtgggggccggaaaagcgaggaggatcgcgagcagcgacgaggcccggccctccctccgcttccaaagaaacgccccccatcgccactatatacatacccccccctctcctcccatccccccaaccctaccaccaccaccaccaccacctcctcccccctcgctgccggacgacgagctcctcccccctccccctccgccgccgccggtaaccaccccgcccctctcctctttctttctccgttttttttttcgtcacggtctcgatctttggccttggtagtttgggtgggcgagagcggcttcgtcgcccagatcggtgcgcgggaggggcgggatctcgcggctggcgactccgggcgtgagtcggcccggatcctcgcggggaatggggctctcggatgtagatcttctttctttcttctttttgtggtagaatttgaatccctcagcattgttcatcggtagtttttcttttcatgatttgtgacaaatgcagcctcgtgcggagcttttttgtaggcctagaag

SEQ ID NO: 4 - DNA, 691 bp, synthetic construct
  misc_feature 1..691: note = p35S promoter sequence
  source 1..691: mol_type = other DNA
gttcagaagaccagagggctattgagacttttcaacaaagggtaatatcgggaaacctcctcggattccattgcccagctatctgtcacttcatcgaaaggacagtagaaaaggaagatggcttctacaaatgccatcattgcgataaaggaaaggctatcgttcaagatgcctctaccgacagtggtcccaaagatggacccccacccacgaggaacatcgtggaaaaagaagacgttccaaccacgtcttcaaagcaagtggattgatgtgatacatggtggagcacgacactctcgtctactccaagaatatcaaagatacagtctcagaagaccagagggctattgagacttttcaacaaagggtaatatcgggaaacctcctcggattccattgcccagctatctgtcacttcatcgaaaggacagtagaaaaggaagatggcttctacaaatgccatcattgcgataaaggaaaggctatcgttcaagatgcctctaccgacagtggtcccaaagatggacccccacccacgaggaacatcgtggaaaaagaagacgttccaaccacgtcttcaaagcaagtggattgatgtgatatctccactgacgtaagggatgacgcacaatcccactatccttcgcaagacccttcctctatataaggaagttcatttcatttggagagg

SEQ ID NO: 5 - DNA, 519 bp, synthetic construct
  misc_feature 1..519: note = Ubi1 intron promoter sequence
  source 1..519: mol_type = other DNA
gtacgccgctcgtcctcccccccccccctctctaccttctctagatcggcgttccggtccatggttagggcccggtagttctacttctgttcatgtttgtgttagatccgtgtttgtgttagatccgtgctgctagcgttcgtacacggatgcgacctgtacgtcagacacgttctgattgctaacttgccagtgtttctctttggggaatcctgggatggctctagccgttccgcagacgggatcgatctaggataggtatacatgttgatgtgggttttactgatgcatatacatgatggcatatgcagcatctattcatatgctctaaccttgagtacctatctattataataaacaagtatgttttataattattttgatcttgatatacttggatgatggcatatgcagcagctatatgtggatttttttagccctgccttcatacgctatttatttgcttggtactgtttcttttgtcgatgctcaccctgttgtttggtgttacttctgcag

SEQ ID NO: 6 - DNA, 1500 bp, synthetic construct
  misc_feature 1..1500: note = pZmUbi1+Ubi1 intron promoter sequence
  source 1..1500: mol_type = other DNA
tgcagcgtgacccggtcgtgcccctctctagagataatgagcattgcatgtctaagttataaaaaattaccacatattttttttgtcacacttgtttgaagtgcagtttatctatctttatacatatatttaaactttactctacgaataatataatctatagtactacaataatatcagtgttttagagaatcatataaatgaacagttagacatggtctaaaggacaattgagtattttgacaacaggactctacagttttatctttttagtgtgcatgtgttctcctttttttttgcaaatagcttcacctatataatacttcatccattttattagtacatccatttagggtttagggttaatggtttttatagactaatttttttagtacatctattttattctattttagcctctaaattaagaaaactaaaactctattttagtttttttatttaataatttagatataaaatagaataaaataaagtgactaaaaattaaacaaataccctttaagaaattaaaaaaactaaggaaacatttttcttgtttcgagtagataatgccagcctgttaaacgccgtcgatcgacgagtctaacggacaccaaccagcgaaccagcagcgtcgcgtcgggccaagcgaagcagacggcacggcatctctgtcgctgcctctggacccctctcgagagttccgctccaccgttggacttgctccgctgtcggcatccagaaattgcgtggcggagcggcagacgtgagccggcacggcaggcggcctcctcctcctctcacggcaccggcagctacgggggattcctttcccaccgctccttcgctttcccttcctcgcccgccgtaataaatagacaccccctccacaccctctttccccaacctcgtgttgttcggagcgcacacacacacaaccagatctcccccaaatccacccgtcggcacctccgcttcaaggtacgccgctcgtcctcccccccccccctctctaccttctctagatcggcgttccggtccatggttagggcccggtagttctacttctgttcatgtttgtgttagatccgtgtttgtgttagatccgtgctgctagcgttcgtacacggatgcgacctgtacgtcagacacgttctgattgctaacttgccagtgtttctctttggggaatcctgggatggctctagccgttccgcagacgggatcgatctaggataggtatacatgttgatgtgggttttactgatgcatatacatgatggcatatgcagcatctattcatatgctctaaccttgagtacctatctattataataaacaagtatgttttataattattttgatcttgatatacttggatgatggcatatgcagcagctatatgtggatttttttagccctgccttcatacgctatttatttgcttggtactgtttcttttgtcgatgctcaccctgttgtttggtgttacttctgcag

SEQ ID NO: 7 - DNA, 2503 bp, Brachypodium distachyon
  source 1..2503: mol_type = genomic DNA
ggagaagaactcgagagggaattgcagatcatgaggcagatggctatttttgtgtcacatatgcgcaaaaagagaggctatatttgtgtccctaggttcttcgttgtattgcagtttccatatcaatctgacttggtcgcatgagaaattgatggttaaataatttgaatctctcatgtagtatcaactattagatattattttcaccaaatatatttccatcggagaagaagaggctacagaggaagcagaagagaggggtgggagaatttttacacttttgtacacccacttaaacagcaaaatccgtatgaaaacaggcccaccaaaacaatgccacgataacaatccgtagaaacaaaagcttcatttaacagcggcgcaacaaagcacgcttatccatggtagttgtagtccgtatgcgatccaaagatcacgattcacgcgtgacggacggacgacgcgtgccacaccacaactaacggcatccatggtagttgtagtccgtatgcgatccaaagatcacgattcacgcgtgacggacggacgacgcgcgccacaccacaactaacagcgtgagccagcgtccaaactccggatggcaacggggacgaaacccgtcgggtagtcactgcccaaacccgtccccgcaaccttcatcccaaacccgtccccgtttccggtcgcgggtttcagttttctaccagacccgtccccatcgggtttttcatccccgtcgggaaatccgaacccgccagcatttcagcaccaagccaaagttgcagcagcaacatgaataaaaaacaacccgtttcaacaccaagataaaacaaaacattataatttagacaacatttcacacgtataacaataacatatagttctcacatataacaacaccatttcacacataaaacaacaccatttgggataaaaatatgggctatatcaggccatttttatgggccatattgagttttcgtgggtttcacaggtaccggatttgtagaatgctgaaccgggtttgaaccgtaaaatccgcgggtattgaatttgacccaatcccgtcgtcccctggtggggtaaaaacaccatcttgagtccaaacggccaccaaccaaactccgacggcaacaaacaaacggcgttgctttgctcctcggtatctccgtgaccgctcaatctcccggctgtttccccggaattgcgtggactctctcatccacacgcaaaccgcctctccctcctctctcgtcctatccgccccggtgccgtagcctcacgggactcttcttcctcccttgctataaaatccccgccccctcccgtctcctctccacacatccaaactctcaatcgcaccgagaaaaatctcctagcgatcgaagcgaagcctctcccgatcctctcaaggtacgcccgtttcccgtcgatcctcctccttccgttcgtgttctgtagccgatcgattcgattcccttacacccgttcgtgttctctcgtggatcgatcgattgtttgttgctagaaggaactcgtagatctggcgtttatgaactgtgattcgggttagtccagatcgattcaggtcggtcgtcgttgagcctctcggctatgtctggattatcgtgtagatctgctggttcagttgattatgttcttctaggagtaatttcgttgggtcagcgcgatttctgcttaatctatgctgcttattgcgcctgtacctatctactaagctatgtgcacctgtaattttgctagattattcgttcatcctcgtagttggtttgtcacagtaatccgtatgggttctgacgatgttattgttggtcatacctaggcttctccagattttattttgttaaaattggatagatctgctactgatagttgatgatggaatttggtgctgaatctatgctatttattgcgcctatacctgatctatcgggctatgtacggctgtagtttactggattattcgttcatcctcggtagttggttcatcgtttgggttctgacgataatattgttgattatgcgtaggcttctgcagattgttgttaaaattggatacatcggttactgatggttgatgatagatttgtgctgaacctatctgtttattgctcctatacctgatctatagggctatgtatgcctgtaatttaccagattattcgttcatcctcgtagttggttcatctctataattcgtatgggttcttatgatgttatcgttgattatgcctagtcttatacagattattgtgtcaagattgaatatacctgctactgatcggtgataatttggttagtagtttgcaatctgctaggaacacgttaccactgtaatctgtaaacatggtttgccagagtagtttgttctactactcttgatatggttgctgattttagtcgcctccttttggatcatgtattgatgtccttgcagatttccgtgtacttaccccggcttttgtgtacttcgtgttaacag

SEQ ID NO: 8 - DNA, 535 bp, Zea mays
  source 1..535: mol_type = genomic DNA
gtccgccttgtttctcctctgtctcttgatctgactaatcttggtttatgattcgttgagtaattttggggaaagcttcgtccacagttttttttcgatgaacagtgccgcagtggcgctgatcttgtatgctatcctgcaatcgtggtgaacttatttcttttatatcctttactcccatgaaaaggctagtaatctttctcgatgtaacatcgtccagcactgctattaccgtgtggtccatccgacagtctggctgaacacatcatacgatctatggagcaaaaatctatcttccctgttctttaatgaaggacgtcattttcattagtatgatctaggaatgttgcaacttgcaaggaggcgtttctttctttgaatttaactaactcgttgagtggccctgtttctcggacgtaaggcctttgctgctccacacatgtccattcgaattttaccgtgtttagcaagggcgaaaagtttgcatcttgatgatttagcttgactatgcgattgctttcctggacccgtgcag

SEQ ID NO: 9 - DNA, 1090 bp, Brachypodium distachyon
  source 1..1090: mol_type = genomic DNA
gtacgcccgtttcccgtcgatcctcctccttccgttcgtgttctgtagccgatcgattcgattcccttacacccgttcgtgttctctcgtggatcgatcgattgtttgttgctagaaggaactcgtagatctggcgtttatgaactgtgattcgggttagtccagatcgattcaggtcggtcgtcgttgagcctctcggctatgtctggattatcgtgtagatctgctggttcagttgattatgttcttctaggagtaatttcgttgggtcagcgcgatttctgcttaatctatgctgcttattgcgcctgtacctatctactaagctatgtgcacctgtaattttgctagattattcgttcatcctcgtagttggtttgtcacagtaatccgtatgggttctgacgatgttattgttggtcatacctaggcttctccagattttattttgttaaaattggatagatctgctactgatagttgatgatggaatttggtgctgaatctatgctatttattgcgcctatacctgatctatcgggctatgtacggctgtagtttactggattattcgttcatcctcggtagttggttcatcgtttgggttctgacgataatattgttgattatgcgtaggcttctgcagattgttgttaaaattggatacatcggttactgatggttgatgatagatttgtgctgaacctatctgtttattgctcctatacctgatctatagggctatgtatgcctgtaatttaccagattattcgttcatcctcgtagttggttcatctctataattcgtatgggttcttatgatgttatcgttgattatgcctagtcttatacagattattgtgtcaagattgaatatacctgctactgatcggtgataatttggttagtagtttgcaatctgctaggaacacgttaccactgtaatctgtaaacatggtttgccagagtagtttgttctactactcttgatatggttgctgattttagtcgcctccttttggatcatgtattgatgtccttgcagatttccgtgtacttaccccggcttttgtgtacttcgtgttaacag

SEQ ID NO: 10 - DNA, 517 bp, Zea mays
  source 1..517: mol_type = genomic DNA
gtacgccgctcgtcctcccccccccctctctaccttctctagatcggcgttccggtccatggttagggcccggtagttctacttctgttcatgtttgtgttagatccgtgtttgtgttagatccgtgctgctagcgttcgtacacggatgcgacctgtacgtcagacacgttctgattgctaacttgccagtgtttctctttggggaatcctgggatggctctagccgttccgcagacgggatcgatctaggataggtatacatgttgatgtgggttttactgatgcatatacatgatggcatatgcagcatctattcatatgctctaaccttgagtacctatctattataataaacaagtatgttttataattattttgatcttgatatacttggatgatggcatatgcagcagctatatgtggatttttttagccctgccttcatacgctatttatttgcttggtactgtttcttttgtcgatgctcaccctgttgtttggtgttacttctgcag

SEQ ID NO: 11 - DNA, 258 bp, synthetic construct
  misc_feature 1..258: note = NosT terminator sequence
  source 1..258: mol_type = other DNA
cgatcgttcaaacatttggcaataaagtttcttaagattgaatcctgttgccggtcttgcgatgattatcatataatttctgttgaattacgttaagcatgtaataattaacatgtaatgcatgacgttatttatgagatgggtttttatgattagagtcccgcaattatacatttaatacgcgatagaaaacaaaatatagcgcgcaaactaggataaattatcgcgcgcggtgtcatctatgttactagatcgatc

SEQ ID NO: 12 - DNA, 204 bp, synthetic construct
  misc_feature 1..204: note = 35S terminator sequence
  source 1..204: mol_type = other DNA
gtcgatcgacaagctcgagtttctccataataatgtgtgagtagttcccagataagggaattagggttcctatagggtttcgctcatgtgttgagcatataagaaacccttagtatgtatttgtatttgtaaaatacttctatcaataaaatttctaattcctaaaaccaaaatccagtactaaaatccagatcccccgaatta

SEQ ID NO: 13 - DNA, 3771 bp, synthetic construct
  misc_feature 1..3771: note = codon optimized polynulceotide
  source 1..3771: mol_type = other DNA
atggcatctagcatggcaccaaagaaaaaaaggaaagtttccaaacttgaaaaatttacaaactgctactccctttccaagacgcttaggtttaaagcgatccccgttggcaagacccaagagaatatcgataacaaaagacttctggtcgaagatgaaaaaagggccgaagactacaagggggtcaagaagttgctcgatcgctattatctttcctttatcaacgatgtgcttcattcaatcaaactgaagaacttgaataactacattagccttttcagaaagaaaacgaggactgaaaaggagaacaaggaacttgagaatcttgaaataaaccttcgcaaagaaattgcaaaagccttcaaggggaacgaaggatataaatctcttttcaaaaaagacattatagaaacaattttgcctgagtttcttgacgacaaggatgaaattgcgctcgtcaatagctttaacggatttacaactgccttcacagggttcttcgacaatagggagaatatgtttagcgaggaggcaaaaagcacatccatcgcattcagatgcatcaatgaaaatcttacccggtacatatcgaatatggacatatttgaaaaagtggatgcaatattcgataagcacgaagtccaggagataaaggaaaagatactgaatagcgactatgatgtcgaagattttttcgaaggtgagttcttcaactttgtcctgactcaagaaggcattgatgtctataatgcaataattggaggttttgtgactgagtctggcgagaagataaagggcttgaacgagtatatcaatctctacaaccagaagactaagcaaaagttgcctaaatttaaaccgctttacaagcaagttttgagcgaccgggaaagcctttccttttacggtgaaggatacacgagcgatgaagaagtcctcgaagtcttccgcaacacactcaacaagaactcagaaatcttttcctcaattaaaaaattggagaagcttttcaagaacttcgatgaatactcttcggcggggatttttgtgaagaacggcccggcaatttccacaatatctaaagacattttcggagaatggaacgtgataagagacaagtggaatgcggagtatgatgacatacacctgaagaagaaggcagttgtgactgaaaaatacgaagatgacaggagaaaaagctttaaaaagatcgggtccttttcactggaacagctgcaggagtatgccgacgccgatctttcggttgtcgaaaagctcaaagaaataattatccagaaggtcgatgaaatctacaaggtgtacggctcaagcgagaagctctttgatgctgacttcgtgttggagaagtctcttaaaaaaaacgacgcagtcgtcgcgataatgaaagatttgctggattcagtgaaatccttcgagaattatatcaaagccttcttcggcgaggggaaggagacaaacagggatgagtccttctatggagacttcgttctggcttacgacatccttcttaaggtcgaccacatctatgacgcaattcggaactatgtgacgcagaagccgtattcgaaagataagttcaagctctatttccaaaaccctcaatttatgggtgggtgggataaagacaaagagaccgattaccgggcaacaattttgcggtacgggtctaaatattacctcgctataatggataagaaatacgctaaatgtctccagaaaattgacaaagatgacgtcaacggcaattatgaaaaaatcaattataaactccttcctggcccaaataaaatgctcccgaaggtgtttttttccaaaaagtggatggcctattataatccatcagaggatattcagaaaatctataaaaatgggacctttaagaagggtgacatgtttaacctgaacgattgccacaagcttatagattttttcaaagactctattagccgctatcccaaatggtctaatgcttatgatttcaacttctctgaaactgaaaagtacaaagatattgcaggattctaccgcgaagttgaagaacaaggttataaggtttcctttgagtctgcgtccaagaaagaggtcgataagttggtcgaagaagggaaattgtatatgtttcaaatttacaataaagacttttccgacaagtcccatggtacacctaatctgcataccatgtacttcaaactgctgttcgatgagaataatcacggtcagattcgcctgagcggaggggcggaactcttcatgaggagagcatcgttgaaaaaagaggagctcgtcgtgcatccggctaacagccccattgctaacaagaatccggataatccaaagaagactactaccctctcctatgacgtctataaggataagagattctctgaggaccagtacgagttgcacatccctattgcgataaataaatgccctaagaacatctttaaaatcaatactgaggtcagagtcctgcttaagcacgacgacaacccgtatgtgatcgggattgataggggtgaaaggaacttgctttatattgtggttgtcgatggaaaaggtaatatagtggaacaatactctctgaatgaaattatcaacaacttcaatggcattaggatcaagaccgactatcattctctgttggacaagaaagagaaagagcgcttcgaggcacggcaaaactggacgtctattgagaacatcaaggagcttaaggctggttacatttctcaggttgtgcacaaaatttgcgaactggtcgagaaatatgatgccgttatcgcacttgaagatctcaacagcggatttaagaattctcgggtgaaagtcgaaaaacaggtgtatcaaaaattcgaaaagatgctgatcgacaagctcaattatatggttgataaaaagagcaacccatgcgccacggggggtgcgcttaagggctatcagattacgaacaaatttgaatccttcaagtcaatgtcgacgcaaaatgggtttatattctatataccggcgtggcttacatctaaaatagatcctagcactgggttcgtgaacctgctgaaaaccaagtacacttcaatcgcagattctaaaaaatttataagcagcttcgacagaatcatgtatgtgcccgaggaagacctcttcgagtttgcccttgattacaaaaatttctcaagaacggatgcagactacataaagaagtggaagctgtactcttatgggaaccggattcggatattcagaaatccgaaaaaaaacaatgtctttgattgggaggaagtttgtcttacctctgcttacaaagagctgttcaataaatatggcattaattaccagcaaggtgatatccgggcgctcctttgcgaacagtctgacaaagctttctattcttcatttatggcgctcatgtcattgatgctgcagatgaggaatagcattacggggaggactgatgttgactttctgatctcgcccgtgaaaaattctgatggaatcttctacgattccaggaattatgaggcccaggaaaatgctatccttcccaagaacgcagacgcaaatggcgcgtacaatatagctcgcaaggttttgtgggctataggccaattcaagaaagccgaagacgaaaagctggacaaagttaagattgctatatctaacaaagagtggcttgagtatgcgcaaacatctgttaaacacaaacgccccgcggctacaaagaaggctggccaggcaaagaagaagaagtga

SEQ ID NO: 14 - DNA, 3684 bp, synthetic construct
  misc_feature 1..3684: note = codon optimized polynucleotide
  source 1..3684: mol_type = other DNA
atgtccaaacttgaaaaatttacaaactgctactccctttccaagacgcttaggtttaaagcgatccccgttggcaagacccaagagaatatcgataacaaaagacttctggtcgaagatgaaaaaagggccgaagactacaagggggtcaagaagttgctcgatcgctattatctttcctttatcaacgatgtgcttcattcaatcaaactgaagaacttgaataactacattagccttttcagaaagaaaacgaggactgaaaaggagaacaaggaacttgagaatcttgaaataaaccttcgcaaagaaattgcaaaagccttcaaggggaacgaaggatataaatctcttttcaaaaaagacattatagaaacaattttgcctgagtttcttgacgacaaggatgaaattgcgctcgtcaatagctttaacggatttacaactgccttcacagggttcttcgacaatagggagaatatgtttagcgaggaggcaaaaagcacatccatcgcattcagatgcatcaatgaaaatcttacccggtacatatcgaatatggacatatttgaaaaagtggatgcaatattcgataagcacgaagtccaggagataaaggaaaagatactgaatagcgactatgatgtcgaagattttttcgaaggtgagttcttcaactttgtcctgactcaagaaggcattgatgtctataatgcaataattggaggttttgtgactgagtctggcgagaagataaagggcttgaacgagtatatcaatctctacaaccagaagactaagcaaaagttgcctaaatttaaaccgctttacaagcaagttttgagcgaccgggaaagcctttccttttacggtgaaggatacacgagcgatgaagaagtcctcgaagtcttccgcaacacactcaacaagaactcagaaatcttttcctcaattaaaaaattggagaagcttttcaagaacttcgatgaatactcttcggcggggatttttgtgaagaacggcccggcaatttccacaatatctaaagacattttcggagaatggaacgtgataagagacaagtggaatgcggagtatgatgacatacacctgaagaagaaggcagttgtgactgaaaaatacgaagatgacaggagaaaaagctttaaaaagatcgggtccttttcactggaacagctgcaggagtatgccgacgccgatctttcggttgtcgaaaagctcaaagaaataattatccagaaggtcgatgaaatctacaaggtgtacggctcaagcgagaagctctttgatgctgacttcgtgttggagaagtctcttaaaaaaaacgacgcagtcgtcgcgataatgaaagatttgctggattcagtgaaatccttcgagaattatatcaaagccttcttcggcgaggggaaggagacaaacagggatgagtccttctatggagacttcgttctggcttacgacatccttcttaaggtcgaccacatctatgacgcaattcggaactatgtgacgcagaagccgtattcgaaagataagttcaagctctatttccaaaaccctcaatttatgggtgggtgggataaagacaaagagaccgattaccgggcaacaattttgcggtacgggtctaaatattacctcgctataatggataagaaatacgctaaatgtctccagaaaattgacaaagatgacgtcaacggcaattatgaaaaaatcaattataaactccttcctggcccaaataaaatgctcccgaaggtgtttttttccaaaaagtggatggcctattataatccatcagaggatattcagaaaatctataaaaatgggacctttaagaagggtgacatgtttaacctgaacgattgccacaagcttatagattttttcaaagactctattagccgctatcccaaatggtctaatgcttatgatttcaacttctctgaaactgaaaagtacaaagatattgcaggattctaccgcgaagttgaagaacaaggttataaggtttcctttgagtctgcgtccaagaaagaggtcgataagttggtcgaagaagggaaattgtatatgtttcaaatttacaataaagacttttccgacaagtcccatggtacacctaatctgcataccatgtacttcaaactgctgttcgatgagaataatcacggtcagattcgcctgagcggaggggcggaactcttcatgaggagagcatcgttgaaaaaagaggagctcgtcgtgcatccggctaacagccccattgctaacaagaatccggataatccaaagaagactactaccctctcctatgacgtctataaggataagagattctctgaggaccagtacgagttgcacatccctattgcgataaataaatgccctaagaacatctttaaaatcaatactgaggtcagagtcctgcttaagcacgacgacaacccgtatgtgatcgggattgataggggtgaaaggaacttgctttatattgtggttgtcgatggaaaaggtaatatagtggaacaatactctctgaatgaaattatcaacaacttcaatggcattaggatcaagaccgactatcattctctgttggacaagaaagagaaagagcgcttcgaggcacggcaaaactggacgtctattgagaacatcaaggagcttaaggctggttacatttctcaggttgtgcacaaaatttgcgaactggtcgagaaatatgatgccgttatcgcacttgaagatctcaacagcggatttaagaattctcgggtgaaagtcgaaaaacaggtgtatcaaaaattcgaaaagatgctgatcgacaagctcaattatatggttgataaaaagagcaacccatgcgccacggggggtgcgcttaagggctatcagattacgaacaaatttgaatccttcaagtcaatgtcgacgcaaaatgggtttatattctatataccggcgtggcttacatctaaaatagatcctagcactgggttcgtgaacctgctgaaaaccaagtacacttcaatcgcagattctaaaaaatttataagcagcttcgacagaatcatgtatgtgcccgaggaagacctcttcgagtttgcccttgattacaaaaatttctcaagaacggatgcagactacataaagaagtggaagctgtactcttatgggaaccggattcggatattcagaaatccgaaaaaaaacaatgtctttgattgggaggaagtttgtcttacctctgcttacaaagagctgttcaataaatatggcattaattaccagcaaggtgatatccgggcgctcctttgcgaacagtctgacaaagctttctattcttcatttatggcgctcatgtcattgatgctgcagatgaggaatagcattacggggaggactgatgttgactttctgatctcgcccgtgaaaaattctgatggaatcttctacgattccaggaattatgaggcccaggaaaatgctatccttcccaagaacgcagacgcaaatggcgcgtacaatatagctcgcaaggttttgtgggctataggccaattcaagaaagccgaagacgaaaagctggacaaagttaagattgctatatctaacaaagagtggcttgagtatgcgcaaacatctgttaaacac

SEQ ID NO: 15 - protein, 1255 aa, synthetic construct
  REGION 1..1255: note = codon optimized polypeptide
MASSMAPKKKRKVSKLEKFTNCYSLSKTLRFKAIPVGKTQENIDNKRLLVEDEKRAEDYKGVKKLLDRYYLSFINDVLHSIKLKNLNNYISLFRKKTRTEKENKELENLEINLRKEIAKAFKGNEGYKSLFKKDIIETILPEFLDDKDEIALVNSFNGFTTAFTGFFDNRENMFSEEAKSTSIAFRCINENLTRYISNMDIFEKVDAIFDKHEVQEIKEKILNSDYDVEDFFEGEFFNFVLTQEGIDVYNAIIGGFVTESGEKIKGLNEYINLYNQKTKQKLPKFKPLYKQVLSDRESLSFYGEGYTSDEEVLEVFRNTLNKNSEIFSSIKKLEKLFKNFDEYSSAGIFVKNGPAISTISKDIFGEWNVIRDKWNAEYDDIHLKKKAVVTEKYEDDRRKSFKKIGSFSLEQLQEYADADLSVVEKLKEIIIQKVDEIYKVYGSSEKLFDADFVLEKSLKKNDAVVAIMKDLLDSVKSFENYIKAFFGEGKETNRDESFYGDFVLAYDILLKVDHIYDAIRNYVTQKPYSKDKFKLYFQNPQFMGGWDKDKETDYRATILRYGSKYYLAIMDKKYAKCLQKIDKDDVNGNYEKINYKLLPGPNKMLPKVFFSKKWMAYYNPSEDIQKIYKNGTFKKGDMFNLNDCHKLIDFFKDSISRYPKWSNAYDFNFSETEKYKDIAGFYREVEEQGYKVSFESASKKEVDKLVEEGKLYMFQIYNKDFSDKSHGTPNLHTMYFKLLFDENNHGQIRLSGGAELFMRRASLKKEELVVHPANSPIANKNPDNPKKTTTLSYDVYKDKRFSEDQYELHIPIAINKCPKNIFKINTEVRVLLKHDDNPYVIGIDRGERNLLYIVVVDGKGNIVEQYSLNEIINNFNGIRIKTDYHSLLDKKEKERFEARQNWTSIENIKELKAGYISQVVHKICELVEKYDAVIALEDLNSGFKNSRVKVEKQVYQKFEKMLIDKLNYMVDKKSNPCATGGALKGYQITNKFESFKSMSTQNGFIFYIPAWLTSKIDPSTGFVNLLKTKYTSIADSKKFISSFDRIMYVPEEDLFEFALDYKNFSRTDADYIKKWKLYSYGNRIRIFRNPKKNNVFDWEEVCLTSAYKELFNKYGINYQQGDIRALLCEQSDKAFYSSFMALMSLMLQMRNSITGRTDVDFLISPVKNSDGIFYDSRNYEAQENAILPKNADANGAYNIARKVLWAIGQFKKAEDEKLDKVKIAISNKEWLEYAQTSVKHKRPAATKKAGQAKKK

SEQ ID NO: 16 - protein, 1228 aa, Lachnospiraceae bacterium
MSKLEKFTNCYSLSKTLRFKAIPVGKTQENIDNKRLLVEDEKRAEDYKGVKKLLDRYYLSFINDVLHSIKLKNLNNYISLFRKKTRTEKENKELENLEINLRKEIAKAFKGNEGYKSLFKKDIIETILPEFLDDKDEIALVNSFNGFTTAFTGFFDNRENMFSEEAKSTSIAFRCINENLTRYISNMDIFEKVDAIFDKHEVQEIKEKILNSDYDVEDFFEGEFFNFVLTQEGIDVYNAIIGGFVTESGEKIKGLNEYINLYNQKTKQKLPKFKPLYKQVLSDRESLSFYGEGYTSDEEVLEVFRNTLNKNSEIFSSIKKLEKLFKNFDEYSSAGIFVKNGPAISTISKDIFGEWNVIRDKWNAEYDDIHLKKKAVVTEKYEDDRRKSFKKIGSFSLEQLQEYADADLSVVEKLKEIIIQKVDEIYKVYGSSEKLFDADFVLEKSLKKNDAVVAIMKDLLDSVKSFENYIKAFFGEGKETNRDESFYGDFVLAYDILLKVDHIYDAIRNYVTQKPYSKDKFKLYFQNPQFMGGWDKDKETDYRATILRYGSKYYLAIMDKKYAKCLQKIDKDDVNGNYEKINYKLLPGPNKMLPKVFFSKKWMAYYNPSEDIQKIYKNGTFKKGDMFNLNDCHKLIDFFKDSISRYPKWSNAYDFNFSETEKYKDIAGFYREVEEQGYKVSFESASKKEVDKLVEEGKLYMFQIYNKDFSDKSHGTPNLHTMYFKLLFDENNHGQIRLSGGAELFMRRASLKKEELVVHPANSPIANKNPDNPKKTTTLSYDVYKDKRFSEDQYELHIPIAINKCPKNIFKINTEVRVLLKHDDNPYVIGIDRGERNLLYIVVVDGKGNIVEQYSLNEIINNFNGIRIKTDYHSLLDKKEKERFEARQNWTSIENIKELKAGYISQVVHKICELVEKYDAVIALEDLNSGFKNSRVKVEKQVYQKFEKMLIDKLNYMVDKKSNPCATGGALKGYQITNKFESFKSMSTQNGFIFYIPAWLTSKIDPSTGFVNLLKTKYTSIADSKKFISSFDRIMYVPEEDLFEFALDYKNFSRTDADYIKKWKLYSYGNRIRIFRNPKKNNVFDWEEVCLTSAYKELFNKYGINYQQGDIRALLCEQSDKAFYSSFMALMSLMLQMRNSITGRTDVDFLISPVKNSDGIFYDSRNYEAQENAILPKNADANGAYNIARKVLWAIGQFKKAEDEKLDKVKIAISNKEWLEYAQTSVKH

SEQ ID NO: 17 - DNA, 37 bp, synthetic construct
  misc_feature 1..37: note = HH ribozyme encoding sequence
  source 1..37: mol_type = other DNA
ctgatgagtccgtgaggacgaaacgagtaagctcgtc

SEQ ID NO: 18 - RNA, 37 nt, synthetic construct
  misc_feature 1..37: note = HH ribozyme sequence
  source 1..37: mol_type = other RNA
ctgatgagtccgtgaggacgaaacgagtaagctcgtc

SEQ ID NO: 19 - DNA, 53 bp, Oryza sativa
  source 1..53: mol_type = other DNA
ccgccaacactgccaatgccggtcccaagcccggataaaagtggagggggcgg

SEQ ID NO: 20 - RNA, 53 nt, Oryza sativa
  source 1..53: mol_type = other RNA
ccgccaacactgccaatgccggtcccaagcccggataaaagtggagggggcgg

SEQ ID NO: 21 - DNA, 63 bp, Helianthus annuus
  source 1..63: mol_type = other DNA
gcggggggcgtcagtcctactctgcacctcctcgtggtgtcgcctgggaaccctctttcgcaa

SEQ ID NO: 22 - RNA, 63 nt, Helianthus annuus
  source 1..63: mol_type = other RNA
gcggggggcgtcagtcctactctgcacctcctcgtggtgtcgcctgggaaccctctttcgcaa

SEQ ID NO: 23 - DNA, 86 bp, Helianthus annuus
  source 1..86: mol_type = other DNA
gcggggggcgtcagtcctactctgcacctcctcgtggtgtcgcctgggaaccctctttcgcaagaaagaggagccaagcagagagg

SEQ ID NO: 24 - RNA, 86 nt, Helianthus annuus
  source 1..86: mol_type = other RNA
gcggggggcgtcagtcctactctgcacctcctcgtggtgtcgcctgggaaccctctttcgcaagaaagaggagccaagcagagagg

SEQ ID NO: 25 - DNA, 80 bp, Cynara scolymus
  source 1..80: mol_type = other DNA
ggcgtcagtcctactctgcacctcctcgtggtgtcgcctgggaaccctctttcacaagaaagaggagccaagcagagagg

SEQ ID NO: 26 - RNA, 80 nt, Cynara scolymus
  source 1..80: mol_type = other RNA
ggcgtcagtcctactctgcacctcctcgtggtgtcgcctgggaaccctctttcacaagaaagaggagccaagcagagagg

SEQ ID NO: 27 - DNA, 68 bp, Hepatitis Delta Virus
  source 1..68: mol_type = other DNA
ggccggcatggtcccagcctcctcgctggcgccggctgggcaacatgcttcggcatggcgaatgggac

SEQ ID NO: 28 - RNA, 68 nt, Hepatitis Delta Virus
  source 1..68: mol_type = other RNA
ggccggcatggtcccagcctcctcgctggcgccggctgggcaacatgcttcggcatggcgaatgggac

SEQ ID NO: 29 - DNA, 21 bp, synthetic construct
  misc_feature 1..21: note = scaffold RNA encoding sequnece
  source 1..21: mol_type = other DNA
taatttctactaagtgtagat

SEQ ID NO: 30 - RNA, 21 nt, synthetic construct
  misc_feature 1..21: note = scaffold RNA sequence
  source 1..21: mol_type = other RNA
taatttctactaagtgtagat

SEQ ID NO: 31 - DNA, 717 bp, synthetic construct
  misc_feature 1..717: note = tdTomato polynucleotide
  source 1..717: mol_type = other DNA
atggtgagcaagggcgaggaggtcatcaaagagttcatgcgcttcaaggtgcgcatggagggctccatgaacggccacgagttcgagatcgagggcgagggcgagggccgcccctacgagggcacccagaccgccaagctgaaggtgaccaagggcggccccctgcccttcgcctgggacatcctgtccccccagttcatgtacggctccaaggcgtacgtgaagcaccccgccgacatccccgattacaagaagctgtccttccccgagggcttcaagtgggagcgcgtgatgaacttcgaggacggcggtctggtgaccgtgacccaggactcctccctgcaggacggcacgctgatctacaaggtgaagatgcgcggcaccaacttcccccccgacggccccgtaatgcagaagaagaccatgggctgggaggcctccaccgagcgcctgtacccccgcgacggcgtgctgaagggcgagatccaccaggccctgaagctgaaggacggcggccactacctggtggagttcaagaccatctacatggccaagaagcccgtgcaactgcccggctactactacgtggacaccaagctggacatcacctcccacaacgaggactacaccatcgtggaacagtacgagcgctccgagggccgccaccacctgttcctgtacggcatggacgagctgtacaagtctagaggtacctga

SEQ ID NO: 32 - DNA, 720 bp, synthetic construct
  misc_feature 1..720: note = mNeoGreen polynucleotide
  source 1..720: mol_type = other DNA
atggcgtcctccgtgagtaaaggagaagaagataacatggcttcgcttccagccacacatgagcttcacatcttcggttccatcaacggcgttgacttcgatatggtcggacaaggcactgggaaccctaatgacggatacgaagagctgaacctcaagagcaccaaaggtgatcttcagttttctccatggattctggtgccacacattggctacggattccatcaataccttccataccctgacggaatgagtccattccaagcagccatggttgatggctccggataccaagtccacaggacaatgcagtttgaggacggtgcttcgctcaccgtcaactaccgttacacttacgaagggagccacatcaaaggagaagcccaagtgaaggggacaggctttcctgctgatggacctgtcatgaccaactccttaactgccgctgattggtgccggtccaagaaaacctaccctaacgacaagaccatcattagtaccttcaaatggtcttacaccacaggcaatggcaagagatatcgctctacagccaggactacctacacattcgctaaaccaatggccgctaactaccttaagaaccaacccatgtacgtgttccgtaagactgagttgaaacattccaagaccgaacttaacttcaaggagtggcagaaggcatttaccgacgtaatgggcatggatgaactatacaaataa

SEQ ID NO: 33 - DNA, 5693 bp, synthetic construct
  misc_feature 1..5693: note = pGEP424 tdT embedded gRNA delivery vector
  source 1..5693: mol_type = other DNA
ctgacgcgccctgtagcggcacgtcacctgcatcaggaattcaggagaagaactcgagagggaattgcagatcatgaggcagatggctatttttgtgtcacatatgcgcaaaaagagaggctatatttgtgtccctaggttcttcgttgtattgcagtttccatatcaatctgacttggtcgcatgagaaattgatggttaaataatttgaatctctcatgtagtatcaactattagatattattttcaccaaatatatttccatcggagaagaagaggctacagaggaagcagaagagaggggtgggagaatttttacacttttgtacacccacttaaacagcaaaatccgtatgaaaacaggcccaccaaaacaatgccacgataacaatccgtagaaacaaaagcttcatttaacagcggcgcaacaaagcacgcttatccatggtagttgtagtccgtatgcgatccaaagatcacgattcacgcgtgacggacggacgacgcgtgccacaccacaactaacggcatccatggtagttgtagtccgtatgcgatccaaagatcacgattcacgcgtgacggacggacgacgcgcgccacaccacaactaacagcgtgagccagcgtccaaactccggatggcaacggggacgaaacccgtcgggtagtcactgcccaaacccgtccccgcaaccttcatcccaaacccgtccccgtttccggtcgcgggtttcagttttctaccagacccgtccccatcgggtttttcatccccgtcgggaaatccgaacccgccagcatttcagcaccaagccaaagttgcagcagcaacatgaataaaaaacaacccgtttcaacaccaagataaaacaaaacattataatttagacaacatttcacacgtataacaataacatatagttctcacatataacaacaccatttcacacataaaacaacaccatttgggataaaaatatgggctatatcaggccatttttatgggccatattgagttttcgtgggtttcacaggtaccggatttgtagaatgctgaaccgggtttgaaccgtaaaatccgcgggtattgaatttgacccaatcccgtcgtcccctggtggggtaaaaacaccatcttgagtccaaacggccaccaaccaaactccgacggcaacaaacaaacggcgttgctttgctcctcggtatctccgtgaccgctcaatctcccggctgtttccccggaattgcgtggactctctcatccacacgcaaaccgcctctccctcctctctcgtcctatccgccccggtgccgtagcctcacgggactcttcttcctcccttgctataaaatccccgccccctcctgtctcctctccacacatccaaactctcaatcgcaccgagaaaaatctcctagcgatcgaagcgaagcctctcccgatcctctcaaggtacgcccgtttcccgtcgatcctcctccttccgttcgtgttctgtagccgatcgattcgattcccttacacccgttcgtgttctctcgtggatcgatcgattgtttgttgctagaaggaactcgtagatctggcgtttatgaactgtgattcgggttagtccagatcgattcaggtcggtcgtcgttgagcctctcggctatgtctggattatcgtgtagatctgctggttcagttgattatgttcttctaggagtaatttcgttgggtcagcgcgatttctgcttaatctatgctgcttattgcgcctgtacctatctactaagctatgtgcacctgtaattttgctagattattcgttcatcctcgtagttggtttgtcacagtaatccgtatgggttctgacgatgttattgttggtcatacctaggcttctccagattttattttgttaaaattggatagatctgctactgatagttgatgatggaatttggtgctgaatctatgctatttattgcgcctatacctgatctatcgggctatgtacggctgtagtttactggattattcgttcatcctcggtagttggttcatcgtttgggttctgacgataatattgttgattatgcgtaggcttctgcagattgttgttaaaattggatacatcggttactgatggttgatgatagatttgtgctgaacctatctgtttattgctcctatacctgatctatagggctatgtatgcctgtaatttaccagattattcgttcatcctcgtagttggttcatctctataattcgtatgggttcttatgatgttatcgttgattatgcctagtcttatacagattattgtgtcaagattgaatatacctgctactgatcggtgataatttggttagtagtttgcaatctgctaggaacacgttaccactgtaatctgtaaacatggtttgccagagtagtttgttctactactcttgatatggttgctgattttagtcgcctccttttggatcatgtattgatgtccttgcagatttccgtgtacttaccccggcttttgtgtacttcgtgttaacagctctagaggatcctctcaacacaacatatacaaaacaaacgaatctcaagcaatcaagcattctacttctattgcagcaatttaaatcatttcttttaaagcaaaagcaattttctgaaaattttcaccatttacgaacgatagggcgcgatcccgccaccatggtgagcaagggcgaggaggtcatcaaagagttcatgcgcttcaaggtgcgcatggagggctccatgaacggccacgagttcgagatcgagggcgagggcgagggccgcccctacgagggcacccagaccgccaagctgaaggtgaccaagggcggccccctgcccttcgcctgggacatcctgtccccccagttcatgtacggctccaaggcgtacgtgaagcaccccgccgacatccccgattacaagaagctgtccttccccgagggcttcaagtgggagcgcgtgatgaacttcgaggacggcggtctggtgaccgtgacccaggactcctccctgcaggacggcacgctgatctacaaggtgaagatgcgcggcaccaacttcccccccgacggccccgtaatgcagaagaagaccatgggctgggaggcctccaccgagcgcctgtacccccgcgacggcgtgctgaagggcgagatccaccaggccctgaagctgaaggacggcggccactacctggtggagttcaagaccatctacatggccaagaagcccgtgcaactgcccggctactactacgtggacaccaagctggacatcacctcccacaacgaggactacaccatcgtggaacagtacgagcgctccgagggccgccaccacctgttcctgtacggcatggacgagctgtacaagtctagaggtacctgataatttctactaagtgtagatgagacggagctcagtctgaccgcggcgtctcttaatttctactaagtgtagatcgaatttccccgatcgttcaaacatttggcaataaagtttcttaagattgaatcctgttgccggtcttgcgatgattatcatataatttctgttgaattacgttaagcatgtaataattaacatgtaatgcatgacgttatttatgagatgggtttttatgattagagtcccgcaattatacatttaatacgcgatagaaaacaaaatatagcgcgcaaactaggataaattatcgcgcgcggtgtcatctatgttactagatcgctcgacgcggccgccatggcctctagtggatcaggtgtcgttcggctgcggcgagcggtatcagctcactcaaaggcggtaatacggttatccacagaatcaggggataacgcaggaaagaacatgtgagcaaaaggccagcaaaaggccaggaaccgtaaaaaggccgcgttgctggcgtttttccataggctccgcccccctgacgagcatcacaaaaatcgacgctcaagtcagaggtggcgaaacccgacaggactataaagataccaggcgtttccccctggaagctccctcgtgcgctctcctgttccgaccctgccgcttaccggatacctgtccgcctttctcccttcgggaagcgtggcgctttctcatagctcacgctgtaggtatctcagttcggtgtaggtcgttcgctccaagctgggctgtgtgcacgaaccccccgttcagcccgaccgctgcgccttatccggtaactatcgtcttgagtccaacccggtaagacacgacttatcgccactggcagcagccactggtaacaggattagcagagcgaggtatgtaggcggtgctacagagttcttgaagtggtggcctaactacggctacactagaaggacagtatttggtatctgcgctctgctgaagccagttaccttcggaaaaagagttggtagctcttgatccggcaaacaaaccaccgctggtagcggtggtttttttgtttgcaagcagcagattacgcgcagaaaaaaaggatctcaagaagatcctttgatcttttctacggggtctgacgctcagtggaacgaaaactcacgttaagggattttggtcatgagattatcaaaaaggatcttcacctagatccttttaaattaaaaatgaagttttaaatcaatctaaagtatatatgagtaaacttggtctgacagttaccaatgcttaatcagtgaggcacctatctcagcgatctgtctatttcgttcatccatagttgcctgactccccgtcgtgtagataactacgatacgggagggcttaccatctggccccagtgctgcaatgataccgcgagacccacgctcaccggctccagatttatcagcaataaaccagccagccggaagggccgagcgcagaagtggtcctgcaactttatccgcctccatccagtctattaattgttgccgggaagctagagtaagtagttcgccagttaatagtttgcgcaacgttgttgccattgctacaggcatcgtggtgtcacgctcgtcgtttggtatggcttcattcagctccggttcccaacgatcaaggcgagttacatgatcccccatgttgtgcaaaaaagcggttagctccttcggtcctccgatcgttgtcagaagtaagttggccgcagtgttatcactcatggttatggcagcactgcataattctcttactgtcatgccatccgtaagatgcttttctgtgactggtgagtactcaaccaagtcattctgagaatagtgtatgcggcgaccgagttgctcttgcccggcgtcaatacgggataataccgcgccacatagcagaactttaaaagtgctcatcattggaaaacgttcttcggggcgaaaactctcaaggatcttaccgctgttgagatccagttcgatgtaacccactcgtgcacccaactgatcttcagcatcttttactttcaccagcgtttctgggtgagcaaaaacaggaaggcaaaatgccgcaaaaaagggaataagggcgacacggaaatgttgaatactcatactcttcctttttcaatattattgaagcatttatcagggttattgtctcatgagcggatacatatttgaatgtatttagaaaaataaacaaataggggttccgcgcacatttccccgaaaagtgccac

SEQ ID NO: 34 - DNA, 4959 bp, synthetic construct
  misc_feature 1..4959: note = pGEP425 vector control guide RNA delivery without tdT
  source 1..4959: mol_type = other DNA
ctgacgcgccctgtagcggcacgtcacctgcatcaggaattcaggagaagaactcgagagggaattgcagatcatgaggcagatggctatttttgtgtcacatatgcgcaaaaagagaggctatatttgtgtccctaggttcttcgttgtattgcagtttccatatcaatctgacttggtcgcatgagaaattgatggttaaataatttgaatctctcatgtagtatcaactattagatattattttcaccaaatatatttccatcggagaagaagaggctacagaggaagcagaagagaggggtgggagaatttttacacttttgtacacccacttaaacagcaaaatccgtatgaaaacaggcccaccaaaacaatgccacgataacaatccgtagaaacaaaagcttcatttaacagcggcgcaacaaagcacgcttatccatggtagttgtagtccgtatgcgatccaaagatcacgattcacgcgtgacggacggacgacgcgtgccacaccacaactaacggcatccatggtagttgtagtccgtatgcgatccaaagatcacgattcacgcgtgacggacggacgacgcgcgccacaccacaactaacagcgtgagccagcgtccaaactccggatggcaacggggacgaaacccgtcgggtagtcactgcccaaacccgtccccgcaaccttcatcccaaacccgtccccgtttccggtcgcgggtttcagttttctaccagacccgtccccatcgggtttttcatccccgtcgggaaatccgaacccgccagcatttcagcaccaagccaaagttgcagcagcaacatgaataaaaaacaacccgtttcaacaccaagataaaacaaaacattataatttagacaacatttcacacgtataacaataacatatagttctcacatataacaacaccatttcacacataaaacaacaccatttgggataaaaatatgggctatatcaggccatttttatgggccatattgagttttcgtgggtttcacaggtaccggatttgtagaatgctgaaccgggtttgaaccgtaaaatccgcgggtattgaatttgacccaatcccgtcgtcccctggtggggtaaaaacaccatcttgagtccaaacggccaccaaccaaactccgacggcaacaaacaaacggcgttgctttgctcctcggtatctccgtgaccgctcaatctcccggctgtttccccggaattgcgtggactctctcatccacacgcaaaccgcctctccctcctctctcgtcctatccgccccggtgccgtagcctcacgggactcttcttcctcccttgctataaaatccccgccccctcctgtctcctctccacacatccaaactctcaatcgcaccgagaaaaatctcctagcgatcgaagcgaagcctctcccgatcctctcaaggtacgcccgtttcccgtcgatcctcctccttccgttcgtgttctgtagccgatcgattcgattcccttacacccgttcgtgttctctcgtggatcgatcgattgtttgttgctagaaggaactcgtagatctggcgtttatgaactgtgattcgggttagtccagatcgattcaggtcggtcgtcgttgagcctctcggctatgtctggattatcgtgtagatctgctggttcagttgattatgttcttctaggagtaatttcgttgggtcagcgcgatttctgcttaatctatgctgcttattgcgcctgtacctatctactaagctatgtgcacctgtaattttgctagattattcgttcatcctcgtagttggtttgtcacagtaatccgtatgggttctgacgatgttattgttggtcatacctaggcttctccagattttattttgttaaaattggatagatctgctactgatagttgatgatggaatttggtgctgaatctatgctatttattgcgcctatacctgatctatcgggctatgtacggctgtagtttactggattattcgttcatcctcggtagttggttcatcgtttgggttctgacgataatattgttgattatgcgtaggcttctgcagattgttgttaaaattggatacatcggttactgatggttgatgatagatttgtgctgaacctatctgtttattgctcctatacctgatctatagggctatgtatgcctgtaatttaccagattattcgttcatcctcgtagttggttcatctctataattcgtatgggttcttatgatgttatcgttgattatgcctagtcttatacagattattgtgtcaagattgaatatacctgctactgatcggtgataatttggttagtagtttgcaatctgctaggaacacgttaccactgtaatctgtaaacatggtttgccagagtagtttgttctactactcttgatatggttgctgattttagtcgcctccttttggatcatgtattgatgtccttgcagatttccgtgtacttaccccggcttttgtgtacttcgtgttaacagctctagaggatcctctcaacacaacatatacaaaacaaacgaatctcaagcaatcaagcattctacttctattgcagcaatttaaatcatttcttttaaagcaaaagcaattttctgaaaattttcaccatttacgaacgatagtaatttctactaagtgtagatgagacggagctcagtctgaccgcggcgtctcttaatttctactaagtgtagatcgaatttccccgatcgttcaaacatttggcaataaagtttcttaagattgaatcctgttgccggtcttgcgatgattatcatataatttctgttgaattacgttaagcatgtaataattaacatgtaatgcatgacgttatttatgagatgggtttttatgattagagtcccgcaattatacatttaatacgcgatagaaaacaaaatatagcgcgcaaactaggataaattatcgcgcgcggtgtcatctatgttactagatcgctcgacgcggccgccatggcctctagtggatcaggtgtcgttcggctgcggcgagcggtatcagctcactcaaaggcggtaatacggttatccacagaatcaggggataacgcaggaaagaacatgtgagcaaaaggccagcaaaaggccaggaaccgtaaaaaggccgcgttgctggcgtttttccataggctccgcccccctgacgagcatcacaaaaatcgacgctcaagtcagaggtggcgaaacccgacaggactataaagataccaggcgtttccccctggaagctccctcgtgcgctctcctgttccgaccctgccgcttaccggatacctgtccgcctttctcccttcgggaagcgtggcgctttctcatagctcacgctgtaggtatctcagttcggtgtaggtcgttcgctccaagctgggctgtgtgcacgaaccccccgttcagcccgaccgctgcgccttatccggtaactatcgtcttgagtccaacccggtaagacacgacttatcgccactggcagcagccactggtaacaggattagcagagcgaggtatgtaggcggtgctacagagttcttgaagtggtggcctaactacggctacactagaaggacagtatttggtatctgcgctctgctgaagccagttaccttcggaaaaagagttggtagctcttgatccggcaaacaaaccaccgctggtagcggtggtttttttgtttgcaagcagcagattacgcgcagaaaaaaaggatctcaagaagatcctttgatcttttctacggggtctgacgctcagtggaacgaaaactcacgttaagggattttggtcatgagattatcaaaaaggatcttcacctagatccttttaaattaaaaatgaagttttaaatcaatctaaagtatatatgagtaaacttggtctgacagttaccaatgcttaatcagtgaggcacctatctcagcgatctgtctatttcgttcatccatagttgcctgactccccgtcgtgtagataactacgatacgggagggcttaccatctggccccagtgctgcaatgataccgcgagacccacgctcaccggctccagatttatcagcaataaaccagccagccggaagggccgagcgcagaagtggtcctgcaactttatccgcctccatccagtctattaattgttgccgggaagctagagtaagtagttcgccagttaatagtttgcgcaacgttgttgccattgctacaggcatcgtggtgtcacgctcgtcgtttggtatggcttcattcagctccggttcccaacgatcaaggcgagttacatgatcccccatgttgtgcaaaaaagcggttagctccttcggtcctccgatcgttgtcagaagtaagttggccgcagtgttatcactcatggttatggcagcactgcataattctcttactgtcatgccatccgtaagatgcttttctgtgactggtgagtactcaaccaagtcattctgagaatagtgtatgcggcgaccgagttgctcttgcccggcgtcaatacgggataataccgcgccacatagcagaactttaaaagtgctcatcattggaaaacgttcttcggggcgaaaactctcaaggatcttaccgctgttgagatccagttcgatgtaacccactcgtgcacccaactgatcttcagcatcttttactttcaccagcgtttctgggtgagcaaaaacaggaaggcaaaatgccgcaaaaaagggaataagggcgacacggaaatgttgaatactcatactcttcctttttcaatattattgaagcatttatcagggttattgtctcatgagcggatacatatttgaatgtatttagaaaaataaacaaataggggttccgcgcacatttccccgaaaagtgccac

SEQ ID NO: 35 - DNA, 10434 bp, synthetic construct
  misc_feature 1..10434: note = pGEP372 LbCpf1 RR construct
  source 1..10434: mol_type = other DNA
actgctgcagtgcagcgtgacccggtcgtgcccctctctagagataatgagcattgcatgtctaagttataaaaaattaccacatattttttttgtcacacttgtttgaagtgcagtttatctatctttatacatatatttaaactttactctacgaataatataatctatagtactacaataatatcagtgttttagagaatcatataaatgaacagttagacatggtctaaaggacaattgagtattttgacaacaggactctacagttttatctttttagtgtgcatgtgttctcctttttttttgcaaatagcttcacctatataatacttcatccattttattagtacatccatttagggtttagggttaatggtttttatagactaatttttttagtacatctattttattctattttagcctctaaattaagaaaactaaaactctattttagtttttttatttaataatttagatataaaatagaataaaataaagtgactaaaaattaaacaaataccctttaagaaattaaaaaaactaaggaaacatttttcttgtttcgagtagataatgccagcctgttaaacgccgtcgatcgacgagtctaacggacaccaaccagcgaaccagcagcgtcgcgtcgggccaagcgaagcagacggcacggcatctctgtcgctgcctctggacccctctcgagagttccgctccaccgttggacttgctccgctgtcggcatccagaaattgcgtggcggagcggcagacgtgagccggcacggcaggcggcctcctcctcctctcacggcaccggcagctacgggggattcctttcccaccgctccttcgctttcccttcctcgcccgccgtaataaatagacaccccctccacaccctctttccccaacctcgtgttgttcggagcgcacacacacacaaccagatctcccccaaatccacccgtcggcacctccgcttcaaggtacgccgctcgtcctccccccccccccctctctaccttctctagatcggcgttccggtccatggttagggcccggtagttctacttctgttcatgtttgtgttagatccgtgtttgtgttagatccgtgctgctagcgttcgtacacggatgcgacctgtacgtcagacacgttctgattgctaacttgccagtgtttctctttggggaatcctgggatggctctagccgttccgcagacgggatcgatctaggataggtatacatgttgatgtgggttttactgatgcatatacatgatggcatatgcagcatctattcatatgctctaaccttgagtacctatctattataataaacaagtatgttttataattattttgatcttgatatacttggatgatggcatatgcagcagctatatgtggatttttttagccctgccttcatacgctatttatttgcttggtactgtttcttttgtcgatgctcaccctgttgtttggtgttacttctgcaggtcgaagcttgaagcaaacatggcatctagcatggcaccaaagaaaaaaaggaaagtttccaaacttgaaaaatttacaaactgctactccctttccaagacgcttaggtttaaagcgatccccgttggcaagacccaagagaatatcgataacaaaagacttctggtcgaagatgaaaaaagggccgaagactacaagggggtcaagaagttgctcgatcgctattatctttcctttatcaacgatgtgcttcattcaatcaaactgaagaacttgaataactacattagccttttcagaaagaaaacgaggactgaaaaggagaacaaggaacttgagaatcttgaaataaaccttcgcaaagaaattgcaaaagccttcaaggggaacgaaggatataaatctcttttcaaaaaagacattatagaaacaattttgcctgagtttcttgacgacaaggatgaaattgcgctcgtcaatagctttaacggatttacaactgccttcacagggttcttcgacaatagggagaatatgtttagcgaggaggcaaaaagcacatccatcgcattcagatgcatcaatgaaaatcttacccggtacatatcgaatatggacatatttgaaaaagtggatgcaatattcgataagcacgaagtccaggagataaaggaaaagatactgaatagcgactatgatgtcgaagattttttcgaaggtgagttcttcaactttgtcctgactcaagaaggcattgatgtctataatgcaataattggaggttttgtgactgagtctggcgagaagataaagggcttgaacgagtatatcaatctctacaaccagaagactaagcaaaagttgcctaaatttaaaccgctttacaagcaagttttgagcgaccgggaaagcctttccttttacggtgaaggatacacgagcgatgaagaagtcctcgaagtcttccgcaacacactcaacaagaactcagaaatcttttcctcaattaaaaaattggagaagcttttcaagaacttcgatgaatactcttcggcggggatttttgtgaagaacggcccggcaatttccacaatatctaaagacattttcggagaatggaacgtgataagagacaagtggaatgcggagtatgatgacatacacctgaagaagaaggcagttgtgactgaaaaatacgaagatgacaggagaaaaagctttaaaaagatcgggtccttttcactggaacagctgcaggagtatgccgacgccgatctttcggttgtcgaaaagctcaaagaaataattatccagaaggtcgatgaaatctacaaggtgtacggctcaagcgagaagctctttgatgctgacttcgtgttggagaagtctcttaaaaaaaacgacgcagtcgtcgcgataatgaaagatttgctggattcagtgaaatccttcgagaattatatcaaagccttcttcggcgaggggaaggagacaaacagggatgagtccttctatggagacttcgttctggcttacgacatccttcttaaggtcgaccacatctatgacgcaattcggaactatgtgacgcagaagccgtattcgaaagataagttcaagctctatttccaaaaccctcaatttatgcgtgggtgggataaagacaaagagaccgattaccgggcaacaattttgcggtacgggtctaaatattacctcgctataatggataagaaatacgctaaatgtctccagaaaattgacaaagatgacgtcaacggcaattatgaaaaaatcaattataaactccttcctggcccaaataaaatgctcccgagggtgtttttttccaaaaagtggatggcctattataatccatcagaggatattcagaaaatctataaaaatgggacctttaagaagggtgacatgtttaacctgaacgattgccacaagcttatagattttttcaaagactctattagccgctatcccaaatggtctaatgcttatgatttcaacttctctgaaactgaaaagtacaaagatattgcaggattctaccgcgaagttgaagaacaaggttataaggtttcctttgagtctgcgtccaagaaagaggtcgataagttggtcgaagaagggaaattgtatatgtttcaaatttacaataaagacttttccgacaagtcccatggtacacctaatctgcataccatgtacttcaaactgctgttcgatgagaataatcacggtcagattcgcctgagcggaggggcggaactcttcatgaggagagcatcgttgaaaaaagaggagctcgtcgtgcatccggctaacagccccattgctaacaagaatccggataatccaaagaagactactaccctctcctatgacgtctataaggataagagattctctgaggaccagtacgagttgcacatccctattgcgataaataaatgccctaagaacatctttaaaatcaatactgaggtcagagtcctgcttaagcacgacgacaacccgtatgtgatcgggattgataggggtgaaaggaacttgctttatattgtggttgtcgatggaaaaggtaatatagtggaacaatactctctgaatgaaattatcaacaacttcaatggcattaggatcaagaccgactatcattctctgttggacaagaaagagaaagagcgcttcgaggcacggcaaaactggacgtctattgagaacatcaaggagcttaaggctggttacatttctcaggttgtgcacaaaatttgcgaactggtcgagaaatatgatgccgttatcgcacttgaagatctcaacagcggatttaagaattctcgggtgaaagtcgaaaaacaggtgtatcaaaaattcgaaaagatgctgatcgacaagctcaattatatggttgataaaaagagcaacccatgcgccacggggggtgcgcttaagggctatcagattacgaacaaatttgaatccttcaagtcaatgtcgacgcaaaatgggtttatattctatataccggcgtggcttacatctaaaatagatcctagcactgggttcgtgaacctgctgaaaaccaagtacacttcaatcgcagattctaaaaaatttataagcagcttcgacagaatcatgtatgtgcccgaggaagacctcttcgagtttgcccttgattacaaaaatttctcaagaacggatgcagactacataaagaagtggaagctgtactcttatgggaaccggattcggatattcagaaatccgaaaaaaaacaatgtctttgattgggaggaagtttgtcttacctctgcttacaaagagctgttcaataaatatggcattaattaccagcaaggtgatatccgggcgctcctttgcgaacagtctgacaaagctttctattcttcatttatggcgctcatgtcattgatgctgcagatgaggaatagcattacggggaggactgatgttgactttctgatctcgcccgtgaaaaattctgatggaatcttctacgattccaggaattatgaggcccaggaaaatgctatccttcccaagaacgcagacgcaaatggcgcgtacaatatagctcgcaaggttttgtgggctataggccaattcaagaaagccgaagacgaaaagctggacaaagttaagattgctatatctaacaaagagtggcttgagtatgcgcaaacatctgttaaacacaaacgccccgcggctacaaagaaggctggccaggcaaagaagaagaagtgagtcgaccgatcgttcaaacatttggcaataaagtttcttaagattgaatcctgttgccggtcttgcgatgattatcatataatttctgttgaattacgttaagcatgtaataattaacatgtaatgcatgacgttatttatgagatgggtttttatgattagagtcccgcaattatacatttaatacgcgatagaaaacaaaatatagcgcgcaaactaggataaattatcgcgcgcggtgtcatctatgttactagatcgatcccgggatatcgcggccgcgtcgttcggctgcggcgagcggtatcagctcactcaaaggcggtaatacggttatccacagaatcaggggataacgcaggaaagaacatgtgagcaaaaggccagcaaaaggccaggaaccgtaaaaaggccgcgttgctggcgtttttccataggctccgcccccctgacgagcatcacaaaaatcgacgctcaagtcagaggtggcgaaacccgacaggactataaagataccaggcgtttccccctggaagctccctcgtgcgctctcctgttccgaccctgccgcttaccggatacctgtccgcctttctcccttcgggaagcgtggcgctttctcatagctcacgctgtaggtatctcagttcggtgtaggtcgttcgctccaagctgggctgtgtgcacgaaccccccgttcagcccgaccgctgcgccttatccggtaactatcgtcttgagtccaacccggtaagacacgacttatcgccactggcagcagccactggtaacaggattagcagagcgaggtatgtaggcggtgctacagagttcttgaagtggtggcctaactacggctacactagaaggacagtatttggtatctgcgctctgctgaagccagttaccttcggaaaaagagttggtagctcttgatccggcaaacaaaccaccgctggtagcggtggtttttttgtttgcaagcagcagattacgcgcagaaaaaaaggatctcaagaagatcctttgatcttttctacggggtctgacgctcagtggaacgaaaactcacgttaagggattttggtcatgagattatcaaaaaggatcttcacctagatccttttaaattaaaaatgaagttttaaatcaatctaaagtatatatgagtaaacttggtctgacagttaccaatgcttaatcagtgaggcacctatctcagcgatctgtctatttcgttcatccatagttgcctgactccccgtcgtgtagataactacgatacgggagggcttaccatctggccccagtgctgcaatgataccgcgagacccacgctcaccggctccagatttatcagcaataaaccagccagccggaagggccgagcgcagaagtggtcctgcaactttatccgcctccatccagtctattaattgttgccgggaagctagagtaagtagttcgccagttaatagtttgcgcaacgttgttgccattgctacaggcatcgtggtgtcacgctcgtcgtttggtatggcttcattcagctccggttcccaacgatcaaggcgagttacatgatcccccatgttgtgcaaaaaagcggttagctccttcggtcctccgatcgttgtcagaagtaagttggccgcagtgttatcactcatggttatggcagcactgcataattctcttactgtcatgccatccgtaagatgcttttctgtgactggtgagtactcaaccaagtcattctgagaatagtgtatgcggcgaccgagttgctcttgcccggcgtcaatacgggataataccgcgccacatagcagaactttaaaagtgctcatcattggaaaacgttcttcggggcgaaaactctcaaggatcttaccgctgttgagatccagttcgatgtaacccactcgtgcacccaactgatcttcagcatcttttactttcaccagcgtttctgggtgagcaaaaacaggaaggcaaaatgccgcaaaaaagggaataagggcgacacggaaatgttgaatactcatactcttcctttttcaatattattgaagcatttatcagggttattgtctcatgagcggatacatatttgaatgtatttagaaaaataaacaaataggggttccgcgcacatttccccgaaaagtgccacctgacgcgccctgtagcggcacgtctaattcgggggatctggattttagtactggattttggttttaggaattagaaattttattgatagaagtattttacaaatacaaatacatactaagggtttcttatatgctcaacacatgagcgaaaccctataggaaccctaattcccttatctgggaactactcacacattattatggagaaactcgagcttgtcgatcgacatgatcagggagctctagattatttgtatagttcatccatgcccattacgtcggtaaatgccttctgccactccttgaagttaagttcggtcttggaatgtttcaactcagtcttacggaacacgtacatgggttggttcttaaggtagttagcggccattggtttagcgaatgtgtaggtagtcctggctgtagagcgatatctcttgccattgcctgtggtgtaagaccatttgaaggtactaatgatggtcttgtcgttagggtaggttttcttggaccggcaccaatcagcggcagttaaggagttggtcatgacaggtccatcagcaggaaagcctgtccccttcacttgggcttctcctttgatgtggctcccttcgtaagtgtaacggtagttgacggtgagcgaagcaccgtcctcaaactgcattgtcctgtggacttggtatccggagccatcaaccatggctgcttggaatggactcattccgtcagggtatggaaggtattgatggaatccgtagccaatgtgtggcaccagaatccatggagaaaactgaagatcacctttggtgctcttgaggttcagctcttcgtatccgtcattagggttcccagtgccttgtccgaccatatcgaagtcaacgccgttgatggaaccgaagatgtgaagctcatgtgtggctggaagcgaagccatgttatcttcttctcctttactcacggaggacgccatggtggcgggatcgcgccctatcgttcgtaaatggtgaaaattttcagaaaattgcttttgctttaaaagaaatgatttaaattgctgcaatagaagtagaatgcttgattgcttgagattcgtttgttttgtatatgttgtgttgagaggatcctcaagcttcgacctgcagaagtaacaccaaacaacagggtgagcatcgacaaaagaaacagtaccaagcaaataaatagcgtatgaaggcagggctaaaaaaatccacatatagctgctgcatatgccatcatccaagtatatcaagatcaaaataattataaaacatacttgtttattataatagataggtactcaaggttagagcatatgaatagatgctgcatatgccatcatgtatatgcatcagtaaaacccacatcaacatgtatacctatcctagatcgatatttccatccatcttaaactcgtaactatgaagatgtatgacacacacatacagttccaaaattaataaatacaccaggtagtttgaaacagtattctactccgatctagaacgaatgaacgaccgcccaaccacaccacatcatcacaaccaagcgaacaaaagcatctctgtatatgcatcagtaaaacccgcatcaacatgtatacctatcctagatcgatatttccatccatcatcttcaattcgtaactatgaatatgtatggcacacacatacagatccaaaattaataaatccaccaggtagtttgaaacagaattctactccgatctagaacgaccgcccaaccagaccacatcatcacaaccaagacaaaaaaaagcatgaaaagatgacccgacaaacaagtgcacggcatatattgaaataaaggaaaagggcaaaccaaaccctatgcaacgaaacaaaaaaaatcatgaaatcgatcccgtctgcggaacggctagagccatcccaggattccccaaagagaaacactggcaagttagcaatcagaacgtgtctgacgtacaggtcgcatccgtgtacgaacgctagcagcacggatctaacacaaacacggatctaacacaaacatgaacagaagtagaactaccgggccctaaccatggaccggaacgccgatctagagaaggtagagagggggggggaggacgagcggcgtaccttgaagcggaggtgccgacgggtggatttgggggagatccactagttctagagcggccgccaccgcggtggaattctcgaggtcctctccaaatgaaatgaacttccttatatagaggaagggtcttgcgaaggatagtgggattgtgcgtcatcccttacgtcagtggagatatcacatcaatccacttgctttgaagacgtggttggaacgtcttctttttccacgatgctcctcgtgggtgggggtccatctttgggaccactgtcggcagaggcatcttgaacgatagcctttcctttatcgcaatgatggcatttgtaggtgccaccttccttttctactgtccttttgatcaagtgaccgatagctgggcaatggaatccgaggaggtttcccgatattaccctttgttgaaaagtctcaatagccctttggtcttctgagactgtatctttgatattcttggagtagacgagagtgtcgtgctccaccatgttatcacatcaattcacttgctttgaagacgtggttggaacgtcttctttttccacgatgctcctcgtgggtgggggtccatctttgggaccactgtcggcagaggcatcttgaacgatagcctttcctttatcgcaatgatggcatttgtaggtgccaccttccttttctactgtccttttgatcaagtgacagatagctgggcaatggaatccgaggaggtttcccgatattaccctttgttgaaaagtctcaatagccctttggtcttctgagacttgcaggcaagcaagcatgaatgcctgggcgcgccgatatc

SEQ ID NO: 36 - DNA, 10434 bp, synthetic construct
  misc_feature 1..10434: note = pGEP373 LbCpf1 RVR construct
  source 1..10434: mol_type = other DNA
actgctgcagtgcagcgtgacccggtcgtgcccctctctagagataatgagcattgcatgtctaagttataaaaaattaccacatattttttttgtcacacttgtttgaagtgcagtttatctatctttatacatatatttaaactttactctacgaataatataatctatagtactacaataatatcagtgttttagagaatcatataaatgaacagttagacatggtctaaaggacaattgagtattttgacaacaggactctacagttttatctttttagtgtgcatgtgttctcctttttttttgcaaatagcttcacctatataatacttcatccattttattagtacatccatttagggtttagggttaatggtttttatagactaatttttttagtacatctattttattctattttagcctctaaattaagaaaactaaaactctattttagtttttttatttaataatttagatataaaatagaataaaataaagtgactaaaaattaaacaaataccctttaagaaattaaaaaaactaaggaaacatttttcttgtttcgagtagataatgccagcctgttaaacgccgtcgatcgacgagtctaacggacaccaaccagcgaaccagcagcgtcgcgtcgggccaagcgaagcagacggcacggcatctctgtcgctgcctctggacccctctcgagagttccgctccaccgttggacttgctccgctgtcggcatccagaaattgcgtggcggagcggcagacgtgagccggcacggcaggcggcctcctcctcctctcacggcaccggcagctacgggggattcctttcccaccgctccttcgctttcccttcctcgcccgccgtaataaatagacaccccctccacaccctctttccccaacctcgtgttgttcggagcgcacacacacacaaccagatctcccccaaatccacccgtcggcacctccgcttcaaggtacgccgctcgtcctccccccccccccctctctaccttctctagatcggcgttccggtccatggttagggcccggtagttctacttctgttcatgtttgtgttagatccgtgtttgtgttagatccgtgctgctagcgttcgtacacggatgcgacctgtacgtcagacacgttctgattgctaacttgccagtgtttctctttggggaatcctgggatggctctagccgttccgcagacgggatcgatctaggataggtatacatgttgatgtgggttttactgatgcatatacatgatggcatatgcagcatctattcatatgctctaaccttgagtacctatctattataataaacaagtatgttttataattattttgatcttgatatacttggatgatggcatatgcagcagctatatgtggatttttttagccctgccttcatacgctatttatttgcttggtactgtttcttttgtcgatgctcaccctgttgtttggtgttacttctgcaggtcgaagcttgaagcaaacatggcatctagcatggcaccaaagaaaaaaaggaaagtttccaaacttgaaaaatttacaaactgctactccctttccaagacgcttaggtttaaagcgatccccgttggcaagacccaagagaatatcgataacaaaagacttctggtcgaagatgaaaaaagggccgaagactacaagggggtcaagaagttgctcgatcgctattatctttcctttatcaacgatgtgcttcattcaatcaaactgaagaacttgaataactacattagccttttcagaaagaaaacgaggactgaaaaggagaacaaggaacttgagaatcttgaaataaaccttcgcaaagaaattgcaaaagccttcaaggggaacgaaggatataaatctcttttcaaaaaagacattatagaaacaattttgcctgagtttcttgacgacaaggatgaaattgcgctcgtcaatagctttaacggatttacaactgccttcacagggttcttcgacaatagggagaatatgtttagcgaggaggcaaaaagcacatccatcgcattcagatgcatcaatgaaaatcttacccggtacatatcgaatatggacatatttgaaaaagtggatgcaatattcgataagcacgaagtccaggagataaaggaaaagatactgaatagcgactatgatgtcgaagattttttcgaaggtgagttcttcaactttgtcctgactcaagaaggcattgatgtctataatgcaataattggaggttttgtgactgagtctggcgagaagataaagggcttgaacgagtatatcaatctctacaaccagaagactaagcaaaagttgcctaaatttaaaccgctttacaagcaagttttgagcgaccgggaaagcctttccttttacggtgaaggatacacgagcgatgaagaagtcctcgaagtcttccgcaacacactcaacaagaactcagaaatcttttcctcaattaaaaaattggagaagcttttcaagaacttcgatgaatactcttcggcggggatttttgtgaagaacggcccggcaatttccacaatatctaaagacattttcggagaatggaacgtgataagagacaagtggaatgcggagtatgatgacatacacctgaagaagaaggcagttgtgactgaaaaatacgaagatgacaggagaaaaagctttaaaaagatcgggtccttttcactggaacagctgcaggagtatgccgacgccgatctttcggttgtcgaaaagctcaaagaaataattatccagaaggtcgatgaaatctacaaggtgtacggctcaagcgagaagctctttgatgctgacttcgtgttggagaagtctcttaaaaaaaacgacgcagtcgtcgcgataatgaaagatttgctggattcagtgaaatccttcgagaattatatcaaagccttcttcggcgaggggaaggagacaaacagggatgagtccttctatggagacttcgttctggcttacgacatccttcttaaggtcgaccacatctatgacgcaattcggaactatgtgacgcagaagccgtattcgaaagataagttcaagctctatttccaaaaccctcaatttatgcgtgggtgggataaagacgtagagaccgatcgccgggcaacaattttgcggtacgggtctaaatattacctcgctataatggataagaaatacgctaaatgtctccagaaaattgacaaagatgacgtcaacggcaattatgaaaaaatcaattataaactccttcctggcccaaataaaatgctcccgaaggtgtttttttccaaaaagtggatggcctattataatccatcagaggatattcagaaaatctataaaaatgggacctttaagaagggtgacatgtttaacctgaacgattgccacaagcttatagattttttcaaagactctattagccgctatcccaaatggtctaatgcttatgatttcaacttctctgaaactgaaaagtacaaagatattgcaggattctaccgcgaagttgaagaacaaggttataaggtttcctttgagtctgcgtccaagaaagaggtcgataagttggtcgaagaagggaaattgtatatgtttcaaatttacaataaagacttttccgacaagtcccatggtacacctaatctgcataccatgtacttcaaactgctgttcgatgagaataatcacggtcagattcgcctgagcggaggggcggaactcttcatgaggagagcatcgttgaaaaaagaggagctcgtcgtgcatccggctaacagccccattgctaacaagaatccggataatccaaagaagactactaccctctcctatgacgtctataaggataagagattctctgaggaccagtacgagttgcacatccctattgcgataaataaatgccctaagaacatctttaaaatcaatactgaggtcagagtcctgcttaagcacgacgacaacccgtatgtgatcgggattgataggggtgaaaggaacttgctttatattgtggttgtcgatggaaaaggtaatatagtggaacaatactctctgaatgaaattatcaacaacttcaatggcattaggatcaagaccgactatcattctctgttggacaagaaagagaaagagcgcttcgaggcacggcaaaactggacgtctattgagaacatcaaggagcttaaggctggttacatttctcaggttgtgcacaaaatttgcgaactggtcgagaaatatgatgccgttatcgcacttgaagatctcaacagcggatttaagaattctcgggtgaaagtcgaaaaacaggtgtatcaaaaattcgaaaagatgctgatcgacaagctcaattatatggttgataaaaagagcaacccatgcgccacggggggtgcgcttaagggctatcagattacgaacaaatttgaatccttcaagtcaatgtcgacgcaaaatgggtttatattctatataccggcgtggcttacatctaaaatagatcctagcactgggttcgtgaacctgctgaaaaccaagtacacttcaatcgcagattctaaaaaatttataagcagcttcgacagaatcatgtatgtgcccgaggaagacctcttcgagtttgcccttgattacaaaaatttctcaagaacggatgcagactacataaagaagtggaagctgtactcttatgggaaccggattcggatattcagaaatccgaaaaaaaacaatgtctttgattgggaggaagtttgtcttacctctgcttacaaagagctgttcaataaatatggcattaattaccagcaaggtgatatccgggcgctcctttgcgaacagtctgacaaagctttctattcttcatttatggcgctcatgtcattgatgctgcagatgaggaatagcattacggggaggactgatgttgactttctgatctcgcccgtgaaaaattctgatggaatcttctacgattccaggaattatgaggcccaggaaaatgctatccttcccaagaacgcagacgcaaatggcgcgtacaatatagctcgcaaggttttgtgggctataggccaattcaagaaagccgaagacgaaaagctggacaaagttaagattgctatatctaacaaagagtggcttgagtatgcgcaaacatctgttaaacacaaacgccccgcggctacaaagaaggctggccaggcaaagaagaagaagtgagtcgaccgatcgttcaaacatttggcaataaagtttcttaagattgaatcctgttgccggtcttgcgatgattatcatataatttctgttgaattacgttaagcatgtaataattaacatgtaatgcatgacgttatttatgagatgggtttttatgattagagtcccgcaattatacatttaatacgcgatagaaaacaaaatatagcgcgcaaactaggataaattatcgcgcgcggtgtcatctatgttactagatcgatcccgggatatcgcggccgcgtcgttcggctgcggcgagcggtatcagctcactcaaaggcggtaatacggttatccacagaatcaggggataacgcaggaaagaacatgtgagcaaaaggccagcaaaaggccaggaaccgtaaaaaggccgcgttgctggcgtttttccataggctccgcccccctgacgagcatcacaaaaatcgacgctcaagtcagaggtggcgaaacccgacaggactataaagataccaggcgtttccccctggaagctccctcgtgcgctctcctgttccgaccctgccgcttaccggatacctgtccgcctttctcccttcgggaagcgtggcgctttctcatagctcacgctgtaggtatctcagttcggtgtaggtcgttcgctccaagctgggctgtgtgcacgaaccccccgttcagcccgaccgctgcgccttatccggtaactatcgtcttgagtccaacccggtaagacacgacttatcgccactggcagcagccactggtaacaggattagcagagcgaggtatgtaggcggtgctacagagttcttgaagtggtggcctaactacggctacactagaaggacagtatttggtatctgcgctctgctgaagccagttaccttcggaaaaagagttggtagctcttgatccggcaaacaaaccaccgctggtagcggtggtttttttgtttgcaagcagcagattacgcgcagaaaaaaaggatctcaagaagatcctttgatcttttctacggggtctgacgctcagtggaacgaaaactcacgttaagggattttggtcatgagattatcaaaaaggatcttcacctagatccttttaaattaaaaatgaagttttaaatcaatctaaagtatatatgagtaaacttggtctgacagttaccaatgcttaatcagtgaggcacctatctcagcgatctgtctatttcgttcatccatagttgcctgactccccgtcgtgtagataactacgatacgggagggcttaccatctggccccagtgctgcaatgataccgcgagacccacgctcaccggctccagatttatcagcaataaaccagccagccggaagggccgagcgcagaagtggtcctgcaactttatccgcctccatccagtctattaattgttgccgggaagctagagtaagtagttcgccagttaatagtttgcgcaacgttgttgccattgctacaggcatcgtggtgtcacgctcgtcgtttggtatggcttcattcagctccggttcccaacgatcaaggcgagttacatgatcccccatgttgtgcaaaaaagcggttagctccttcggtcctccgatcgttgtcagaagtaagttggccgcagtgttatcactcatggttatggcagcactgcataattctcttactgtcatgccatccgtaagatgcttttctgtgactggtgagtactcaaccaagtcattctgagaatagtgtatgcggcgaccgagttgctcttgcccggcgtcaatacgggataataccgcgccacatagcagaactttaaaagtgctcatcattggaaaacgttcttcggggcgaaaactctcaaggatcttaccgctgttgagatccagttcgatgtaacccactcgtgcacccaactgatcttcagcatcttttactttcaccagcgtttctgggtgagcaaaaacaggaaggcaaaatgccgcaaaaaagggaataagggcgacacggaaatgttgaatactcatactcttcctttttcaatattattgaagcatttatcagggttattgtctcatgagcggatacatatttgaatgtatttagaaaaataaacaaataggggttccgcgcacatttccccgaaaagtgccacctgacgcgccctgtagcggcacgtctaattcgggggatctggattttagtactggattttggttttaggaattagaaattttattgatagaagtattttacaaatacaaatacatactaagggtttcttatatgctcaacacatgagcgaaaccctataggaaccctaattcccttatctgggaactactcacacattattatggagaaactcgagcttgtcgatcgacatgatcagggagctctagattatttgtatagttcatccatgcccattacgtcggtaaatgccttctgccactccttgaagttaagttcggtcttggaatgtttcaactcagtcttacggaacacgtacatgggttggttcttaaggtagttagcggccattggtttagcgaatgtgtaggtagtcctggctgtagagcgatatctcttgccattgcctgtggtgtaagaccatttgaaggtactaatgatggtcttgtcgttagggtaggttttcttggaccggcaccaatcagcggcagttaaggagttggtcatgacaggtccatcagcaggaaagcctgtccccttcacttgggcttctcctttgatgtggctcccttcgtaagtgtaacggtagttgacggtgagcgaagcaccgtcctcaaactgcattgtcctgtggacttggtatccggagccatcaaccatggctgcttggaatggactcattccgtcagggtatggaaggtattgatggaatccgtagccaatgtgtggcaccagaatccatggagaaaactgaagatcacctttggtgctcttgaggttcagctcttcgtatccgtcattagggttcccagtgccttgtccgaccatatcgaagtcaacgccgttgatggaaccgaagatgtgaagctcatgtgtggctggaagcgaagccatgttatcttcttctcctttactcacggaggacgccatggtggcgggatcgcgccctatcgttcgtaaatggtgaaaattttcagaaaattgcttttgctttaaaagaaatgatttaaattgctgcaatagaagtagaatgcttgattgcttgagattcgtttgttttgtatatgttgtgttgagaggatcctcaagcttcgacctgcagaagtaacaccaaacaacagggtgagcatcgacaaaagaaacagtaccaagcaaataaatagcgtatgaaggcagggctaaaaaaatccacatatagctgctgcatatgccatcatccaagtatatcaagatcaaaataattataaaacatacttgtttattataatagataggtactcaaggttagagcatatgaatagatgctgcatatgccatcatgtatatgcatcagtaaaacccacatcaacatgtatacctatcctagatcgatatttccatccatcttaaactcgtaactatgaagatgtatgacacacacatacagttccaaaattaataaatacaccaggtagtttgaaacagtattctactccgatctagaacgaatgaacgaccgcccaaccacaccacatcatcacaaccaagcgaacaaaagcatctctgtatatgcatcagtaaaacccgcatcaacatgtatacctatcctagatcgatatttccatccatcatcttcaattcgtaactatgaatatgtatggcacacacatacagatccaaaattaataaatccaccaggtagtttgaaacagaattctactccgatctagaacgaccgcccaaccagaccacatcatcacaaccaagacaaaaaaaagcatgaaaagatgacccgacaaacaagtgcacggcatatattgaaataaaggaaaagggcaaaccaaaccctatgcaacgaaacaaaaaaaatcatgaaatcgatcccgtctgcggaacggctagagccatcccaggattccccaaagagaaacactggcaagttagcaatcagaacgtgtctgacgtacaggtcgcatccgtgtacgaacgctagcagcacggatctaacacaaacacggatctaacacaaacatgaacagaagtagaactaccgggccctaaccatggaccggaacgccgatctagagaaggtagagagggggggggaggacgagcggcgtaccttgaagcggaggtgccgacgggtggatttgggggagatccactagttctagagcggccgccaccgcggtggaattctcgaggtcctctccaaatgaaatgaacttccttatatagaggaagggtcttgcgaaggatagtgggattgtgcgtcatcccttacgtcagtggagatatcacatcaatccacttgctttgaagacgtggttggaacgtcttctttttccacgatgctcctcgtgggtgggggtccatctttgggaccactgtcggcagaggcatcttgaacgatagcctttcctttatcgcaatgatggcatttgtaggtgccaccttccttttctactgtccttttgatcaagtgaccgatagctgggcaatggaatccgaggaggtttcccgatattaccctttgttgaaaagtctcaatagccctttggtcttctgagactgtatctttgatattcttggagtagacgagagtgtcgtgctccaccatgttatcacatcaattcacttgctttgaagacgtggttggaacgtcttctttttccacgatgctcctcgtgggtgggggtccatctttgggaccactgtcggcagaggcatcttgaacgatagcctttcctttatcgcaatgatggcatttgtaggtgccaccttccttttctactgtccttttgatcaagtgacagatagctgggcaatggaatccgaggaggtttcccgatattaccctttgttgaaaagtctcaatagccctttggtcttctgagacttgcaggcaagcaagcatgaatgcctgggcgcgccgatatc

SEQ ID NO: 37 - DNA, 10432 bp, synthetic construct
  misc_feature 1..10432: note = pGEP315 Corn strategy LbCpf1 vector
  source 1..10432: mol_type = other DNA
actgctgcagtgcagcgtgacccggtcgtgcccctctctagagataatgagcattgcatgtctaagttataaaaaattaccacatattttttttgtcacacttgtttgaagtgcagtttatctatctttatacatatatttaaactttactctacgaataatataatctatagtactacaataatatcagtgttttagagaatcatataaatgaacagttagacatggtctaaaggacaattgagtattttgacaacaggactctacagttttatctttttagtgtgcatgtgttctcctttttttttgcaaatagcttcacctatataatacttcatccattttattagtacatccatttagggtttagggttaatggtttttatagactaatttttttagtacatctattttattctattttagcctctaaattaagaaaactaaaactctattttagtttttttatttaataatttagatataaaatagaataaaataaagtgactaaaaattaaacaaataccctttaagaaattaaaaaaactaaggaaacatttttcttgtttcgagtagataatgccagcctgttaaacgccgtcgatcgacgagtctaacggacaccaaccagcgaaccagcagcgtcgcgtcgggccaagcgaagcagacggcacggcatctctgtcgctgcctctggacccctctcgagagttccgctccaccgttggacttgctccgctgtcggcatccagaaattgcgtggcggagcggcagacgtgagccggcacggcaggcggcctcctcctcctctcacggcaccggcagctacgggggattcctttcccaccgctccttcgctttcccttcctcgcccgccgtaataaatagacaccccctccacaccctctttccccaacctcgtgttgttcggagcgcacacacacacaaccagatctcccccaaatccacccgtcggcacctccgcttcaaggtacgccgctcgtcctcccccccccctctctaccttctctagatcggcgttccggtccatggttagggcccggtagttctacttctgttcatgtttgtgttagatccgtgtttgtgttagatccgtgctgctagcgttcgtacacggatgcgacctgtacgtcagacacgttctgattgctaacttgccagtgtttctctttggggaatcctgggatggctctagccgttccgcagacgggatcgatctaggataggtatacatgttgatgtgggttttactgatgcatatacatgatggcatatgcagcatctattcatatgctctaaccttgagtacctatctattataataaacaagtatgttttataattattttgatcttgatatacttggatgatggcatatgcagcagctatatgtggatttttttagccctgccttcatacgctatttatttgcttggtactgtttcttttgtcgatgctcaccctgttgtttggtgttacttctgcaggtcgaagcttgaagcaaacatggcatctagcatggcaccaaagaaaaaaaggaaagtttccaaacttgaaaaatttacaaactgctactccctttccaagacgcttaggtttaaagcgatccccgttggcaagacccaagagaatatcgataacaaaagacttctggtcgaagatgaaaaaagggccgaagactacaagggggtcaagaagttgctcgatcgctattatctttcctttatcaacgatgtgcttcattcaatcaaactgaagaacttgaataactacattagccttttcagaaagaaaacgaggactgaaaaggagaacaaggaacttgagaatcttgaaataaaccttcgcaaagaaattgcaaaagccttcaaggggaacgaaggatataaatctcttttcaaaaaagacattatagaaacaattttgcctgagtttcttgacgacaaggatgaaattgcgctcgtcaatagctttaacggatttacaactgccttcacagggttcttcgacaatagggagaatatgtttagcgaggaggcaaaaagcacatccatcgcattcagatgcatcaatgaaaatcttacccggtacatatcgaatatggacatatttgaaaaagtggatgcaatattcgataagcacgaagtccaggagataaaggaaaagatactgaatagcgactatgatgtcgaagattttttcgaaggtgagttcttcaactttgtcctgactcaagaaggcattgatgtctataatgcaataattggaggttttgtgactgagtctggcgagaagataaagggcttgaacgagtatatcaatctctacaaccagaagactaagcaaaagttgcctaaatttaaaccgctttacaagcaagttttgagcgaccgggaaagcctttccttttacggtgaaggatacacgagcgatgaagaagtcctcgaagtcttccgcaacacactcaacaagaactcagaaatcttttcctcaattaaaaaattggagaagcttttcaagaacttcgatgaatactcttcggcggggatttttgtgaagaacggcccggcaatttccacaatatctaaagacattttcggagaatggaacgtgataagagacaagtggaatgcggagtatgatgacatacacctgaagaagaaggcagttgtgactgaaaaatacgaagatgacaggagaaaaagctttaaaaagatcgggtccttttcactggaacagctgcaggagtatgccgacgccgatctttcggttgtcgaaaagctcaaagaaataattatccagaaggtcgatgaaatctacaaggtgtacggctcaagcgagaagctctttgatgctgacttcgtgttggagaagtctcttaaaaaaaacgacgcagtcgtcgcgataatgaaagatttgctggattcagtgaaatccttcgagaattatatcaaagccttcttcggcgaggggaaggagacaaacagggatgagtccttctatggagacttcgttctggcttacgacatccttcttaaggtcgaccacatctatgacgcaattcggaactatgtgacgcagaagccgtattcgaaagataagttcaagctctatttccaaaaccctcaatttatgggtgggtgggataaagacaaagagaccgattaccgggcaacaattttgcggtacgggtctaaatattacctcgctataatggataagaaatacgctaaatgtctccagaaaattgacaaagatgacgtcaacggcaattatgaaaaaatcaattataaactccttcctggcccaaataaaatgctcccgaaggtgtttttttccaaaaagtggatggcctattataatccatcagaggatattcagaaaatctataaaaatgggacctttaagaagggtgacatgtttaacctgaacgattgccacaagcttatagattttttcaaagactctattagccgctatcccaaatggtctaatgcttatgatttcaacttctctgaaactgaaaagtacaaagatattgcaggattctaccgcgaagttgaagaacaaggttataaggtttcctttgagtctgcgtccaagaaagaggtcgataagttggtcgaagaagggaaattgtatatgtttcaaatttacaataaagacttttccgacaagtcccatggtacacctaatctgcataccatgtacttcaaactgctgttcgatgagaataatcacggtcagattcgcctgagcggaggggcggaactcttcatgaggagagcatcgttgaaaaaagaggagctcgtcgtgcatccggctaacagccccattgctaacaagaatccggataatccaaagaagactactaccctctcctatgacgtctataaggataagagattctctgaggaccagtacgagttgcacatccctattgcgataaataaatgccctaagaacatctttaaaatcaatactgaggtcagagtcctgcttaagcacgacgacaacccgtatgtgatcgggattgataggggtgaaaggaacttgctttatattgtggttgtcgatggaaaaggtaatatagtggaacaatactctctgaatgaaattatcaacaacttcaatggcattaggatcaagaccgactatcattctctgttggacaagaaagagaaagagcgcttcgaggcacggcaaaactggacgtctattgagaacatcaaggagcttaaggctggttacatttctcaggttgtgcacaaaatttgcgaactggtcgagaaatatgatgccgttatcgcacttgaagatctcaacagcggatttaagaattctcgggtgaaagtcgaaaaacaggtgtatcaaaaattcgaaaagatgctgatcgacaagctcaattatatggttgataaaaagagcaacccatgcgccacggggggtgcgcttaagggctatcagattacgaacaaatttgaatccttcaagtcaatgtcgacgcaaaatgggtttatattctatataccggcgtggcttacatctaaaatagatcctagcactgggttcgtgaacctgctgaaaaccaagtacacttcaatcgcagattctaaaaaatttataagcagcttcgacagaatcatgtatgtgcccgaggaagacctcttcgagtttgcccttgattacaaaaatttctcaagaacggatgcagactacataaagaagtggaagctgtactcttatgggaaccggattcggatattcagaaatccgaaaaaaaacaatgtctttgattgggaggaagtttgtcttacctctgcttacaaagagctgttcaataaatatggcattaattaccagcaaggtgatatccgggcgctcctttgcgaacagtctgacaaagctttctattcttcatttatggcgctcatgtcattgatgctgcagatgaggaatagcattacggggaggactgatgttgactttctgatctcgcccgtgaaaaattctgatggaatcttctacgattccaggaattatgaggcccaggaaaatgctatccttcccaagaacgcagacgcaaatggcgcgtacaatatagctcgcaaggttttgtgggctataggccaattcaagaaagccgaagacgaaaagctggacaaagttaagattgctatatctaacaaagagtggcttgagtatgcgcaaacatctgttaaacacaaacgccccgcggctacaaagaaggctggccaggcaaagaagaagaagtgagtcgaccgatcgttcaaacatttggcaataaagtttcttaagattgaatcctgttgccggtcttgcgatgattatcatataatttctgttgaattacgttaagcatgtaataattaacatgtaatgcatgacgttatttatgagatgggtttttatgattagagtcccgcaattatacatttaatacgcgatagaaaacaaaatatagcgcgcaaactaggataaattatcgcgcgcggtgtcatctatgttactagatcgatcccgggatatcgcggccggtcgttcggctgcggcgagcggtatcagctcactcaaaggcggtaatacggttatccacagaatcaggggataacgcaggaaagaacatgtgagcaaaaggccagcaaaaggccaggaaccgtaaaaaggccgcgttgctggcgtttttccataggctccgcccccctgacgagcatcacaaaaatcgacgctcaagtcagaggtggcgaaacccgacaggactataaagataccaggcgtttccccctggaagctccctcgtgcgctctcctgttccgaccctgccgcttaccggatacctgtccgcctttctcccttcgggaagcgtggcgctttctcatagctcacgctgtaggtatctcagttcggtgtaggtcgttcgctccaagctgggctgtgtgcacgaaccccccgttcagcccgaccgctgcgccttatccggtaactatcgtcttgagtccaacccggtaagacacgacttatcgccactggcagcagccactggtaacaggattagcagagcgaggtatgtaggcggtgctacagagttcttgaagtggtggcctaactacggctacactagaagaacagtatttggtatctgcgctctgctgaagccagttaccttcggaaaaagagttggtagctcttgatccggcaaacaaaccaccgctggtagcggtggtttttttgtttgcaagcagcagattacgcgcagaaaaaaaggatctcaagaagatcctttgatcttttctacggggtctgacgctcagtggaacgaaaactcacgttaagggattttggtcatgagattatcaaaaaggatcttcacctagatccttttaaattaaaaatgaagttttaaatcaatctaaagtatatatgagtaaacttggtctgacagttaccaatgcttaatcagtgaggcacctatctcagcgatctgtctatttcgttcatccatagttgcctgactccccgtcgtgtagataactacgatacgggagggcttaccatctggccccagtgctgcaatgataccgcgagacccacgctcaccggctccagatttatcagcaataaaccagccagccggaagggccgagcgcagaagtggtcctgcaactttatccgcctccatccagtctattaattgttgccgggaagctagagtaagtagttcgccagttaatagtttgcgcaacgttgttgccattgctacaggcatcgtggtgtcacgctcgtcgtttggtatggcttcattcagctccggttcccaacgatcaaggcgagttacatgatcccccatgttgtgcaaaaaagcggttagctccttcggtcctccgatcgttgtcagaagtaagttggccgcagtgttatcactcatggttatggcagcactgcataattctcttactgtcatgccatccgtaagatgcttttctgtgactggtgagtactcaaccaagtcattctgagaatagtgtatgcggcgaccgagttgctcttgcccggcgtcaatacgggataataccgcgccacatagcagaactttaaaagtgctcatcattggaaaacgttcttcggggcgaaaactctcaaggatcttaccgctgttgagatccagttcgatgtaacccactcgtgcacccaactgatcttcagcatcttttactttcaccagcgtttctgggtgagcaaaaacaggaaggcaaaatgccgcaaaaaagggaataagggcgacacggaaatgttgaatactcatactcttcctttttcaatattattgaagcatttatcagggttattgtctcatgagcggatacatatttgaatgtatttagaaaaataaacaaataggggttccgcgcacatttccccgaaaagtgccacctgacgcgccctgtatcggcacgtctaattcgggggatctggattttagtactggattttggttttaggaattagaaattttattgatagaagtattttacaaatacaaatacatactaagggtttcttatatgctcaacacatgagcgaaaccctataggaaccctaattcccttatctgggaactactcacacattattatggagaaactcgagcttgtcgatcgacatgatcagggagccctagattatttgtatagttcatccatgcccattacgtcggtaaatgccttctgccactccttgaagttaagttcggtcttggaatgtttcaactcagtcttacggaacacgtacatgggttggttcttaaggtagttagcggccattggtttagcgaatgtgtaggtagtcctggctgtagagcgatatctcttgccattgcctgtggtgtaagaccatttgaaggtactaatgatggtcttgtcgttagggtaggttttcttggaccggcaccaatcagcggcagttaaggagttggtcatgacaggtccatcagcaggaaagcctgtccccttcacttgggcttctcctttgatgtggctcccttcgtaagtgtaacggtagttgacggtgagcgaagcaccgtcctcaaactgcattgtcctgtggacttggtatccggagccatcaaccatggctgcttggaatggactcattccgtcagggtatggaaggtattgatggaatccgtagccaatgtgtggcaccagaatccatggagaaaactgaagatcacctttggtgctcttgaggttcagctcttcgtatccgtcattagggttcccagtgccttgtccgaccatatcgaagtcaacgccgttgatggaaccgaagatgtgaagctcatgtgtggctggaagcgaagccatgttatcttcttctcctttactcacggaggacgccatggtggcgggatcgcgccctatcgttcgtaaatggtgaaaattttcagaaaattgcttttgctttaaaagaaatgatttaaattgctgcaatagaagtagaatgcttgattgcttgagattcgtttgttttgtatatgttgtgttgagaggatcctcaagcttcgacctgcagaagtaacaccaaacaacagggtgagcatcgacaaaagaaacagtaccaagcaaataaatagcgtatgaaggcagggctaaaaaaatccacatatagctgctgcatatgccatcatccaagtatatcaagatcaaaataattataaaacatacttgtttattataatagataggtactcaaggttagagcatatgaatagatgctgcatatgccatcatgtatatgcatcagtaaaacccacatcaacatgtatacctatcctagatcgatatttccatccatcttaaactcgtaactatgaagatgtatgacacacacatacagttccaaaattaataaatacaccaggtagtttgaaacagtattctactccgatctagaacgaatgaacgaccgcccaaccacaccacatcatcacaaccaagcgaacaaaaagcatctctgtatatgcatcagtaaaacccgcatcaacatgtatacctatcctagatcgatatttccatccatcatcttcaattcgtaactatgaatatgtatggcacacacatacagatccaaaattaataaatccaccaggtagtttgaaacagaattctactccgatctagaacgaccgcccaaccagaccacatcatcacaaccaagacaaaaaaaagcatgaaaagatgacccgacaaacaagtgcacggcatatattgaaataaaggaaaagggcaaaccaaaccctatgcaacgaaacaaaaaaaatcatgaaatcgatcccgtctgcggaacggctagagccatcccaggattccccaaagagaaacactggcaagttagcaatcagaacgtgtctgacgtacaggtcgcatccgtgtacgaacgctagcagcacggatctaacacaaacacggatctaacacaaacatgaacagaagtagaactaccgggccctaaccatggaccggaacgccgatctagagaaggtagagaggggggggggggaggacgagcggcgtaccttgaagcggaggtgccgacgggtggatttgggggagatccactagttctagagcggccgccaccgcggtggaattctcgaggtcctctccaaatgaaatgaacttccttatatagaggaagggtcttgcgaaggatagtgggattgtgcgtcatcccttacgtcagtggagatatcacatcaatccacttgctttgaagacgtggttggaacgtcttctttttccacgatgttcctcgtgggtgggggtccatctttgggaccactgtcggtagaggcatcttgaacgatagcctttcctttatcgcaatgatggcatttgtagaagccatcttccttttctactgtcctttcgatgaagtgacagatagctgggcaatggaatccgaggaggtttcccgatattaccctttgttgaaaagtctcaatagccctctggtcttctgagactgtatctttgatattcttggagtagacgagagtgtcgtgctccaccatgtatcacatcaatccacttgctttgaagacgtggttggaacgtcttctttttccacgatgttcctcgtgggtgggggtccatctttgggaccactgtcggtagaggcatcttgaacgatagcctttcctttatcgcaatgatggcatttgtagaagccatcttccttttctactgtcctttcgatgaagtgacagatagctgggcaatggaatccgaggaggtttcccgatattaccctttgttgaaaagtctcaatagccctctggtcttctgaacctgcaggcaagcaagcatgaatgcctgggcgcgccgatatc

SEQ ID NO: 38 - DNA, 3684 bp, synthetic construct
  misc_feature 1..3684: note = LbCpf1 RR coding sequence codon optimized
  source 1..3684: mol_type = other DNA
atgtccaaacttgaaaaatttacaaactgctactccctttccaagacgcttaggtttaaagcgatccccgttggcaagacccaagagaatatcgataacaaaagacttctggtcgaagatgaaaaaagggccgaagactacaagggggtcaagaagttgctcgatcgctattatctttcctttatcaacgatgtgcttcattcaatcaaactgaagaacttgaataactacattagccttttcagaaagaaaacgaggactgaaaaggagaacaaggaacttgagaatcttgaaataaaccttcgcaaagaaattgcaaaagccttcaaggggaacgaaggatataaatctcttttcaaaaaagacattatagaaacaattttgcctgagtttcttgacgacaaggatgaaattgcgctcgtcaatagctttaacggatttacaactgccttcacagggttcttcgacaatagggagaatatgtttagcgaggaggcaaaaagcacatccatcgcattcagatgcatcaatgaaaatcttacccggtacatatcgaatatggacatatttgaaaaagtggatgcaatattcgataagcacgaagtccaggagataaaggaaaagatactgaatagcgactatgatgtcgaagattttttcgaaggtgagttcttcaactttgtcctgactcaagaaggcattgatgtctataatgcaataattggaggttttgtgactgagtctggcgagaagataaagggcttgaacgagtatatcaatctctacaaccagaagactaagcaaaagttgcctaaatttaaaccgctttacaagcaagttttgagcgaccgggaaagcctttccttttacggtgaaggatacacgagcgatgaagaagtcctcgaagtcttccgcaacacactcaacaagaactcagaaatcttttcctcaattaaaaaattggagaagcttttcaagaacttcgatgaatactcttcggcggggatttttgtgaagaacggcccggcaatttccacaatatctaaagacattttcggagaatggaacgtgataagagacaagtggaatgcggagtatgatgacatacacctgaagaagaaggcagttgtgactgaaaaatacgaagatgacaggagaaaaagctttaaaaagatcgggtccttttcactggaacagctgcaggagtatgccgacgccgatctttcggttgtcgaaaagctcaaagaaataattatccagaaggtcgatgaaatctacaaggtgtacggctcaagcgagaagctctttgatgctgacttcgtgttggagaagtctcttaaaaaaaacgacgcagtcgtcgcgataatgaaagatttgctggattcagtgaaatccttcgagaattatatcaaagccttcttcggcgaggggaaggagacaaacagggatgagtccttctatggagacttcgttctggcttacgacatccttcttaaggtcgaccacatctatgacgcaattcggaactatgtgacgcagaagccgtattcgaaagataagttcaagctctatttccaaaaccctcaatttatgcgtgggtgggataaagacaaagagaccgattaccgggcaacaattttgcggtacgggtctaaatattacctcgctataatggataagaaatacgctaaatgtctccagaaaattgacaaagatgacgtcaacggcaattatgaaaaaatcaattataaactccttcctggcccaaataaaatgctcccgagggtgtttttttccaaaaagtggatggcctattataatccatcagaggatattcagaaaatctataaaaatgggacctttaagaagggtgacatgtttaacctgaacgattgccacaagcttatagattttttcaaagactctattagccgctatcccaaatggtctaatgcttatgatttcaacttctctgaaactgaaaagtacaaagatattgcaggattctaccgcgaagttgaagaacaaggttataaggtttcctttgagtctgcgtccaagaaagaggtcgataagttggtcgaagaagggaaattgtatatgtttcaaatttacaataaagacttttccgacaagtcccatggtacacctaatctgcataccatgtacttcaaactgctgttcgatgagaataatcacggtcagattcgcctgagcggaggggcggaactcttcatgaggagagcatcgttgaaaaaagaggagctcgtcgtgcatccggctaacagccccattgctaacaagaatccggataatccaaagaagactactaccctctcctatgacgtctataaggataagagattctctgaggaccagtacgagttgcacatccctattgcgataaataaatgccctaagaacatctttaaaatcaatactgaggtcagagtcctgcttaagcacgacgacaacccgtatgtgatcgggattgataggggtgaaaggaacttgctttatattgtggttgtcgatggaaaaggtaatatagtggaacaatactctctgaatgaaattatcaacaacttcaatggcattaggatcaagaccgactatcattctctgttggacaagaaagagaaagagcgcttcgaggcacggcaaaactggacgtctattgagaacatcaaggagcttaaggctggttacatttctcaggttgtgcacaaaatttgcgaactggtcgagaaatatgatgccgttatcgcacttgaagatctcaacagcggatttaagaattctcgggtgaaagtcgaaaaacaggtgtatcaaaaattcgaaaagatgctgatcgacaagctcaattatatggttgataaaaagagcaacccatgcgccacggggggtgcgcttaagggctatcagattacgaacaaatttgaatccttcaagtcaatgtcgacgcaaaatgggtttatattctatataccggcgtggcttacatctaaaatagatcctagcactgggttcgtgaacctgctgaaaaccaagtacacttcaatcgcagattctaaaaaatttataagcagcttcgacagaatcatgtatgtgcccgaggaagacctcttcgagtttgcccttgattacaaaaatttctcaagaacggatgcagactacataaagaagtggaagctgtactcttatgggaaccggattcggatattcagaaatccgaaaaaaaacaatgtctttgattgggaggaagtttgtcttacctctgcttacaaagagctgttcaataaatatggcattaattaccagcaaggtgatatccgggcgctcctttgcgaacagtctgacaaagctttctattcttcatttatggcgctcatgtcattgatgctgcagatgaggaatagcattacggggaggactgatgttgactttctgatctcgcccgtgaaaaattctgatggaatcttctacgattccaggaattatgaggcccaggaaaatgctatccttcccaagaacgcagacgcaaatggcgcgtacaatatagctcgcaaggttttgtgggctataggccaattcaagaaagccgaagacgaaaagctggacaaagttaagattgctatatctaacaaagagtggcttgagtatgcgcaaacatctgttaaacac

SEQ ID NO: 39 - DNA, 3684 bp, synthetic construct
  misc_feature 1..3684: note = LbCpf1 RVR coding sequence codon optimized
  source 1..3684: mol_type = other DNA
atgtccaaacttgaaaaatttacaaactgctactccctttccaagacgcttaggtttaaagcgatccccgttggcaagacccaagagaatatcgataacaaaagacttctggtcgaagatgaaaaaagggccgaagactacaagggggtcaagaagttgctcgatcgctattatctttcctttatcaacgatgtgcttcattcaatcaaactgaagaacttgaataactacattagccttttcagaaagaaaacgaggactgaaaaggagaacaaggaacttgagaatcttgaaataaaccttcgcaaagaaattgcaaaagccttcaaggggaacgaaggatataaatctcttttcaaaaaagacattatagaaacaattttgcctgagtttcttgacgacaaggatgaaattgcgctcgtcaatagctttaacggatttacaactgccttcacagggttcttcgacaatagggagaatatgtttagcgaggaggcaaaaagcacatccatcgcattcagatgcatcaatgaaaatcttacccggtacatatcgaatatggacatatttgaaaaagtggatgcaatattcgataagcacgaagtccaggagataaaggaaaagatactgaatagcgactatgatgtcgaagattttttcgaaggtgagttcttcaactttgtcctgactcaagaaggcattgatgtctataatgcaataattggaggttttgtgactgagtctggcgagaagataaagggcttgaacgagtatatcaatctctacaaccagaagactaagcaaaagttgcctaaatttaaaccgctttacaagcaagttttgagcgaccgggaaagcctttccttttacggtgaaggatacacgagcgatgaagaagtcctcgaagtcttccgcaacacactcaacaagaactcagaaatcttttcctcaattaaaaaattggagaagcttttcaagaacttcgatgaatactcttcggcggggatttttgtgaagaacggcccggcaatttccacaatatctaaagacattttcggagaatggaacgtgataagagacaagtggaatgcggagtatgatgacatacacctgaagaagaaggcagttgtgactgaaaaatacgaagatgacaggagaaaaagctttaaaaagatcgggtccttttcactggaacagctgcaggagtatgccgacgccgatctttcggttgtcgaaaagctcaaagaaataattatccagaaggtcgatgaaatctacaaggtgtacggctcaagcgagaagctctttgatgctgacttcgtgttggagaagtctcttaaaaaaaacgacgcagtcgtcgcgataatgaaagatttgctggattcagtgaaatccttcgagaattatatcaaagccttcttcggcgaggggaaggagacaaacagggatgagtccttctatggagacttcgttctggcttacgacatccttcttaaggtcgaccacatctatgacgcaattcggaactatgtgacgcagaagccgtattcgaaagataagttcaagctctatttccaaaaccctcaatttatgcgtgggtgggataaagacgtagagaccgatcgccgggcaacaattttgcggtacgggtctaaatattacctcgctataatggataagaaatacgctaaatgtctccagaaaattgacaaagatgacgtcaacggcaattatgaaaaaatcaattataaactccttcctggcccaaataaaatgctcccgaaggtgtttttttccaaaaagtggatggcctattataatccatcagaggatattcagaaaatctataaaaatgggacctttaagaagggtgacatgtttaacctgaacgattgccacaagcttatagattttttcaaagactctattagccgctatcccaaatggtctaatgcttatgatttcaacttctctgaaactgaaaagtacaaagatattgcaggattctaccgcgaagttgaagaacaaggttataaggtttcctttgagtctgcgtccaagaaagaggtcgataagttggtcgaagaagggaaattgtatatgtttcaaatttacaataaagacttttccgacaagtcccatggtacacctaatctgcataccatgtacttcaaactgctgttcgatgagaataatcacggtcagattcgcctgagcggaggggcggaactcttcatgaggagagcatcgttgaaaaaagaggagctcgtcgtgcatccggctaacagccccattgctaacaagaatccggataatccaaagaagactactaccctctcctatgacgtctataaggataagagattctctgaggaccagtacgagttgcacatccctattgcgataaataaatgccctaagaacatctttaaaatcaatactgaggtcagagtcctgcttaagcacgacgacaacccgtatgtgatcgggattgataggggtgaaaggaacttgctttatattgtggttgtcgatggaaaaggtaatatagtggaacaatactctctgaatgaaattatcaacaacttcaatggcattaggatcaagaccgactatcattctctgttggacaagaaagagaaagagcgcttcgaggcacggcaaaactggacgtctattgagaacatcaaggagcttaaggctggttacatttctcaggttgtgcacaaaatttgcgaactggtcgagaaatatgatgccgttatcgcacttgaagatctcaacagcggatttaagaattctcgggtgaaagtcgaaaaacaggtgtatcaaaaattcgaaaagatgctgatcgacaagctcaattatatggttgataaaaagagcaacccatgcgccacggggggtgcgcttaagggctatcagattacgaacaaatttgaatccttcaagtcaatgtcgacgcaaaatgggtttatattctatataccggcgtggcttacatctaaaatagatcctagcactgggttcgtgaacctgctgaaaaccaagtacacttcaatcgcagattctaaaaaatttataagcagcttcgacagaatcatgtatgtgcccgaggaagacctcttcgagtttgcccttgattacaaaaatttctcaagaacggatgcagactacataaagaagtggaagctgtactcttatgggaaccggattcggatattcagaaatccgaaaaaaaacaatgtctttgattgggaggaagtttgtcttacctctgcttacaaagagctgttcaataaatatggcattaattaccagcaaggtgatatccgggcgctcctttgcgaacagtctgacaaagctttctattcttcatttatggcgctcatgtcattgatgctgcagatgaggaatagcattacggggaggactgatgttgactttctgatctcgcccgtgaaaaattctgatggaatcttctacgattccaggaattatgaggcccaggaaaatgctatccttcccaagaacgcagacgcaaatggcgcgtacaatatagctcgcaaggttttgtgggctataggccaattcaagaaagccgaagacgaaaagctggacaaagttaagattgctatatctaacaaagagtggcttgagtatgcgcaaacatctgttaaacac

SEQ ID NO: 40 - protein, 1228 aa, synthetic construct
  REGION 1..1228: note = LbCpf1 RR polypeptide
MSKLEKFTNCYSLSKTLRFKAIPVGKTQENIDNKRLLVEDEKRAEDYKGVKKLLDRYYLSFINDVLHSIKLKNLNNYISLFRKKTRTEKENKELENLEINLRKEIAKAFKGNEGYKSLFKKDIIETILPEFLDDKDEIALVNSFNGFTTAFTGFFDNRENMFSEEAKSTSIAFRCINENLTRYISNMDIFEKVDAIFDKHEVQEIKEKILNSDYDVEDFFEGEFFNFVLTQEGIDVYNAIIGGFVTESGEKIKGLNEYINLYNQKTKQKLPKFKPLYKQVLSDRESLSFYGEGYTSDEEVLEVFRNTLNKNSEIFSSIKKLEKLFKNFDEYSSAGIFVKNGPAISTISKDIFGEWNVIRDKWNAEYDDIHLKKKAVVTEKYEDDRRKSFKKIGSFSLEQLQEYADADLSVVEKLKEIIIQKVDEIYKVYGSSEKLFDADFVLEKSLKKNDAVVAIMKDLLDSVKSFENYIKAFFGEGKETNRDESFYGDFVLAYDILLKVDHIYDAIRNYVTQKPYSKDKFKLYFQNPQFMRGWDKDKETDYRATILRYGSKYYLAIMDKKYAKCLQKIDKDDVNGNYEKINYKLLPGPNKMLPRVFFSKKWMAYYNPSEDIQKIYKNGTFKKGDMFNLNDCHKLIDFFKDSISRYPKWSNAYDFNFSETEKYKDIAGFYREVEEQGYKVSFESASKKEVDKLVEEGKLYMFQIYNKDFSDKSHGTPNLHTMYFKLLFDENNHGQIRLSGGAELFMRRASLKKEELVVHPANSPIANKNPDNPKKTTTLSYDVYKDKRFSEDQYELHIPIAINKCPKNIFKINTEVRVLLKHDDNPYVIGIDRGERNLLYIVVVDGKGNIVEQYSLNEIINNFNGIRIKTDYHSLLDKKEKERFEARQNWTSIENIKELKAGYISQVVHKICELVEKYDAVIALEDLNSGFKNSRVKVEKQVYQKFEKMLIDKLNYMVDKKSNPCATGGALKGYQITNKFESFKSMSTQNGFIFYIPAWLTSKIDPSTGFVNLLKTKYTSIADSKKFISSFDRIMYVPEEDLFEFALDYKNFSRTDADYIKKWKLYSYGNRIRIFRNPKKNNVFDWEEVCLTSAYKELFNKYGINYQQGDIRALLCEQSDKAFYSSFMALMSLMLQMRNSITGRTDVDFLISPVKNSDGIFYDSRNYEAQENAILPKNADANGAYNIARKVLWAIGQFKKAEDEKLDKVKIAISNKEWLEYAQTSVKH

SEQ ID NO: 41 - protein, 1228 aa, synthetic construct
  REGION 1..1228: note = LbCpf1 RVR polypeptide
MSKLEKFTNCYSLSKTLRFKAIPVGKTQENIDNKRLLVEDEKRAEDYKGVKKLLDRYYLSFINDVLHSIKLKNLNNYISLFRKKTRTEKENKELENLEINLRKEIAKAFKGNEGYKSLFKKDIIETILPEFLDDKDEIALVNSFNGFTTAFTGFFDNRENMFSEEAKSTSIAFRCINENLTRYISNMDIFEKVDAIFDKHEVQEIKEKILNSDYDVEDFFEGEFFNFVLTQEGIDVYNAIIGGFVTESGEKIKGLNEYINLYNQKTKQKLPKFKPLYKQVLSDRESLSFYGEGYTSDEEVLEVFRNTLNKNSEIFSSIKKLEKLFKNFDEYSSAGIFVKNGPAISTISKDIFGEWNVIRDKWNAEYDDIHLKKKAVVTEKYEDDRRKSFKKIGSFSLEQLQEYADADLSVVEKLKEIIIQKVDEIYKVYGSSEKLFDADFVLEKSLKKNDAVVAIMKDLLDSVKSFENYIKAFFGEGKETNRDESFYGDFVLAYDILLKVDHIYDAIRNYVTQKPYSKDKFKLYFQNPQFMRGWDKDVETDRRATILRYGSKYYLAIMDKKYAKCLQKIDKDDVNGNYEKINYKLLPGPNKMLPKVFFSKKWMAYYNPSEDIQKIYKNGTFKKGDMFNLNDCHKLIDFFKDSISRYPKWSNAYDFNFSETEKYKDIAGFYREVEEQGYKVSFESASKKEVDKLVEEGKLYMFQIYNKDFSDKSHGTPNLHTMYFKLLFDENNHGQIRLSGGAELFMRRASLKKEELVVHPANSPIANKNPDNPKKTTTLSYDVYKDKRFSEDQYELHIPIAINKCPKNIFKINTEVRVLLKHDDNPYVIGIDRGERNLLYIVVVDGKGNIVEQYSLNEIINNFNGIRIKTDYHSLLDKKEKERFEARQNWTSIENIKELKAGYISQVVHKICELVEKYDAVIALEDLNSGFKNSRVKVEKQVYQKFEKMLIDKLNYMVDKKSNPCATGGALKGYQITNKFESFKSMSTQNGFIFYIPAWLTSKIDPSTGFVNLLKTKYTSIADSKKFISSFDRIMYVPEEDLFEFALDYKNFSRTDADYIKKWKLYSYGNRIRIFRNPKKNNVFDWEEVCLTSAYKELFNKYGINYQQGDIRALLCEQSDKAFYSSFMALMSLMLQMRNSITGRTDVDFLISPVKNSDGIFYDSRNYEAQENAILPKNADANGAYNIARKVLWAIGQFKKAEDEKLDKVKIAISNKEWLEYAQTSVKH

SEQ ID NO: 42 - DNA, 27 bp, synthetic construct
  misc_feature 1..27: note = SV40 NLS
  source 1..27: mol_type = other DNA
atggcaccaaagaaaaaaaggaaagtt

SEQ ID NO: 43 - DNA, 48 bp, synthetic construct
  misc_feature 1..48: note = Nucleoplasmin NLS
  source 1..48: mol_type = other DNA
aaacgccccgcggctacaaagaaggctggccaggcaaagaagaagaag

SEQ ID NO: 44 - DNA, 3849 bp, synthetic construct
  misc_feature 1..3849: note = pGEP296 Ribozyme strategy vector
  source 1..3849: mol_type = other DNA
ctgacgcgccctgtagcggcctgcagtgcagcgtgacccggtcgtgcccctctctagagataatgagcattgcatgtctaagttataaaaaattaccacatattttttttgtcacacttgtttgaagtgcagtttatctatctttatacatatatttaaactttactctacgaataatataatctatagtactacaataatatcagtgttttagagaatcatataaatgaacagttagacatggtctaaaggacaattgagtattttgacaacaggactctacagttttatctttttagtgtgcatgtgttctcctttttttttgcaaatagcttcacctatataatacttcatccattttattagtacatccatttagggtttagggttaatggtttttatagactaatttttttagtacatctattttattctattttagcctctaaattaagaaaactaaaactctattttagtttttttatttaataatttagatataaaatagaataaaataaagtgactaaaaattaaacaaataccctttaagaaattaaaaaaactaaggaaacatttttcttgtttcgagtagataatgccagcctgttaaacgccgtcgatcgacgagtctaacggacaccaaccagcgaaccagcagcgtcgcgtcgggccaagcgaagcagacggcacggcatctctgtcgctgcctctggacccctctcgagagttccgctccaccgttggacttgctccgctgtcggcatccagaaattgcgtggcggagcggcagacgtgagccggcacggcaggcggcctcctcctcctctcacggcaccggcagctacgggggattcctttcccaccgctccttcgctttcccttcctcgcccgccgtaataaatagacaccccctccacaccctctttccccaacctcgtgttgttcggagcgcacacacacacaaccagatctcccccaaatccacccgtcggcacctccgcttcaaggtacgccgctcgtcctccccccccccccctctctaccttctctagatcggcgttccggtccatggttagggcccggtagttctacttctgttcatgtttgtgttagatccgtgtttgtgttagatccgtgctgctagcgttcgtacacggatgcgacctgtacgtcagacacgttctgattgctaacttgccagtgtttctctttggggaatcctgggatggctctagccgttccgcagacgggatcgatctaggataggtatacatgttgatgtgggttttactgatgcatatacatgatggcatatgcagcatctattcatatgctctaaccttgagtacctatctattataataaacaagtatgttttataattattttgatcttgatatacttggatgatggcatatgcagcagctatatgtggatttttttagccctgccttcatacgctatttatttgcttggtactgtttcttttgtcgatgctcaccctgttgtttggtgttacttctgcagggatccaaattactgatgagtccgtgaggacgaaacgagtaagctcgtctaatttctactaagtgtagatgagacggagctcagtctgaccgcggcgtctctggccggcatggtcccagcctcctcgctggcgccggctgggcaacatgcttcggcatggcgaatgggaccgatcgttcaaacatttggcaataaagtttcttaagattgaatcctgttgccggtcttgcgatgattatcatataatttctgttgaattacgttaagcatgtaataattaacatgtaatgcatgacgttatttatgagatgggtttttatgattagagtcccgcaattatacatttaatacgcgatagaaaacaaaatatagcgcgcaaactaggataaattatcgcgcgcggtgtcatctatgttactagatcgatcgtcgttcggctgcggcgagcggtatcagctcactcaaaggcggtaatacggttatccacagaatcaggggataacgcaggaaagaacatgtgagcaaaaggccagcaaaaggccaggaaccgtaaaaaggccgcgttgctggcgtttttccataggctccgcccccctgacgagcatcacaaaaatcgacgctcaagtcagaggtggcgaaacccgacaggactataaagataccaggcgtttccccctggaagctccctcgtgcgctctcctgttccgaccctgccgcttaccggatacctgtccgcctttctcccttcgggaagcgtggcgctttctcatagctcacgctgtaggtatctcagttcggtgtaggtcgttcgctccaagctgggctgtgtgcacgaaccccccgttcagcccgaccgctgcgccttatccggtaactatcgtcttgagtccaacccggtaagacacgacttatcgccactggcagcagccactggtaacaggattagcagagcgaggtatgtaggcggtgctacagagttcttgaagtggtggcctaactacggctacactagaagaacagtatttggtatctgcgctctgctgaagccagttaccttcggaaaaagagttggtagctcttgatccggcaaacaaaccaccgctggtagcggtggtttttttgtttgcaagcagcagattacgcgcagaaaaaaaggatctcaagaagatcctttgatcttttctacggggtctgacgctcagtggaacgaaaactcacgttaagggattttggtcatgagattatcaaaaaggatcttcacctagatccttttaaattaaaaatgaagttttaaatcaatctaaagtatatatgagtaaacttggtctgacagttaccaatgcttaatcagtgaggcacctatctcagcgatctgtctatttcgttcatccatagttgcctgactccccgtcgtgtagataactacgatacgggagggcttaccatctggccccagtgctgcaatgataccgcgagacccacgctcaccggctccagatttatcagcaataaaccagccagccggaagggccgagcgcagaagtggtcctgcaactttatccgcctccatccagtctattaattgttgccgggaagctagagtaagtagttcgccagttaatagtttgcgcaacgttgttgccattgctacaggcatcgtggtgtcacgctcgtcgtttggtatggcttcattcagctccggttcccaacgatcaaggcgagttacatgatcccccatgttgtgcaaaaaagcggttagctccttcggtcctccgatcgttgtcagaagtaagttggccgcagtgttatcactcatggttatggcagcactgcataattctcttactgtcatgccatccgtaagatgcttttctgtgactggtgagtactcaaccaagtcattctgagaatagtgtatgcggcgaccgagttgctcttgcccggcgtcaatacgggataataccgcgccacatagcagaactttaaaagtgctcatcattggaaaacgttcttcggggcgaaaactctcaaggatcttaccgctgttgagatccagttcgatgtaacccactcgtgcacccaactgatcttcagcatcttttactttcaccagcgtttctgggtgagcaaaaacaggaaggcaaaatgccgcaaaaaagggaataagggcgacacggaaatgttgaatactcatactcttcctttttcaatattattgaagcatttatcagggttattgtctcatgagcggatacatatttgaatgtatttagaaaaataaacaaataggggttccgcgcacatttccccgaaaagtgccac

SEQ ID NO: 45 - DNA, 3834 bp, synthetic construct
  misc_feature 1..3834: note = pGEP374 vector with rice HDV-like ribozyme sequence
  source 1..3834: mol_type = other DNA
ctgacgcgccctgtagcggcctgcagtgcagcgtgacccggtcgtgcccctctctagagataatgagcattgcatgtctaagttataaaaaattaccacatattttttttgtcacacttgtttgaagtgcagtttatctatctttatacatatatttaaactttactctacgaataatataatctatagtactacaataatatcagtgttttagagaatcatataaatgaacagttagacatggtctaaaggacaattgagtattttgacaacaggactctacagttttatctttttagtgtgcatgtgttctcctttttttttgcaaatagcttcacctatataatacttcatccattttattagtacatccatttagggtttagggttaatggtttttatagactaatttttttagtacatctattttattctattttagcctctaaattaagaaaactaaaactctattttagtttttttatttaataatttagatataaaatagaataaaataaagtgactaaaaattaaacaaataccctttaagaaattaaaaaaactaaggaaacatttttcttgtttcgagtagataatgccagcctgttaaacgccgtcgatcgacgagtctaacggacaccaaccagcgaaccagcagcgtcgcgtcgggccaagcgaagcagacggcacggcatctctgtcgctgcctctggacccctctcgagagttccgctccaccgttggacttgctccgctgtcggcatccagaaattgcgtggcggagcggcagacgtgagccggcacggcaggcggcctcctcctcctctcacggcaccggcagctacgggggattcctttcccaccgctccttcgctttcccttcctcgcccgccgtaataaatagacaccccctccacaccctctttccccaacctcgtgttgttcggagcgcacacacacacaaccagatctcccccaaatccacccgtcggcacctccgcttcaaggtacgccgctcgtcctccccccccccccctctctaccttctctagatcggcgttccggtccatggttagggcccggtagttctacttctgttcatgtttgtgttagatccgtgtttgtgttagatccgtgctgctagcgttcgtacacggatgcgacctgtacgtcagacacgttctgattgctaacttgccagtgtttctctttggggaatcctgggatggctctagccgttccgcagacgggatcgatctaggataggtatacatgttgatgtgggttttactgatgcatatacatgatggcatatgcagcatctattcatatgctctaaccttgagtacctatctattataataaacaagtatgttttataattattttgatcttgatatacttggatgatggcatatgcagcagctatatgtggatttttttagccctgccttcatacgctatttatttgcttggtactgtttcttttgtcgatgctcaccctgttgtttggtgttacttctgcagggatccaaattactgatgagtccgtgaggacgaaacgagtaagctcgtctaatttctactaagtgtagatgagacggagctcagtctgaccgcggcgtctctccgccaacactgccaatgccggtcccaagcccggataaaagtggagggggcggcgatcgttcaaacatttggcaataaagtttcttaagattgaatcctgttgccggtcttgcgatgattatcatataatttctgttgaattacgttaagcatgtaataattaacatgtaatgcatgacgttatttatgagatgggtttttatgattagagtcccgcaattatacatttaatacgcgatagaaaacaaaatatagcgcgcaaactaggataaattatcgcgcgcggtgtcatctatgttactagatcgatcgtcgttcggctgcggcgagcggtatcagctcactcaaaggcggtaatacggttatccacagaatcaggggataacgcaggaaagaacatgtgagcaaaaggccagcaaaaggccaggaaccgtaaaaaggccgcgttgctggcgtttttccataggctccgcccccctgacgagcatcacaaaaatcgacgctcaagtcagaggtggcgaaacccgacaggactataaagataccaggcgtttccccctggaagctccctcgtgcgctctcctgttccgaccctgccgcttaccggatacctgtccgcctttctcccttcgggaagcgtggcgctttctcatagctcacgctgtaggtatctcagttcggtgtaggtcgttcgctccaagctgggctgtgtgcacgaaccccccgttcagcccgaccgctgcgccttatccggtaactatcgtcttgagtccaacccggtaagacacgacttatcgccactggcagcagccactggtaacaggattagcagagcgaggtatgtaggcggtgctacagagttcttgaagtggtggcctaactacggctacactagaagaacagtatttggtatctgcgctctgctgaagccagttaccttcggaaaaagagttggtagctcttgatccggcaaacaaaccaccgctggtagcggtggtttttttgtttgcaagcagcagattacgcgcagaaaaaaaggatctcaagaagatcctttgatcttttctacggggtctgacgctcagtggaacgaaaactcacgttaagggattttggtcatgagattatcaaaaaggatcttcacctagatccttttaaattaaaaatgaagttttaaatcaatctaaagtatatatgagtaaacttggtctgacagttaccaatgcttaatcagtgaggcacctatctcagcgatctgtctatttcgttcatccatagttgcctgactccccgtcgtgtagataactacgatacgggagggcttaccatctggccccagtgctgcaatgataccgcgagacccacgctcaccggctccagatttatcagcaataaaccagccagccggaagggccgagcgcagaagtggtcctgcaactttatccgcctccatccagtctattaattgttgccgggaagctagagtaagtagttcgccagttaatagtttgcgcaacgttgttgccattgctacaggcatcgtggtgtcacgctcgtcgtttggtatggcttcattcagctccggttcccaacgatcaaggcgagttacatgatcccccatgttgtgcaaaaaagcggttagctccttcggtcctccgatcgttgtcagaagtaagttggccgcagtgttatcactcatggttatggcagcactgcataattctcttactgtcatgccatccgtaagatgcttttctgtgactggtgagtactcaaccaagtcattctgagaatagtgtatgcggcgaccgagttgctcttgcccggcgtcaatacgggataataccgcgccacatagcagaactttaaaagtgctcatcattggaaaacgttcttcggggcgaaaactctcaaggatcttaccgctgttgagatccagttcgatgtaacccactcgtgcacccaactgatcttcagcatcttttactttcaccagcgtttctgggtgagcaaaaacaggaaggcaaaatgccgcaaaaaagggaataagggcgacacggaaatgttgaatactcatactcttcctttttcaatattattgaagcatttatcagggttattgtctcatgagcggatacatatttgaatgtatttagaaaaataaacaaataggggttccgcgcacatttccccgaaaagtgccac

SEQ ID NO: 46 - DNA, 3844 bp, synthetic construct
  misc_feature 1..3844: note = pGEP375 vector with sunflower HDV-like sequence
  source 1..3844: mol_type = other DNA
ctgacgcgccctgtagcggcctgcagtgcagcgtgacccggtcgtgcccctctctagagataatgagcattgcatgtctaagttataaaaaattaccacatattttttttgtcacacttgtttgaagtgcagtttatctatctttatacatatatttaaactttactctacgaataatataatctatagtactacaataatatcagtgttttagagaatcatataaatgaacagttagacatggtctaaaggacaattgagtattttgacaacaggactctacagttttatctttttagtgtgcatgtgttctcctttttttttgcaaatagcttcacctatataatacttcatccattttattagtacatccatttagggtttagggttaatggtttttatagactaatttttttagtacatctattttattctattttagcctctaaattaagaaaactaaaactctattttagtttttttatttaataatttagatataaaatagaataaaataaagtgactaaaaattaaacaaataccctttaagaaattaaaaaaactaaggaaacatttttcttgtttcgagtagataatgccagcctgttaaacgccgtcgatcgacgagtctaacggacaccaaccagcgaaccagcagcgtcgcgtcgggccaagcgaagcagacggcacggcatctctgtcgctgcctctggacccctctcgagagttccgctccaccgttggacttgctccgctgtcggcatccagaaattgcgtggcggagcggcagacgtgagccggcacggcaggcggcctcctcctcctctcacggcaccggcagctacgggggattcctttcccaccgctccttcgctttcccttcctcgcccgccgtaataaatagacaccccctccacaccctctttccccaacctcgtgttgttcggagcgcacacacacacaaccagatctcccccaaatccacccgtcggcacctccgcttcaaggtacgccgctcgtcctccccccccccccctctctaccttctctagatcggcgttccggtccatggttagggcccggtagttctacttctgttcatgtttgtgttagatccgtgtttgtgttagatccgtgctgctagcgttcgtacacggatgcgacctgtacgtcagacacgttctgattgctaacttgccagtgtttctctttggggaatcctgggatggctctagccgttccgcagacgggatcgatctaggataggtatacatgttgatgtgggttttactgatgcatatacatgatggcatatgcagcatctattcatatgctctaaccttgagtacctatctattataataaacaagtatgttttataattattttgatcttgatatacttggatgatggcatatgcagcagctatatgtggatttttttagccctgccttcatacgctatttatttgcttggtactgtttcttttgtcgatgctcaccctgttgtttggtgttacttctgcagggatccaaattactgatgagtccgtgaggacgaaacgagtaagctcgtctaatttctactaagtgtagatgagacggagctcagtctgaccgcggcgtctctgcggggggcgtcagtcctactctgcacctcctcgtggtgtcgcctgggaaccctctttcgcaacgatcgttcaaacatttggcaataaagtttcttaagattgaatcctgttgccggtcttgcgatgattatcatataatttctgttgaattacgttaagcatgtaataattaacatgtaatgcatgacgttatttatgagatgggtttttatgattagagtcccgcaattatacatttaatacgcgatagaaaacaaaatatagcgcgcaaactaggataaattatcgcgcgcggtgtcatctatgttactagatcgatcgtcgttcggctgcggcgagcggtatcagctcactcaaaggcggtaatacggttatccacagaatcaggggataacgcaggaaagaacatgtgagcaaaaggccagcaaaaggccaggaaccgtaaaaaggccgcgttgctggcgtttttccataggctccgcccccctgacgagcatcacaaaaatcgacgctcaagtcagaggtggcgaaacccgacaggactataaagataccaggcgtttccccctggaagctccctcgtgcgctctcctgttccgaccctgccgcttaccggatacctgtccgcctttctcccttcgggaagcgtggcgctttctcatagctcacgctgtaggtatctcagttcggtgtaggtcgttcgctccaagctgggctgtgtgcacgaaccccccgttcagcccgaccgctgcgccttatccggtaactatcgtcttgagtccaacccggtaagacacgacttatcgccactggcagcagccactggtaacaggattagcagagcgaggtatgtaggcggtgctacagagttcttgaagtggtggcctaactacggctacactagaagaacagtatttggtatctgcgctctgctgaagccagttaccttcggaaaaagagttggtagctcttgatccggcaaacaaaccaccgctggtagcggtggtttttttgtttgcaagcagcagattacgcgcagaaaaaaaggatctcaagaagatcctttgatcttttctacggggtctgacgctcagtggaacgaaaactcacgttaagggattttggtcatgagattatcaaaaaggatcttcacctagatccttttaaattaaaaatgaagttttaaatcaatctaaagtatatatgagtaaacttggtctgacagttaccaatgcttaatcagtgaggcacctatctcagcgatctgtctatttcgttcatccatagttgcctgactccccgtcgtgtagataactacgatacgggagggcttaccatctggccccagtgctgcaatgataccgcgagacccacgctcaccggctccagatttatcagcaataaaccagccagccggaagggccgagcgcagaagtggtcctgcaactttatccgcctccatccagtctattaattgttgccgggaagctagagtaagtagttcgccagttaatagtttgcgcaacgttgttgccattgctacaggcatcgtggtgtcacgctcgtcgtttggtatggcttcattcagctccggttcccaacgatcaaggcgagttacatgatcccccatgttgtgcaaaaaagcggttagctccttcggtcctccgatcgttgtcagaagtaagttggccgcagtgttatcactcatggttatggcagcactgcataattctcttactgtcatgccatccgtaagatgcttttctgtgactggtgagtactcaaccaagtcattctgagaatagtgtatgcggcgaccgagttgctcttgcccggcgtcaatacgggataataccgcgccacatagcagaactttaaaagtgctcatcattggaaaacgttcttcggggcgaaaactctcaaggatcttaccgctgttgagatccagttcgatgtaacccactcgtgcacccaactgatcttcagcatcttttactttcaccagcgtttctgggtgagcaaaaacaggaaggcaaaatgccgcaaaaaagggaataagggcgacacggaaatgttgaatactcatactcttcctttttcaatattattgaagcatttatcagggttattgtctcatgagcggatacatatttgaatgtatttagaaaaataaacaaataggggttccgcgcacatttccccgaaaagtgccac

SEQ ID NO: 47 - DNA, 3867 bp, synthetic construct
  misc_feature 1..3867: note = pGEP375 vector with sunflower HDV-like sequence_long
  source 1..3867: mol_type = other DNA
ctgacgcgccctgtagcggcctgcagtgcagcgtgacccggtcgtgcccctctctagagataatgagcattgcatgtctaagttataaaaaattaccacatattttttttgtcacacttgtttgaagtgcagtttatctatctttatacatatatttaaactttactctacgaataatataatctatagtactacaataatatcagtgttttagagaatcatataaatgaacagttagacatggtctaaaggacaattgagtattttgacaacaggactctacagttttatctttttagtgtgcatgtgttctcctttttttttgcaaatagcttcacctatataatacttcatccattttattagtacatccatttagggtttagggttaatggtttttatagactaatttttttagtacatctattttattctattttagcctctaaattaagaaaactaaaactctattttagtttttttatttaataatttagatataaaatagaataaaataaagtgactaaaaattaaacaaataccctttaagaaattaaaaaaactaaggaaacatttttcttgtttcgagtagataatgccagcctgttaaacgccgtcgatcgacgagtctaacggacaccaaccagcgaaccagcagcgtcgcgtcgggccaagcgaagcagacggcacggcatctctgtcgctgcctctggacccctctcgagagttccgctccaccgttggacttgctccgctgtcggcatccagaaattgcgtggcggagcggcagacgtgagccggcacggcaggcggcctcctcctcctctcacggcaccggcagctacgggggattcctttcccaccgctccttcgctttcccttcctcgcccgccgtaataaatagacaccccctccacaccctctttccccaacctcgtgttgttcggagcgcacacacacacaaccagatctcccccaaatccacccgtcggcacctccgcttcaaggtacgccgctcgtcctccccccccccccctctctaccttctctagatcggcgttccggtccatggttagggcccggtagttctacttctgttcatgtttgtgttagatccgtgtttgtgttagatccgtgctgctagcgttcgtacacggatgcgacctgtacgtcagacacgttctgattgctaacttgccagtgtttctctttggggaatcctgggatggctctagccgttccgcagacgggatcgatctaggataggtatacatgttgatgtgggttttactgatgcatatacatgatggcatatgcagcatctattcatatgctctaaccttgagtacctatctattataataaacaagtatgttttataattattttgatcttgatatacttggatgatggcatatgcagcagctatatgtggatttttttagccctgccttcatacgctatttatttgcttggtactgtttcttttgtcgatgctcaccctgttgtttggtgttacttctgcagggatccaaattactgatgagtccgtgaggacgaaacgagtaagctcgtctaatttctactaagtgtagatgagacggagctcagtctgaccgcggcgtctctgcggggggcgtcagtcctactctgcacctcctcgtggtgtcgcctgggaaccctctttcgcaagaaagaggagccaagcagagaggcgatcgttcaaacatttggcaataaagtttcttaagattgaatcctgttgccggtcttgcgatgattatcatataatttctgttgaattacgttaagcatgtaataattaacatgtaatgcatgacgttatttatgagatgggtttttatgattagagtcccgcaattatacatttaatacgcgatagaaaacaaaatatagcgcgcaaactaggataaattatcgcgcgcggtgtcatctatgttactagatcgatcgtcgttcggctgcggcgagcggtatcagctcactcaaaggcggtaatacggttatccacagaatcaggggataacgcaggaaagaacatgtgagcaaaaggccagcaaaaggccaggaaccgtaaaaaggccgcgttgctggcgtttttccataggctccgcccccctgacgagcatcacaaaaatcgacgctcaagtcagaggtggcgaaacccgacaggactataaagataccaggcgtttccccctggaagctccctcgtgcgctctcctgttccgaccctgccgcttaccggatacctgtccgcctttctcccttcgggaagcgtggcgctttctcatagctcacgctgtaggtatctcagttcggtgtaggtcgttcgctccaagctgggctgtgtgcacgaaccccccgttcagcccgaccgctgcgccttatccggtaactatcgtcttgagtccaacccggtaagacacgacttatcgccactggcagcagccactggtaacaggattagcagagcgaggtatgtaggcggtgctacagagttcttgaagtggtggcctaactacggctacactagaagaacagtatttggtatctgcgctctgctgaagccagttaccttcggaaaaagagttggtagctcttgatccggcaaacaaaccaccgctggtagcggtggtttttttgtttgcaagcagcagattacgcgcagaaaaaaaggatctcaagaagatcctttgatcttttctacggggtctgacgctcagtggaacgaaaactcacgttaagggattttggtcatgagattatcaaaaaggatcttcacctagatccttttaaattaaaaatgaagttttaaatcaatctaaagtatatatgagtaaacttggtctgacagttaccaatgcttaatcagtgaggcacctatctcagcgatctgtctatttcgttcatccatagttgcctgactccccgtcgtgtagataactacgatacgggagggcttaccatctggccccagtgctgcaatgataccgcgagacccacgctcaccggctccagatttatcagcaataaaccagccagccggaagggccgagcgcagaagtggtcctgcaactttatccgcctccatccagtctattaattgttgccgggaagctagagtaagtagttcgccagttaatagtttgcgcaacgttgttgccattgctacaggcatcgtggtgtcacgctcgtcgtttggtatggcttcattcagctccggttcccaacgatcaaggcgagttacatgatcccccatgttgtgcaaaaaagcggttagctccttcggtcctccgatcgttgtcagaagtaagttggccgcagtgttatcactcatggttatggcagcactgcataattctcttactgtcatgccatccgtaagatgcttttctgtgactggtgagtactcaaccaagtcattctgagaatagtgtatgcggcgaccgagttgctcttgcccggcgtcaatacgggataataccgcgccacatagcagaactttaaaagtgctcatcattggaaaacgttcttcggggcgaaaactctcaaggatcttaccgctgttgagatccagttcgatgtaacccactcgtgcacccaactgatcttcagcatcttttactttcaccagcgtttctgggtgagcaaaaacaggaaggcaaaatgccgcaaaaaagggaataagggcgacacggaaatgttgaatactcatactcttcctttttcaatattattgaagcatttatcagggttattgtctcatgagcggatacatatttgaatgtatttagaaaaataaacaaataggggttccgcgcacatttccccgaaaagtgccac

SEQ ID NO: 48 - DNA, 3861 bp, synthetic construct
  misc_feature 1..3861: note = pGEP376 vector with artichoke HDV-like sequence
  source 1..3861: mol_type = other DNA
ctgacgcgccctgtagcggcctgcagtgcagcgtgacccggtcgtgcccctctctagagataatgagcattgcatgtctaagttataaaaaattaccacatattttttttgtcacacttgtttgaagtgcagtttatctatctttatacatatatttaaactttactctacgaataatataatctatagtactacaataatatcagtgttttagagaatcatataaatgaacagttagacatggtctaaaggacaattgagtattttgacaacaggactctacagttttatctttttagtgtgcatgtgttctcctttttttttgcaaatagcttcacctatataatacttcatccattttattagtacatccatttagggtttagggttaatggtttttatagactaatttttttagtacatctattttattctattttagcctctaaattaagaaaactaaaactctattttagtttttttatttaataatttagatataaaatagaataaaataaagtgactaaaaattaaacaaataccctttaagaaattaaaaaaactaaggaaacatttttcttgtttcgagtagataatgccagcctgttaaacgccgtcgatcgacgagtctaacggacaccaaccagcgaaccagcagcgtcgcgtcgggccaagcgaagcagacggcacggcatctctgtcgctgcctctggacccctctcgagagttccgctccaccgttggacttgctccgctgtcggcatccagaaattgcgtggcggagcggcagacgtgagccggcacggcaggcggcctcctcctcctctcacggcaccggcagctacgggggattcctttcccaccgctccttcgctttcccttcctcgcccgccgtaataaatagacaccccctccacaccctctttccccaacctcgtgttgttcggagcgcacacacacacaaccagatctcccccaaatccacccgtcggcacctccgcttcaaggtacgccgctcgtcctccccccccccccctctctaccttctctagatcggcgttccggtccatggttagggcccggtagttctacttctgttcatgtttgtgttagatccgtgtttgtgttagatccgtgctgctagcgttcgtacacggatgcgacctgtacgtcagacacgttctgattgctaacttgccagtgtttctctttggggaatcctgggatggctctagccgttccgcagacgggatcgatctaggataggtatacatgttgatgtgggttttactgatgcatatacatgatggcatatgcagcatctattcatatgctctaaccttgagtacctatctattataataaacaagtatgttttataattattttgatcttgatatacttggatgatggcatatgcagcagctatatgtggatttttttagccctgccttcatacgctatttatttgcttggtactgtttcttttgtcgatgctcaccctgttgtttggtgttacttctgcagggatccaaattactgatgagtccgtgaggacgaaacgagtaagctcgtctaatttctactaagtgtagatgagacggagctcagtctgaccgcggcgtctctggcgtcagtcctactctgcacctcctcgtggtgtcgcctgggaaccctctttcacaagaaagaggagccaagcagagaggcgatcgttcaaacatttggcaataaagtttcttaagattgaatcctgttgccggtcttgcgatgattatcatataatttctgttgaattacgttaagcatgtaataattaacatgtaatgcatgacgttatttatgagatgggtttttatgattagagtcccgcaattatacatttaatacgcgatagaaaacaaaatatagcgcgcaaactaggataaattatcgcgcgcggtgtcatctatgttactagatcgatcgtcgttcggctgcggcgagcggtatcagctcactcaaaggcggtaatacggttatccacagaatcaggggataacgcaggaaagaacatgtgagcaaaaggccagcaaaaggccaggaaccgtaaaaaggccgcgttgctggcgtttttccataggctccgcccccctgacgagcatcacaaaaatcgacgctcaagtcagaggtggcgaaacccgacaggactataaagataccaggcgtttccccctggaagctccctcgtgcgctctcctgttccgaccctgccgcttaccggatacctgtccgcctttctcccttcgggaagcgtggcgctttctcatagctcacgctgtaggtatctcagttcggtgtaggtcgttcgctccaagctgggctgtgtgcacgaaccccccgttcagcccgaccgctgcgccttatccggtaactatcgtcttgagtccaacccggtaagacacgacttatcgccactggcagcagccactggtaacaggattagcagagcgaggtatgtaggcggtgctacagagttcttgaagtggtggcctaactacggctacactagaagaacagtatttggtatctgcgctctgctgaagccagttaccttcggaaaaagagttggtagctcttgatccggcaaacaaaccaccgctggtagcggtggtttttttgtttgcaagcagcagattacgcgcagaaaaaaaggatctcaagaagatcctttgatcttttctacggggtctgacgctcagtggaacgaaaactcacgttaagggattttggtcatgagattatcaaaaaggatcttcacctagatccttttaaattaaaaatgaagttttaaatcaatctaaagtatatatgagtaaacttggtctgacagttaccaatgcttaatcagtgaggcacctatctcagcgatctgtctatttcgttcatccatagttgcctgactccccgtcgtgtagataactacgatacgggagggcttaccatctggccccagtgctgcaatgataccgcgagacccacgctcaccggctccagatttatcagcaataaaccagccagccggaagggccgagcgcagaagtggtcctgcaactttatccgcctccatccagtctattaattgttgccgggaagctagagtaagtagttcgccagttaatagtttgcgcaacgttgttgccattgctacaggcatcgtggtgtcacgctcgtcgtttggtatggcttcattcagctccggttcccaacgatcaaggcgagttacatgatcccccatgttgtgcaaaaaagcggttagctccttcggtcctccgatcgttgtcagaagtaagttggccgcagtgttatcactcatggttatggcagcactgcataattctcttactgtcatgccatccgtaagatgcttttctgtgactggtgagtactcaaccaagtcattctgagaatagtgtatgcggcgaccgagttgctcttgcccggcgtcaatacgggataataccgcgccacatagcagaactttaaaagtgctcatcattggaaaacgttcttcggggcgaaaactctcaaggatcttaccgctgttgagatccagttcgatgtaacccactcgtgcacccaactgatcttcagcatcttttactttcaccagcgtttctgggtgagcaaaaacaggaaggcaaaatgccgcaaaaaagggaataagggcgacacggaaatgttgaatactcatactcttcctttttcaatattattgaagcatttatcagggttattgtctcatgagcggatacatatttgaatgtatttagaaaaataaacaaataggggttccgcgcacatttccccgaaaagtgccac

SEQ ID NO: 49 - DNA, 24 bp, Zea mays
  source 1..24: mol_type = genomic DNA
ctcgtcacgattcccctctcctgg

SEQ ID NO: 50 - DNA, 24 bp, Zea mays
  source 1..24: mol_type = genomic DNA
cccacctgaaaagttcgaccagga

SEQ ID NO: 51 - DNA, 24 bp, Zea mays
  source 1..24: mol_type = genomic DNA
tgtgtggtcacacttgccagccag

SEQ ID NO: 52 - DNA, 24 bp, Zea mays
  source 1..24: mol_type = genomic DNA
gtggtcggatttctggcatcgctg

SEQ ID NO: 53 - DNA, 23 bp, Zea mays
  source 1..23: mol_type = genomic DNA
gtctatgtcgatgaccagcagat

SEQ ID NO: 54 - DNA, 24 bp, Zea mays
  source 1..24: mol_type = genomic DNA
cctctcctggtcgaacttttcagg

SEQ ID NO: 55 - DNA, 24 bp, Zea mays
  source 1..24: mol_type = genomic DNA
accaggagaggggaatcgtgacga

SEQ ID NO: 56 - DNA, 24 bp, Zea mays
  source 1..24: mol_type = genomic DNA
ttatagcacgacaaaagtaaaaat

SEQ ID NO: 57 - DNA, 24 bp, Zea mays
  source 1..24: mol_type = genomic DNA
attgtcgtcatcatcggctaacat

SEQ ID NO: 58 - DNA, 24 bp, Zea mays
  source 1..24: mol_type = genomic DNA
tactttgacttttcccttaatgac

SEQ ID NO: 59 - DNA, 24 bp, Zea mays
  source 1..24: mol_type = genomic DNA
gggccggtcataaagcagctctca

SEQ ID NO: 60 - DNA, 24 bp, Zea mays
  source 1..24: mol_type = genomic DNA
acggatagcgctcctcgttggcgc

SEQ ID NO: 61 - DNA, 24 bp, Zea mays
  source 1..24: mol_type = genomic DNA
acaatgttagccgatgatgacgac

SEQ ID NO: 62 - DNA, 24 bp, Zea mays
  source 1..24: mol_type = genomic DNA
ggtaaccgtcctccgtacgtcgtc

SEQ ID NO: 63 - DNA, 24 bp, Zea mays
  source 1..24: mol_type = genomic DNA
cctctctacgacgacgtacggagg

SEQ ID NO: 64 - DNA, 24 bp, Zea mays
  source 1..24: mol_type = genomic DNA
gttacgggcagtgcagttgagcaa

SEQ ID NO: 65 - DNA, 24 bp, Zea mays
  source 1..24: mol_type = genomic DNA
ctgactgtccagtggccacctaga

SEQ ID NO: 66 - skipped

SEQ ID NO: 67 - DNA, 1226 bp, synthetic construct
  misc_feature 1..1226: note = p35S+Adh1 intron promoter sequence
  source 1..1226: mol_type = other DNA
gttcagaagaccagagggctattgagacttttcaacaaagggtaatatcgggaaacctcctcggattccattgcccagctatctgtcacttcatcgaaaggacagtagaaaaggaagatggcttctacaaatgccatcattgcgataaaggaaaggctatcgttcaagatgcctctaccgacagtggtcccaaagatggacccccacccacgaggaacatcgtggaaaaagaagacgttccaaccacgtcttcaaagcaagtggattgatgtgatacatggtggagcacgacactctcgtctactccaagaatatcaaagatacagtctcagaagaccagagggctattgagacttttcaacaaagggtaatatcgggaaacctcctcggattccattgcccagctatctgtcacttcatcgaaaggacagtagaaaaggaagatggcttctacaaatgccatcattgcgataaaggaaaggctatcgttcaagatgcctctaccgacagtggtcccaaagatggacccccacccacgaggaacatcgtggaaaaagaagacgttccaaccacgtcttcaaagcaagtggattgatgtgatatctccactgacgtaagggatgacgcacaatcccactatccttcgcaagacccttcctctatataaggaagttcatttcatttggagagggtccgccttgtttctcctctgtctcttgatctgactaatcttggtttatgattcgttgagtaattttggggaaagcttcgtccacagttttttttcgatgaacagtgccgcagtggcgctgatcttgtatgctatcctgcaatcgtggtgaacttatttcttttatatcctttactcccatgaaaaggctagtaatctttctcgatgtaacatcgtccagcactgctattaccgtgtggtccatccgacagtctggctgaacacatcatacgatctatggagcaaaaatctatcttccctgttctttaatgaaggacgtcattttcattagtatgatctaggaatgttgcaacttgcaaggaggcgtttctttctttgaatttaactaactcgttgagtggccctgtttctcggacgtaaggcctttgctgctccacacatgtccattcgaattttaccgtgtttagcaagggcgaaaagtttgcatcttgatgatttagcttgactatgcgattgctttcctggacccgtgcag

SEQ ID NO: 68 - DNA, 5770 bp, synthetic construct
  misc_feature 1..5770: note = pGEP471 mRNA array vector construct
  source 1..5770: mol_type = other DNA
ctgacgcgccctgtagcggcacgtcacctgcatcaggaattcaggagaagaactcgagagggaattgcagatcatgaggcagatggctatttttgtgtcacatatgcgcaaaaagagaggctatatttgtgtccctaggttcttcgttgtattgcagtttccatatcaatctgacttggtcgcatgagaaattgatggttaaataatttgaatctctcatgtagtatcaactattagatattattttcaccaaatatatttccatcggagaagaagaggctacagaggaagcagaagagaggggtgggagaatttttacacttttgtacacccacttaaacagcaaaatccgtatgaaaacaggcccaccaaaacaatgccacgataacaatccgtagaaacaaaagcttcatttaacagcggcgcaacaaagcacgcttatccatggtagttgtagtccgtatgcgatccaaagatcacgattcacgcgtgacggacggacgacgcgtgccacaccacaactaacggcatccatggtagttgtagtccgtatgcgatccaaagatcacgattcacgcgtgacggacggacgacgcgcgccacaccacaactaacagcgtgagccagcgtccaaactccggatggcaacggggacgaaacccgtcgggtagtcactgcccaaacccgtccccgcaaccttcatcccaaacccgtccccgtttccggtcgcgggtttcagttttctaccagacccgtccccatcgggtttttcatccccgtcgggaaatccgaacccgccagcatttcagcaccaagccaaagttgcagcagcaacatgaataaaaaacaacccgtttcaacaccaagataaaacaaaacattataatttagacaacatttcacacgtataacaataacatatagttctcacatataacaacaccatttcacacataaaacaacaccatttgggataaaaatatgggctatatcaggccatttttatgggccatattgagttttcgtgggtttcacaggtaccggatttgtagaatgctgaaccgggtttgaaccgtaaaatccgcgggtattgaatttgacccaatcccgtcgtcccctggtggggtaaaaacaccatcttgagtccaaacggccaccaaccaaactccgacggcaacaaacaaacggcgttgctttgctcctcggtatctccgtgaccgctcaatctcccggctgtttccccggaattgcgtggactctctcatccacacgcaaaccgcctctccctcctctctcgtcctatccgccccggtgccgtagcctcacgggactcttcttcctcccttgctataaaatccccgccccctcctgtctcctctccacacatccaaactctcaatcgcaccgagaaaaatctcctagcgatcgaagcgaagcctctcccgatcctctcaaggtacgcccgtttcccgtcgatcctcctccttccgttcgtgttctgtagccgatcgattcgattcccttacacccgttcgtgttctctcgtggatcgatcgattgtttgttgctagaaggaactcgtagatctggcgtttatgaactgtgattcgggttagtccagatcgattcaggtcggtcgtcgttgagcctctcggctatgtctggattatcgtgtagatctgctggttcagttgattatgttcttctaggagtaatttcgttgggtcagcgcgatttctgcttaatctatgctgcttattgcgcctgtacctatctactaagctatgtgcacctgtaattttgctagattattcgttcatcctcgtagttggtttgtcacagtaatccgtatgggttctgacgatgttattgttggtcatacctaggcttctccagattttattttgttaaaattggatagatctgctactgatagttgatgatggaatttggtgctgaatctatgctatttattgcgcctatacctgatctatcgggctatgtacggctgtagtttactggattattcgttcatcctcggtagttggttcatcgtttgggttctgacgataatattgttgattatgcgtaggcttctgcagattgttgttaaaattggatacatcggttactgatggttgatgatagatttgtgctgaacctatctgtttattgctcctatacctgatctatagggctatgtatgcctgtaatttaccagattattcgttcatcctcgtagttggttcatctctataattcgtatgggttcttatgatgttatcgttgattatgcctagtcttatacagattattgtgtcaagattgaatatacctgctactgatcggtgataatttggttagtagtttgcaatctgctaggaacacgttaccactgtaatctgtaaacatggtttgccagagtagtttgttctactactcttgatatggttgctgattttagtcgcctccttttggatcatgtattgatgtccttgcagatttccgtgtacttaccccggcttttgtgtacttcgtgttaacagctctagaggatcctctcaacacaacatatacaaaacaaacgaatctcaagcaatcaagcattctacttctattgcagcaatttaaatcatttcttttaaagcaaaagcaattttctgaaaattttcaccatttacgaacgatagggcgcgatcccgccaccatggtgagcaagggcgaggaggtcatcaaagagttcatgcgcttcaaggtgcgcatggagggctccatgaacggccacgagttcgagatcgagggcgagggcgagggccgcccctacgagggcacccagaccgccaagctgaaggtgaccaagggcggccccctgcccttcgcctgggacatcctgtccccccagttcatgtacggctccaaggcgtacgtgaagcaccccgccgacatccccgattacaagaagctgtccttccccgagggcttcaagtgggagcgcgtgatgaacttcgaggacggcggtctggtgaccgtgacccaggactcctccctgcaggacggcacgctgatctacaaggtgaagatgcgcggcaccaacttcccccccgacggccccgtaatgcagaagaagaccatgggctgggaggcctccaccgagcgcctgtacccccgcgacggcgtgctgaagggcgagatccaccaggccctgaagctgaaggacggcggccactacctggtggagttcaagaccatctacatggccaagaagcccgtgcaactgcccggctactactacgtggacaccaagctggacatcacctcccacaacgaggactacaccatcgtggaacagtacgagcgctccgagggccgccaccacctgttcctgtacggcatggacgagctgtacaagtctagaggtacctgataatttctactaagtgtagatctcgtcacgattcccctctcctggaatttctactcttgtagattgtgtggtcacacttgccagccagaatttctactcttgtagatgtctatgtcgatgaccagcagattaatttctactaagtgtagatcgaatttccccgatcgttcaaacatttggcaataaagtttcttaagattgaatcctgttgccggtcttgcgatgattatcatataatttctgttgaattacgttaagcatgtaataattaacatgtaatgcatgacgttatttatgagatgggtttttatgattagagtcccgcaattatacatttaatacgcgatagaaaacaaaatatagcgcgcaaactaggataaattatcgcgcgcggtgtcatctatgttactagatcgctcgacgcggccgccatggcctctagtggatcaggtgtcgttcggctgcggcgagcggtatcagctcactcaaaggcggtaatacggttatccacagaatcaggggataacgcaggaaagaacatgtgagcaaaaggccagcaaaaggccaggaaccgtaaaaaggccgcgttgctggcgtttttccataggctccgcccccctgacgagcatcacaaaaatcgacgctcaagtcagaggtggcgaaacccgacaggactataaagataccaggcgtttccccctggaagctccctcgtgcgctctcctgttccgaccctgccgcttaccggatacctgtccgcctttctcccttcgggaagcgtggcgctttctcatagctcacgctgtaggtatctcagttcggtgtaggtcgttcgctccaagctgggctgtgtgcacgaaccccccgttcagcccgaccgctgcgccttatccggtaactatcgtcttgagtccaacccggtaagacacgacttatcgccactggcagcagccactggtaacaggattagcagagcgaggtatgtaggcggtgctacagagttcttgaagtggtggcctaactacggctacactagaaggacagtatttggtatctgcgctctgctgaagccagttaccttcggaaaaagagttggtagctcttgatccggcaaacaaaccaccgctggtagcggtggtttttttgtttgcaagcagcagattacgcgcagaaaaaaaggatctcaagaagatcctttgatcttttctacggggtctgacgctcagtggaacgaaaactcacgttaagggattttggtcatgagattatcaaaaaggatcttcacctagatccttttaaattaaaaatgaagttttaaatcaatctaaagtatatatgagtaaacttggtctgacagttaccaatgcttaatcagtgaggcacctatctcagcgatctgtctatttcgttcatccatagttgcctgactccccgtcgtgtagataactacgatacgggagggcttaccatctggccccagtgctgcaatgataccgcgagacccacgctcaccggctccagatttatcagcaataaaccagccagccggaagggccgagcgcagaagtggtcctgcaactttatccgcctccatccagtctattaattgttgccgggaagctagagtaagtagttcgccagttaatagtttgcgcaacgttgttgccattgctacaggcatcgtggtgtcacgctcgtcgtttggtatggcttcattcagctccggttcccaacgatcaaggcgagttacatgatcccccatgttgtgcaaaaaagcggttagctccttcggtcctccgatcgttgtcagaagtaagttggccgcagtgttatcactcatggttatggcagcactgcataattctcttactgtcatgccatccgtaagatgcttttctgtgactggtgagtactcaaccaagtcattctgagaatagtgtatgcggcgaccgagttgctcttgcccggcgtcaatacgggataataccgcgccacatagcagaactttaaaagtgctcatcattggaaaacgttcttcggggcgaaaactctcaaggatcttaccgctgttgagatccagttcgatgtaacccactcgtgcacccaactgatcttcagcatcttttactttcaccagcgtttctgggtgagcaaaaacaggaaggcaaaatgccgcaaaaaagggaataagggcgacacggaaatgttgaatactcatactcttcctttttcaatattattgaagcatttatcagggttattgtctcatgagcggatacatatttgaatgtatttagaaaaataaacaaataggggttccgcgcacatttccccgaaaagtgccac

SEQ ID NO: 69 - DNA, 5770 bp, synthetic construct
  misc_feature 1..5770: note = pGEP472 mRNA array vector construct
  source 1..5770: mol_type = other DNA
ctgacgcgccctgtagcggcacgtcacctgcatcaggaattcaggagaagaactcgagagggaattgcagatcatgaggcagatggctatttttgtgtcacatatgcgcaaaaagagaggctatatttgtgtccctaggttcttcgttgtattgcagtttccatatcaatctgacttggtcgcatgagaaattgatggttaaataatttgaatctctcatgtagtatcaactattagatattattttcaccaaatatatttccatcggagaagaagaggctacagaggaagcagaagagaggggtgggagaatttttacacttttgtacacccacttaaacagcaaaatccgtatgaaaacaggcccaccaaaacaatgccacgataacaatccgtagaaacaaaagcttcatttaacagcggcgcaacaaagcacgcttatccatggtagttgtagtccgtatgcgatccaaagatcacgattcacgcgtgacggacggacgacgcgtgccacaccacaactaacggcatccatggtagttgtagtccgtatgcgatccaaagatcacgattcacgcgtgacggacggacgacgcgcgccacaccacaactaacagcgtgagccagcgtccaaactccggatggcaacggggacgaaacccgtcgggtagtcactgcccaaacccgtccccgcaaccttcatcccaaacccgtccccgtttccggtcgcgggtttcagttttctaccagacccgtccccatcgggtttttcatccccgtcgggaaatccgaacccgccagcatttcagcaccaagccaaagttgcagcagcaacatgaataaaaaacaacccgtttcaacaccaagataaaacaaaacattataatttagacaacatttcacacgtataacaataacatatagttctcacatataacaacaccatttcacacataaaacaacaccatttgggataaaaatatgggctatatcaggccatttttatgggccatattgagttttcgtgggtttcacaggtaccggatttgtagaatgctgaaccgggtttgaaccgtaaaatccgcgggtattgaatttgacccaatcccgtcgtcccctggtggggtaaaaacaccatcttgagtccaaacggccaccaaccaaactccgacggcaacaaacaaacggcgttgctttgctcctcggtatctccgtgaccgctcaatctcccggctgtttccccggaattgcgtggactctctcatccacacgcaaaccgcctctccctcctctctcgtcctatccgccccggtgccgtagcctcacgggactcttcttcctcccttgctataaaatccccgccccctcctgtctcctctccacacatccaaactctcaatcgcaccgagaaaaatctcctagcgatcgaagcgaagcctctcccgatcctctcaaggtacgcccgtttcccgtcgatcctcctccttccgttcgtgttctgtagccgatcgattcgattcccttacacccgttcgtgttctctcgtggatcgatcgattgtttgttgctagaaggaactcgtagatctggcgtttatgaactgtgattcgggttagtccagatcgattcaggtcggtcgtcgttgagcctctcggctatgtctggattatcgtgtagatctgctggttcagttgattatgttcttctaggagtaatttcgttgggtcagcgcgatttctgcttaatctatgctgcttattgcgcctgtacctatctactaagctatgtgcacctgtaattttgctagattattcgttcatcctcgtagttggtttgtcacagtaatccgtatgggttctgacgatgttattgttggtcatacctaggcttctccagattttattttgttaaaattggatagatctgctactgatagttgatgatggaatttggtgctgaatctatgctatttattgcgcctatacctgatctatcgggctatgtacggctgtagtttactggattattcgttcatcctcggtagttggttcatcgtttgggttctgacgataatattgttgattatgcgtaggcttctgcagattgttgttaaaattggatacatcggttactgatggttgatgatagatttgtgctgaacctatctgtttattgctcctatacctgatctatagggctatgtatgcctgtaatttaccagattattcgttcatcctcgtagttggttcatctctataattcgtatgggttcttatgatgttatcgttgattatgcctagtcttatacagattattgtgtcaagattgaatatacctgctactgatcggtgataatttggttagtagtttgcaatctgctaggaacacgttaccactgtaatctgtaaacatggtttgccagagtagtttgttctactactcttgatatggttgctgattttagtcgcctccttttggatcatgtattgatgtccttgcagatttccgtgtacttaccccggcttttgtgtacttcgtgttaacagctctagaggatcctctcaacacaacatatacaaaacaaacgaatctcaagcaatcaagcattctacttctattgcagcaatttaaatcatttcttttaaagcaaaagcaattttctgaaaattttcaccatttacgaacgatagggcgcgatcccgccaccatggtgagcaagggcgaggaggtcatcaaagagttcatgcgcttcaaggtgcgcatggagggctccatgaacggccacgagttcgagatcgagggcgagggcgagggccgcccctacgagggcacccagaccgccaagctgaaggtgaccaagggcggccccctgcccttcgcctgggacatcctgtccccccagttcatgtacggctccaaggcgtacgtgaagcaccccgccgacatccccgattacaagaagctgtccttccccgagggcttcaagtgggagcgcgtgatgaacttcgaggacggcggtctggtgaccgtgacccaggactcctccctgcaggacggcacgctgatctacaaggtgaagatgcgcggcaccaacttcccccccgacggccccgtaatgcagaagaagaccatgggctgggaggcctccaccgagcgcctgtacccccgcgacggcgtgctgaagggcgagatccaccaggccctgaagctgaaggacggcggccactacctggtggagttcaagaccatctacatggccaagaagcccgtgcaactgcccggctactactacgtggacaccaagctggacatcacctcccacaacgaggactacaccatcgtggaacagtacgagcgctccgagggccgccaccacctgttcctgtacggcatggacgagctgtacaagtctagaggtacctgataatttctactaagtgtagatgtctatgtcgatgaccagcagataatttctactcttgtagatctcgtcacgattcccctctcctggaatttctactcttgtagattgtgtggtcacacttgccagccagtaatttctactaagtgtagatcgaatttccccgatcgttcaaacatttggcaataaagtttcttaagattgaatcctgttgccggtcttgcgatgattatcatataatttctgttgaattacgttaagcatgtaataattaacatgtaatgcatgacgttatttatgagatgggtttttatgattagagtcccgcaattatacatttaatacgcgatagaaaacaaaatatagcgcgcaaactaggataaattatcgcgcgcggtgtcatctatgttactagatcgctcgacgcggccgccatggcctctagtggatcaggtgtcgttcggctgcggcgagcggtatcagctcactcaaaggcggtaatacggttatccacagaatcaggggataacgcaggaaagaacatgtgagcaaaaggccagcaaaaggccaggaaccgtaaaaaggccgcgttgctggcgtttttccataggctccgcccccctgacgagcatcacaaaaatcgacgctcaagtcagaggtggcgaaacccgacaggactataaagataccaggcgtttccccctggaagctccctcgtgcgctctcctgttccgaccctgccgcttaccggatacctgtccgcctttctcccttcgggaagcgtggcgctttctcatagctcacgctgtaggtatctcagttcggtgtaggtcgttcgctccaagctgggctgtgtgcacgaaccccccgttcagcccgaccgctgcgccttatccggtaactatcgtcttgagtccaacccggtaagacacgacttatcgccactggcagcagccactggtaacaggattagcagagcgaggtatgtaggcggtgctacagagttcttgaagtggtggcctaactacggctacactagaaggacagtatttggtatctgcgctctgctgaagccagttaccttcggaaaaagagttggtagctcttgatccggcaaacaaaccaccgctggtagcggtggtttttttgtttgcaagcagcagattacgcgcagaaaaaaaggatctcaagaagatcctttgatcttttctacggggtctgacgctcagtggaacgaaaactcacgttaagggattttggtcatgagattatcaaaaaggatcttcacctagatccttttaaattaaaaatgaagttttaaatcaatctaaagtatatatgagtaaacttggtctgacagttaccaatgcttaatcagtgaggcacctatctcagcgatctgtctatttcgttcatccatagttgcctgactccccgtcgtgtagataactacgatacgggagggcttaccatctggccccagtgctgcaatgataccgcgagacccacgctcaccggctccagatttatcagcaataaaccagccagccggaagggccgagcgcagaagtggtcctgcaactttatccgcctccatccagtctattaattgttgccgggaagctagagtaagtagttcgccagttaatagtttgcgcaacgttgttgccattgctacaggcatcgtggtgtcacgctcgtcgtttggtatggcttcattcagctccggttcccaacgatcaaggcgagttacatgatcccccatgttgtgcaaaaaagcggttagctccttcggtcctccgatcgttgtcagaagtaagttggccgcagtgttatcactcatggttatggcagcactgcataattctcttactgtcatgccatccgtaagatgcttttctgtgactggtgagtactcaaccaagtcattctgagaatagtgtatgcggcgaccgagttgctcttgcccggcgtcaatacgggataataccgcgccacatagcagaactttaaaagtgctcatcattggaaaacgttcttcggggcgaaaactctcaaggatcttaccgctgttgagatccagttcgatgtaacccactcgtgcacccaactgatcttcagcatcttttactttcaccagcgtttctgggtgagcaaaaacaggaaggcaaaatgccgcaaaaaagggaataagggcgacacggaaatgttgaatactcatactcttcctttttcaatattattgaagcatttatcagggttattgtctcatgagcggatacatatttgaatgtatttagaaaaataaacaaataggggttccgcgcacatttccccgaaaagtgccac

SEQ ID NO: 70 - DNA, 3938 bp, synthetic construct
  misc_feature 1..3938: note = pGEP473 ribozyme array vector construct
  source 1..3938: mol_type = other DNA
ctgacgcgccctgtagcggcctgcagtgcagcgtgacccggtcgtgcccctctctagagataatgagcattgcatgtctaagttataaaaaattaccacatattttttttgtcacacttgtttgaagtgcagtttatctatctttatacatatatttaaactttactctacgaataatataatctatagtactacaataatatcagtgttttagagaatcatataaatgaacagttagacatggtctaaaggacaattgagtattttgacaacaggactctacagttttatctttttagtgtgcatgtgttctcctttttttttgcaaatagcttcacctatataatacttcatccattttattagtacatccatttagggtttagggttaatggtttttatagactaatttttttagtacatctattttattctattttagcctctaaattaagaaaactaaaactctattttagtttttttatttaataatttagatataaaatagaataaaataaagtgactaaaaattaaacaaataccctttaagaaattaaaaaaactaaggaaacatttttcttgtttcgagtagataatgccagcctgttaaacgccgtcgatcgacgagtctaacggacaccaaccagcgaaccagcagcgtcgcgtcgggccaagcgaagcagacggcacggcatctctgtcgctgcctctggacccctctcgagagttccgctccaccgttggacttgctccgctgtcggcatccagaaattgcgtggcggagcggcagacgtgagccggcacggcaggcggcctcctcctcctctcacggcaccggcagctacgggggattcctttcccaccgctccttcgctttcccttcctcgcccgccgtaataaatagacaccccctccacaccctctttccccaacctcgtgttgttcggagcgcacacacacacaaccagatctcccccaaatccacccgtcggcacctccgcttcaaggtacgccgctcgtcctccccccccccccctctctaccttctctagatcggcgttccggtccatggttagggcccggtagttctacttctgttcatgtttgtgttagatccgtgtttgtgttagatccgtgctgctagcgttcgtacacggatgcgacctgtacgtcagacacgttctgattgctaacttgccagtgtttctctttggggaatcctgggatggctctagccgttccgcagacgggatcgatctaggataggtatacatgttgatgtgggttttactgatgcatatacatgatggcatatgcagcatctattcatatgctctaaccttgagtacctatctattataataaacaagtatgttttataattattttgatcttgatatacttggatgatggcatatgcagcagctatatgtggatttttttagccctgccttcatacgctatttatttgcttggtactgtttcttttgtcgatgctcaccctgttgtttggtgttacttctgcagggatccaaattactgatgagtccgtgaggacgaaacgagtaagctcgtctaatttctactaagtgtagatctcgtcacgattcccctctcctggaatttctactcttgtagattgtgtggtcacacttgccagccagaatttctactcttgtagatgtctatgtcgatgaccagcagatggcgtcagtcctactctgcacctcctcgtggtgtcgcctgggaaccctctttcacaagaaagaggagccaagcagagaggcgatcgttcaaacatttggcaataaagtttcttaagattgaatcctgttgccggtcttgcgatgattatcatataatttctgttgaattacgttaagcatgtaataattaacatgtaatgcatgacgttatttatgagatgggtttttatgattagagtcccgcaattatacatttaatacgcgatagaaaacaaaatatagcgcgcaaactaggataaattatcgcgcgcggtgtcatctatgttactagatcgatcgtcgttcggctgcggcgagcggtatcagctcactcaaaggcggtaatacggttatccacagaatcaggggataacgcaggaaagaacatgtgagcaaaaggccagcaaaaggccaggaaccgtaaaaaggccgcgttgctggcgtttttccataggctccgcccccctgacgagcatcacaaaaatcgacgctcaagtcagaggtggcgaaacccgacaggactataaagataccaggcgtttccccctggaagctccctcgtgcgctctcctgttccgaccctgccgcttaccggatacctgtccgcctttctcccttcgggaagcgtggcgctttctcatagctcacgctgtaggtatctcagttcggtgtaggtcgttcgctccaagctgggctgtgtgcacgaaccccccgttcagcccgaccgctgcgccttatccggtaactatcgtcttgagtccaacccggtaagacacgacttatcgccactggcagcagccactggtaacaggattagcagagcgaggtatgtaggcggtgctacagagttcttgaagtggtggcctaactacggctacactagaagaacagtatttggtatctgcgctctgctgaagccagttaccttcggaaaaagagttggtagctcttgatccggcaaacaaaccaccgctggtagcggtggtttttttgtttgcaagcagcagattacgcgcagaaaaaaaggatctcaagaagatcctttgatcttttctacggggtctgacgctcagtggaacgaaaactcacgttaagggattttggtcatgagattatcaaaaaggatcttcacctagatccttttaaattaaaaatgaagttttaaatcaatctaaagtatatatgagtaaacttggtctgacagttaccaatgcttaatcagtgaggcacctatctcagcgatctgtctatttcgttcatccatagttgcctgactccccgtcgtgtagataactacgatacgggagggcttaccatctggccccagtgctgcaatgataccgcgagacccacgctcaccggctccagatttatcagcaataaaccagccagccggaagggccgagcgcagaagtggtcctgcaactttatccgcctccatccagtctattaattgttgccgggaagctagagtaagtagttcgccagttaatagtttgcgcaacgttgttgccattgctacaggcatcgtggtgtcacgctcgtcgtttggtatggcttcattcagctccggttcccaacgatcaaggcgagttacatgatcccccatgttgtgcaaaaaagcggttagctccttcggtcctccgatcgttgtcagaagtaagttggccgcagtgttatcactcatggttatggcagcactgcataattctcttactgtcatgccatccgtaagatgcttttctgtgactggtgagtactcaaccaagtcattctgagaatagtgtatgcggcgaccgagttgctcttgcccggcgtcaatacgggataataccgcgccacatagcagaactttaaaagtgctcatcattggaaaacgttcttcggggcgaaaactctcaaggatcttaccgctgttgagatccagttcgatgtaacccactcgtgcacccaactgatcttcagcatcttttactttcaccagcgtttctgggtgagcaaaaacaggaaggcaaaatgccgcaaaaaagggaataagggcgacacggaaatgttgaatactcatactcttcctttttcaatattattgaagcatttatcagggttattgtctcatgagcggatacatatttgaatgtatttagaaaaataaacaaataggggttccgcgcacatttccccgaaaagtgccac

SEQ ID NO: 71 - DNA, 3938 bp, synthetic construct
  misc_feature 1..3938: note = pGEP474 ribozyme array vector construct
  source 1..3938: mol_type = other DNA
ctgacgcgccctgtagcggcctgcagtgcagcgtgacccggtcgtgcccctctctagagataatgagcattgcatgtctaagttataaaaaattaccacatattttttttgtcacacttgtttgaagtgcagtttatctatctttatacatatatttaaactttactctacgaataatataatctatagtactacaataatatcagtgttttagagaatcatataaatgaacagttagacatggtctaaaggacaattgagtattttgacaacaggactctacagttttatctttttagtgtgcatgtgttctcctttttttttgcaaatagcttcacctatataatacttcatccattttattagtacatccatttagggtttagggttaatggtttttatagactaatttttttagtacatctattttattctattttagcctctaaattaagaaaactaaaactctattttagtttttttatttaataatttagatataaaatagaataaaataaagtgactaaaaattaaacaaataccctttaagaaattaaaaaaactaaggaaacatttttcttgtttcgagtagataatgccagcctgttaaacgccgtcgatcgacgagtctaacggacaccaaccagcgaaccagcagcgtcgcgtcgggccaagcgaagcagacggcacggcatctctgtcgctgcctctggacccctctcgagagttccgctccaccgttggacttgctccgctgtcggcatccagaaattgcgtggcggagcggcagacgtgagccggcacggcaggcggcctcctcctcctctcacggcaccggcagctacgggggattcctttcccaccgctccttcgctttcccttcctcgcccgccgtaataaatagacaccccctccacaccctctttccccaacctcgtgttgttcggagcgcacacacacacaaccagatctcccccaaatccacccgtcggcacctccgcttcaaggtacgccgctcgtcctccccccccccccctctctaccttctctagatcggcgttccggtccatggttagggcccggtagttctacttctgttcatgtttgtgttagatccgtgtttgtgttagatccgtgctgctagcgttcgtacacggatgcgacctgtacgtcagacacgttctgattgctaacttgccagtgtttctctttggggaatcctgggatggctctagccgttccgcagacgggatcgatctaggataggtatacatgttgatgtgggttttactgatgcatatacatgatggcatatgcagcatctattcatatgctctaaccttgagtacctatctattataataaacaagtatgttttataattattttgatcttgatatacttggatgatggcatatgcagcagctatatgtggatttttttagccctgccttcatacgctatttatttgcttggtactgtttcttttgtcgatgctcaccctgttgtttggtgttacttctgcagggatccaaattactgatgagtccgtgaggacgaaacgagtaagctcgtctaatttctactaagtgtagatgtctatgtcgatgaccagcagataatttctactcttgtagatctcgtcacgattcccctctcctggaatttctactcttgtagattgtgtggtcacacttgccagccagggcgtcagtcctactctgcacctcctcgtggtgtcgcctgggaaccctctttcacaagaaagaggagccaagcagagaggcgatcgttcaaacatttggcaataaagtttcttaagattgaatcctgttgccggtcttgcgatgattatcatataatttctgttgaattacgttaagcatgtaataattaacatgtaatgcatgacgttatttatgagatgggtttttatgattagagtcccgcaattatacatttaatacgcgatagaaaacaaaatatagcgcgcaaactaggataaattatcgcgcgcggtgtcatctatgttactagatcgatcgtcgttcggctgcggcgagcggtatcagctcactcaaaggcggtaatacggttatccacagaatcaggggataacgcaggaaagaacatgtgagcaaaaggccagcaaaaggccaggaaccgtaaaaaggccgcgttgctggcgtttttccataggctccgcccccctgacgagcatcacaaaaatcgacgctcaagtcagaggtggcgaaacccgacaggactataaagataccaggcgtttccccctggaagctccctcgtgcgctctcctgttccgaccctgccgcttaccggatacctgtccgcctttctcccttcgggaagcgtggcgctttctcatagctcacgctgtaggtatctcagttcggtgtaggtcgttcgctccaagctgggctgtgtgcacgaaccccccgttcagcccgaccgctgcgccttatccggtaactatcgtcttgagtccaacccggtaagacacgacttatcgccactggcagcagccactggtaacaggattagcagagcgaggtatgtaggcggtgctacagagttcttgaagtggtggcctaactacggctacactagaagaacagtatttggtatctgcgctctgctgaagccagttaccttcggaaaaagagttggtagctcttgatccggcaaacaaaccaccgctggtagcggtggtttttttgtttgcaagcagcagattacgcgcagaaaaaaaggatctcaagaagatcctttgatcttttctacggggtctgacgctcagtggaacgaaaactcacgttaagggattttggtcatgagattatcaaaaaggatcttcacctagatccttttaaattaaaaatgaagttttaaatcaatctaaagtatatatgagtaaacttggtctgacagttaccaatgcttaatcagtgaggcacctatctcagcgatctgtctatttcgttcatccatagttgcctgactccccgtcgtgtagataactacgatacgggagggcttaccatctggccccagtgctgcaatgataccgcgagacccacgctcaccggctccagatttatcagcaataaaccagccagccggaagggccgagcgcagaagtggtcctgcaactttatccgcctccatccagtctattaattgttgccgggaagctagagtaagtagttcgccagttaatagtttgcgcaacgttgttgccattgctacaggcatcgtggtgtcacgctcgtcgtttggtatggcttcattcagctccggttcccaacgatcaaggcgagttacatgatcccccatgttgtgcaaaaaagcggttagctccttcggtcctccgatcgttgtcagaagtaagttggccgcagtgttatcactcatggttatggcagcactgcataattctcttactgtcatgccatccgtaagatgcttttctgtgactggtgagtactcaaccaagtcattctgagaatagtgtatgcggcgaccgagttgctcttgcccggcgtcaatacgggataataccgcgccacatagcagaactttaaaagtgctcatcattggaaaacgttcttcggggcgaaaactctcaaggatcttaccgctgttgagatccagttcgatgtaacccactcgtgcacccaactgatcttcagcatcttttactttcaccagcgtttctgggtgagcaaaaacaggaaggcaaaatgccgcaaaaaagggaataagggcgacacggaaatgttgaatactcatactcttcctttttcaatattattgaagcatttatcagggttattgtctcatgagcggatacatatttgaatgtatttagaaaaataaacaaataggggttccgcgcacatttccccgaaaagtgccac

SEQ ID NO: 72 - DNA, 3759 bp, synthetic construct
  misc_feature 1..3759: note = codon optimized LbCpf1
  source 1..3759: mol_type = other DNA
atggcgccgaagaagaagcgcaaggtgtccaagctcgagaagttcacgaactgctactccctctccaagaccctccgcttcaaggccatccccgtgggcaagacccaggagaacatcgacaacaagcgcctcctggtcgaggacgagaagagggcggaggactacaagggcgtgaagaagctcctggaccgctactacctctccttcatcaacgacgtcctgcacagcatcaagctcaagaacctgaacaactacatctccctgttccgcaagaagacgaggaccgagaaggagaacaaggagctcgagaacctggagatcaacctccgcaaggagatcgccaaggcgttcaagggcaacgagggctacaagagcctgttcaagaaggacatcatcgagacgatcctcccggagttcctggacgacaaggacgagatcgccctcgtgaactccttcaacggcttcaccacggcgttcaccggcttcttcgacaaccgcgagaacatgttcagcgaggaggccaagtccacgagcatcgcgttccgctgcatcaacgagaacctgaccaggtacatctccaacatggacatcttcgagaaggtcgacgccatcttcgacaagcacgaggtgcaggagatcaaggagaagatcctcaacagcgactacgacgtcgaggacttcttcgagggcgagttcttcaacttcgtcctgacgcaggagggcatcgacgtgtacaacgccatcatcggtggcttcgtgaccgagtccggcgagaagatcaagggcctcaacgagtacatcaacctgtacaaccagaagaccaagcagaagctcccgaagttcaagcccctctacaagcaggtcctgtccgaccgcgagtccctgagcttctacggcgagggctacacgagcgacgaggaggtcctcgaggtgttcaggaacaccctgaacaagaacagcgagatcttctccagcatcaagaagctcgagaagctgttcaagaacttcgacgagtactccagcgccggcatcttcgtcaagaacggcccggcgatctccacgatcagcaaggatatcttcggcgagtggaacgtgatcagggacaagtggaacgccgagtacgacgacatccacctcaagaagaaggcggtggtcaccgagaagtacgaggacgaccgcaggaagtccttcaagaagatcggctccttcagcctcgagcagctgcaggagtacgccgacgcggacctctccgtggtcgagaagctgaaggagatcatcatccagaaggtcgacgagatctacaaggtgtacggctccagcgagaagctgttcgacgccgacttcgtcctcgagaagtccctgaagaagaacgacgccgtggtcgcgatcatgaaggacctcctggactccgtgaagagcttcgagaactacatcaaggcgttcttcggcgagggcaaggagacgaaccgcgacgagtccttctacggcgacttcgtcctcgcctacgacatcctcctgaaggtggaccacatctacgacgcgatcaggaactacgtgacccagaagccgtacagcaaggacaagttcaagctgtacttccagaacccccagttcatgggcggctgggacaaggacaaggagacggactaccgcgccaccatcctccgctacggcagcaagtactacctggccatcatggacaagaagtacgcgaagtgcctccagaagatcgacaaggacgacgtcaacggcaactacgagaagatcaactacaagctcctgccgggccccaacaagatgctgccgaaggtgttcttctccaagaagtggatggcctactacaaccccagcgaggacatccagaagatctacaagaacggcacgttcaagaagggcgacatgttcaacctcaacgactgccacaagctgatcgacttcttcaaggactccatcagccgctacccgaagtggtccaacgcctacgacttcaacttcagcgagacagagaagtacaaggacatcgcgggcttctacagggaggtcgaggagcagggctacaaggtgtccttcgagtccgccagcaagaaggaggtcgacaagctcgtggaggagggcaagctgtacatgttccagatctacaacaaggacttctccgacaagagccacggcacgcccaacctccacaccatgtacttcaagctcctgttcgacgagaacaaccacggccagatccgcctctccggcggcgccgagctgttcatgaggagggcgagcctcaagaaggaggagctggtggtccaccccgctaacagcccaatcgcgaacaagaacccggacaaccccaagaagaccacgaccctctcctacgacgtgtacaaggacaagcgcttcagcgaggaccagtacgagctgcacatcccgatcgccatcaacaagtgccccaagaacatcttcaagatcaacaccgaggtcagggtgctcctgaagcacgacgacaacccctacgtgatcggcatcgaccgcggcgagaggaacctcctgtacatcgtggtcgtggacggcaagggcaacatcgtggagcagtactccctgaacgagatcatcaacaacttcaacggcatccgcatcaagacggactaccacagcctcctggacaagaaggagaaggagcgcttcgaggccaggcagaactggacctccatcgagaacatcaaggagctcaaggcgggctacatcagccaggtcgtgcacaagatctgcgagctggtcgagaagtacgacgccgtgatcgcgctcgaggacctgaactccggcttcaagaacagcagggtcaaggtggagaagcaggtctaccagaagttcgagaagatgctcatcgacaagctgaactacatggtggacaagaagtccaacccgtgcgctacgggcggcgcgctcaagggctaccagatcaccaacaagttcgagagcttcaagtccatgagcacccagaacggcttcatcttctacatcccggcctggctgacgtccaagatcgaccccagcaccggcttcgtcaacctcctgaagacgaagtacacctccatcgcggacagcaagaagttcatctccagcttcgaccgcatcatgtatgtgccggaggaggacctcttcgagttcgccctggactacaagaacttctccaggacggacgcggattacatcaagaagtggaagctctacagctacggcaaccgcatcaggatcttccgcaaccccaagaagaacaacgtcttcgactgggaggaggtgtgcctcacctccgcctacaaggagctgttcaacaagtacggcatcaactaccagcagggcgacatcagggcgctcctgtgcgagcagagcgacaaggccttctactccagcttcatggcgctcatgtccctcatgctgcagatgcgcaacagcatcacgggcaggaccgacgtcgacttcctgatctccccggtgaagaacagcgacggcatcttctacgacagccgcaactacgaggcccaggagaacgcgatcctgccaaagaacgcggacgccaacggcgcctacaacatcgcgaggaaggtgctgtgggccatcggccagttcaagaaggcggaggacgagaagctcgacaaggtcaagatcgccatctccaacaaggagtggctggagtacgcgcagacctcggtgaagcacaagaggcccgctgccaccaagaaggcgggccaggccaagaagaagaagtga

SEQ ID NO: 73 - DNA, 3759 bp, synthetic construct
  misc_feature 1..3759: note = codon optimimized LbCpf1
  source 1..3759: mol_type = other DNA
atggcccccaagaagaagcgcaaggtgagcaagctggagaagtttacaaactgctactccctgtctaagactctgcgcttcaaggccatccctgtgggcaagacccaggagaacatcgacaataagcggctgctggtggaggacgagaagagagccgaggattataagggcgtgaagaagctgctggatcgctactatctgtcttttatcaacgacgtgctgcacagcatcaagctgaagaatctgaacaattacatcagcctgttccggaagaaaaccagaaccgagaaggagaataaggagctggagaacctggagatcaatctgcggaaggagatcgccaaggccttcaagggcaacgagggctacaagtccctgtttaagaaggatatcatcgagacaatcctgccagagttcctggacgataaggacgagatcgccctggtgaacagcttcaatggctttaccacagccttcaccggcttctttgataacagagagaatatgttttccgaggaggccaagagcacatccatcgccttcaggtgtatcaacgagaatctgacccgctacatctctaatatggacatcttcgagaaggtggacgccatctttgataagcacgaggtgcaggagatcaaggagaagatcctgaacagcgactatgatgtggaggatttctttgagggcgagttctttaactttgtgctgacacaggagggcatcgacgtgtataacgccatcatcggcggcttcgtgaccgagagcggcgagaagatcaagggcctgaacgagtacatcaacctgtataatcagaaaaccaagcagaagctgcctaagtttaagccactgtataagcaggtgctgagcgatcgggagtctctgagcttctacggcgagggctatacatccgatgaggaggtgctggaggtgtttagaaacaccctgaacaagaacagcgagatcttcagctccatcaagaagctggagaagctgttcaagaattttgacgagtactctagcgccggcatctttgtgaagaacggccccgccatcagcacaatctccaaggatatcttcggcgagtggaacgtgatccgggacaagtggaatgccgagtatgacgatatccacctgaagaagaaggccgtggtgaccgagaagtacgaggacgatcggagaaagtccttcaagaagatcggctccttttctctggagcagctgcaggagtacgccgacgccgatctgtctgtggtggagaagctgaaggagatcatcatccagaaggtggatgagatctacaaggtgtatggctcctctgagaagctgttcgacgccgattttgtgctggagaagagcctgaagaagaacgacgccgtggtggccatcatgaaggacctgctggattctgtgaagagcttcgagaattacatcaaggccttctttggcgagggcaaggagacaaacagggacgagtccttctatggcgattttgtgctggcctacgacatcctgctgaaggtggaccacatctacgatgccatccgcaattatgtgacccagaagccctactctaaggataagttcaagctgtattttcagaaccctcagttcatgggcggctgggacaaggataaggagacagactatcgggccaccatcctgagatacggctccaagtactatctggccatcatggataagaagtacgccaagtgcctgcagaagatcgacaaggacgatgtgaacggcaattacgagaagatcaactataagctgctgcccggccctaataagatgctgccaaaggtgttcttttctaagaagtggatggcctactataaccccagcgaggacatccagaagatctacaagaatggcacattcaagaagggcgatatgtttaacctgaatgactgtcacaagctgatcgacttctttaaggatagcatctcccggtatccaaagtggtccaatgcctacgatttcaacttttctgagacagagaagtataaggacatcgccggcttttacagagaggtggaggagcagggctataaggtgagcttcgagtctgccagcaagaaggaggtggataagctggtggaggagggcaagctgtatatgttccagatctataacaaggacttttccgataagtctcacggcacacccaatctgcacaccatgtacttcaagctgctgtttgacgagaacaatcacggacagatcaggctgagcggaggagcagagctgttcatgaggcgcgcctccctgaagaaggaggagctggtggtgcacccagccaactcccctatcgccaacaagaatccagataatcccaagaaaaccacaaccctgtcctacgacgtgtataaggataagaggttttctgaggaccagtacgagctgcacatcccaatcgccatcaataagtgccccaagaacatcttcaagatcaatacagaggtgcgcgtgctgctgaagcacgacgataacccctatgtgatcggcatcgataggggcgagcgcaatctgctgtatatcgtggtggtggacggcaagggcaacatcgtggagcagtattccctgaacgagatcatcaacaacttcaacggcatcaggatcaagacagattaccactctctgctggacaagaaggagaaggagaggttcgaggcccgccagaactggacctccatcgagaatatcaaggagctgaaggccggctatatctctcaggtggtgcacaagatctgcgagctggtggagaagtacgatgccgtgatcgccctggaggacctgaactctggctttaagaatagccgcgtgaaggtggagaagcaggtgtatcagaagttcgagaagatgctgatcgataagctgaactacatggtggacaagaagtctaatccttgtgcaacaggcggcgccctgaagggctatcagatcaccaataagttcgagagctttaagtccatgtctacccagaacggcttcatcttttacatccctgcctggctgacatccaagatcgatccatctaccggctttgtgaacctgctgaaaaccaagtataccagcatcgccgattccaagaagttcatcagctcctttgacaggatcatgtatgtgcccgaggaggatctgttcgagtttgccctggactataagaacttctctcgcacagacgccgattacatcaagaagtggaagctgtactcctacggcaaccggatcagaatcttccggaatcctaagaagaacaacgtgttcgactgggaggaggtgtgcctgaccagcgcctataaggagctgttcaacaagtacggcatcaattatcagcagggcgatatcagagccctgctgtgcgagcagtccgacaaggccttctactctagctttatggccctgatgagcctgatgctgcagatgcggaacagcatcacaggccgcaccgacgtggattttctgatcagccctgtgaagaactccgacggcatcttctacgatagccggaactatgaggcccaggagaatgccatcctgccaaagaacgccgacgccaatggcgcctataacatcgccagaaaggtgctgtgggccatcggccagttcaagaaggccgaggacgagaagctggataaggtgaagatcgccatctctaacaaggagtggctggagtacgcccagaccagcgtgaagcacaaaaggccggcggccacgaaaaaggccggccaggcaaaaaagaaaaagtga

SEQ ID NO: 74 - DNA, 3783 bp, synthetic construct
  misc_feature 1..3783: note = codon optimized LbCpf1
  source 1..3783: mol_type = other DNA
atggctcctaagaagaagcggaaggttggtattcacggggtgcctgcggcttcaaagctcgagaaattcaccaactgttattcgttgagcaaaacactgcggtttaaagcgattccagtcggcaagactcaagagaatatagacaataagcggctgttggtggaagatgaaaagcgcgcggaagactacaaaggggtgaagaagttgttggacagatactacctctcttttatcaatgatgtcttgcactcaatcaaattgaagaatctgaacaactacatctccctcttcagaaagaaaacaaggacagaaaaggagaataaggaacttgaaaatttggagatcaatctgaggaaagagatcgcgaaagcctttaaaggcaacgaaggatacaaaagtctgttcaagaaggatataattgagacaattttgccagagttcctcgatgacaaggacgagattgcgctggtcaattcgttcaacggattcacaacagcattcacaggcttctttgataatcgggaaaatatgttctctgaggaggcaaagtccacttctattgcgttcaggtgtatcaatgagaatctcactaggtacatttccaacatggatatctttgagaaggttgacgcaatttttgacaagcacgaagttcaggagattaaggagaagatcctcaattccgattatgacgttgaggacttcttcgaaggtgagttttttaatttcgtgctcactcaagagggtatcgacgtgtataatgcgatcatcggtgggttcgtgactgagtccggtgaaaagattaagggattgaacgagtatatcaacctttacaaccaaaagacgaaacagaagctgccaaagttcaagcctctttacaaacaggttctttcagaccgcgagtcactctcgttctatggggagggctacacttcggatgaggaagtcctggaggtgttcaggaatactctcaataagaattcggagattttctcttctataaaaaaactggaaaagttgtttaagaattttgacgaatactctagcgccggcatatttgtgaaaaacggcccggccatatcaacgataagtaaagatatcttcggcgaatggaacgtgatcagagacaaatggaacgcggagtatgacgatattcacctgaagaagaaggctgtcgtaacggagaagtacgaggatgatcgcaggaaaagcttcaaaaagatcggaagtttcagcctggaacagttgcaggagtatgctgacgccgatcttagcgtcgtcgagaagttgaaggagataatcatccaaaaggtcgacgagatatataaagtctatggatcaagtgaaaaactgttcgacgccgacttcgttttggagaagtccctgaagaagaacgacgctgttgttgccattatgaaggatctgctcgacagcgtgaagagtttcgagaactatattaaggcttttttcggggaggggaaggagactaacagagatgagtccttctacggagacttcgtcctcgcgtacgatatactccttaaggtagaccacatctacgacgcaatcagaaattacgtgacacaaaagccgtacagcaaggacaagttcaaactctacttccagaacccccagttcatgggcggctgggacaaggacaaggaaacggattacagggctacgatcttgaggtatggttcaaaatactacttggcgattatggacaagaagtacgccaagtgtctccagaagattgacaaagacgatgtcaatggcaattatgagaagatcaactacaagctgcttccgggtccgaacaagatgctcccaaaggttttcttcagcaagaaatggatggcctactataacccaagcgaggacatccagaagatttataagaacggtacgttcaagaagggcgacatgttcaatcttaacgactgtcacaagctgatcgacttcttcaaagactcaattagccggtacccaaagtggtctaacgcctatgacttcaacttttcggaaaccgagaagtacaaggatatagccggattttatagagaggtggaagagcagggctacaaggtgtcattcgagtccgccagcaagaaggaagtggacaagctcgtggaagagggtaagctctacatgttccagatttataataaagactttagcgataagagccacgggacacctaatctccacacaatgtatttcaagctgctcttcgacgagaataaccacggccaaatcaggttgtcaggaggggctgaactcttcatgcggcgcgctagccttaagaaggaggagcttgtagtccaccctgcgaatagtccaattgcgaataagaacccggacaatcctaaaaagactacaacattgagctacgacgtgtacaaggataagaggttttccgaggatcagtacgagctccacatcccgattgcgatcaacaagtgcccaaagaatattttcaagataaacacagaggtgcgtgtactcctgaagcatgacgacaatccttacgtcattgggattgatcggggcgagaggaacctcctctatattgtggtggtggacgggaaggggaacatagtcgaacagtactcccttaacgaaataattaacaatttcaacggcatccgtatcaagaccgactaccattcgttgctggacaagaaggagaaggagagatttgaggcgcggcaaaattggacaagtatcgagaacatcaaggaactcaaagcaggttatatctctcaagttgtgcataagatatgcgagctggttgagaagtatgacgcagtgatcgctcttgaggacctcaactcgggctttaagaattctagagttaaagtggagaagcaggtctatcaaaagttcgagaagatgcttatagataagctcaactacatggtcgataagaaatcgaacccatgtgccaccggcggcgcactcaaaggttaccaaataacaaacaaattcgagtccttcaaatcgatgagtactcagaatgggttcatattttatataccggcgtggcttacgtctaagatcgacccgtcaactggttttgtcaacctgttgaagacgaaatacacgtccattgccgattcgaaaaagttcatatctagttttgatcgtattatgtacgtcccagaggaagatcttttcgagtttgctctcgactacaaaaacttttcgcggaccgatgcggattacattaaaaaatggaaactctattcgtacggcaacagaatcaggatttttcgcaaccctaagaagaataacgtctttgattgggaggaagtttgcttgactagcgcgtacaaggagctctttaataagtatggcattaactaccaacagggtgatatcagagcactgctttgcgaacaatctgacaaggctttctactcatccttcatggctttgatgagcctgatgctccagatgagaaattcaattacaggcagaaccgacgtggatttcttgatctccccggttaaaaattctgatggcatcttttacgatagcaggaactatgaagcgcaagagaatgcgattctgccaaaaaatgcagacgccaacggtgcctataacatcgccaggaaagtcctgtgggcgatcggccagttcaaaaaggccgaagacgaaaaattggacaaggtcaaaatcgctatcagcaacaaagagtggctggagtatgctcagacatccgtaaagcataagcgtcctgctgccaccaaaaaggccggacaggctaagaaaaagaagtga

SEQ ID NO: 75 - DNA, 3759 bp, synthetic construct
  misc_feature 1..3759: note = codon optimized LbCpf1
  source 1..3759: mol_type = other DNA
atggccccgaagaagaagaggaaggtcagcaagctcgagaagttcaccaactgctacagcctgagcaagaccctgaggttcaaggctatcccggtgggcaagacccaagagaacatcgacaacaagaggctgctggtcgaggacgagaagcgcgctgaggattacaagggcgtgaagaagctgctggacaggtactacctgagcttcatcaacgacgtgctgcacagcatcaagctgaagaacctgaacaactacatcagcctgttccgcaagaaaaccaggaccgagaaagagaacaaagagcttgagaacctcgagatcaacctgaggaaagagatcgccaaggccttcaagggcaacgagggctacaagagcctgttcaagaaggacatcatcgagactatcctgccagagttcctggacgacaaggacgagatcgccctggtgaacagcttcaacggcttcacgaccgccttcaccggtttcttcgacaaccgcgagaatatgttcagcgaggaagccaagagcacctctatcgccttccgctgcatcaacgagaacctgacgcgctacatctccaacatggatatcttcgagaaggtggacgccatcttcgataagcacgaggtgcaagagatcaaagaaaagatcctgaacagcgactacgacgtcgaggacttcttcgagggcgagttcttcaacttcgtgctcacccaagagggcatcgatgtgtacaacgccatcatcggcggcttcgtgactgagagcggcgagaagatcaagggcctgaacgagtacatcaacctctacaatcaaaagaccaagcagaagctgccgaagttcaagccgctgtacaagcaggttctgagcgaccgcgagagcctgtctttctacggcgagggttacaccagcgacgaagaggtgttggaggttttccgcaacaccctgaacaagaacagcgagatcttcagctccatcaagaagctggaaaagctgtttaagaacttcgacgagtacagcagcgccggcatcttcgtgaagaacggcccagctatcagcaccatcagcaaggacatcttcggcgagtggaacgtgatcagggacaagtggaacgccgagtacgacgacatccacctgaagaaaaaggccgtggtgaccgagaagtacgaggacgacaggcgcaagagcttcaagaagatcggctccttcagcctcgagcagctgcaagagtacgctgacgctgacctgagcgtggtcgagaagctcaaagagatcatcatccagaaggtcgacgagatctacaaggtgtacggcagcagcgagaagcttttcgacgccgacttcgtccttgagaagtccctcaagaaaaacgacgccgtggtggccatcatgaaggacctgctggactccgtgaagtccttcgagaactacattaaggctttcttcggtgagggcaaagagactaacagggacgagagcttctacggggatttcgtgctggcctacgacatcctgctcaaggtggaccacatctacgacgccatccgcaactacgtgacccagaagccgtactccaaggacaagtttaagctgtacttccagaatccgcagttcatgggcggctgggacaaagacaaagaaaccgactacagggccaccatcctgaggtacggctccaagtactacctcgccatcatggacaagaaatacgccaagtgcctgcagaagatcgataaggacgacgtgaacggcaactacgagaagattaactacaagctgctgccagggccgaacaagatgctcccgaaggtgttctttagcaagaaatggatggcctactacaacccgagcgaggatatccagaaaatctacaagaacggcaccttcaagaaaggcgacatgttcaacctgaacgactgccacaagctgatcgatttcttcaaggacagcatctctcgctacccgaagtggtccaacgcctacgatttcaacttcagcgagactgaaaagtacaaggatatcgccggcttctaccgcgaggtcgaggaacagggttacaaggtgagcttcgagagcgccagcaagaaagaggtggacaagctggtcgaagagggcaagctgtacatgttccagatctataacaaggacttctccgacaagagccacggcaccccaaacctgcacaccatgtacttcaagttgctgttcgacgagaacaaccacggccagatcaggctttctggcggcgctgagcttttcatgagaagggccagcctgaaaaaagaggaactggtcgttcacccggcgaacagcccaatcgccaacaagaacccggacaacccgaaaaagaccaccacgctgagctacgacgtgtacaaggacaaaaggttctccgaggaccagtacgagctgcacatcccgatcgccatcaacaagtgcccgaagaacatcttcaagatcaacaccgaggtgagggtgctgctgaagcacgacgacaacccatacgtgatcggcatcgataggggcgagcgcaacctgctctacatcgtggtggttgacggcaagggcaatatcgtcgagcagtacagccttaacgagatcattaacaacttcaatggcatcaggatcaagaccgactaccacagcctgctcgacaagaaagaaaaagagcgcttcgaggccaggcagaactggaccagcatcgagaatatcaaagagctgaaggccggctacattagccaggtggtgcacaagatctgcgagctggtggaaaagtacgacgcggtgatcgctctcgaggacctgaactccgggttcaagaactcccgcgtgaaggttgagaagcaggtctaccaaaagttcgagaagatgctgatcgacaagctcaactacatggtggacaaaaagagcaacccctgcgccacaggcggcgctcttaagggctaccagatcacgaacaagttcgagtccttcaagagcatgagcacccagaatggcttcatcttctacatcccggcctggctgaccagcaagatcgatccatctaccggcttcgtcaacctcctcaagaccaagtacaccagcattgccgacagcaagaagttcatctccagcttcgacaggatcatgtacgtgccggaagaggacctgttcgagttcgcgctcgattacaagaacttcagcaggaccgacgcggactatattaagaagtggaagctctacagctacggcaacaggatccgcatcttcagaaacccgaagaaaaacaacgtgttcgactgggaagaagtgtgcctgaccagcgcctacaaagaactgttcaacaagtacggcatcaactaccagcagggcgacatcagggctctgctgtgcgagcagtctgacaaggcgttctacagctccttcatggccctgatgagcctgatgctgcagatgaggaacagcatcaccggcaggacggacgtcgacttcctgatcagcccagtgaagaattccgacggcattttctacgactctaggaactacgaggctcaagagaacgccatcctgccgaagaacgccgatgctaacggcgcgtacaacattgcccgcaaggtgctgtgggctatcggccagtttaagaaggccgaggacgaaaaactggacaaggtgaagatcgccattagcaacaaagagtggctcgagtacgcccagaccagcgtgaagcacaaaaggccagccgccactaagaaggctggccaggccaaaaagaagaagtga

SEQ ID NO: 76 - DNA, 3759 bp, synthetic construct
  misc_feature 1..3759: note = codon optimized LbCpf1
  source 1..3759: mol_type = other DNA
atggcacccaagaagaagcgcaaagtgtcaaagctcgagaagttcacaaactgttactccttatctaaaaccctgcgctttaaagcaattcctgtcggtaaaacccaagagaacatcgacaacaagagactgctcgttgaagatgaaaagagagccgaggattacaagggcgtgaagaagctcctcgatcgctattacctgtccttcattaacgatgtgctccatagcatcaagctcaagaaccttaacaactatatctcattattccgcaagaaaactagaacggagaaggaaaacaaagagctagagaaccttgaaatcaacctcagaaaggaaatagccaaggcgtttaaggggaatgaaggctacaagagtttgtttaagaaagacatcattgagacaatattacctgaattccttgatgacaaggacgagatcgctctagtgaacagctttaatggtttcaccactgcgttcacgggcttcttcgataacagggagaatatgttttctgaggaagccaagtcaacttccatcgcgtttcgctgcatcaacgagaatctgacccgttacataagtaacatggacatattcgagaaagttgacgctatcttcgacaagcatgaggtgcaagaaatcaaggaaaagatccttaactctgactacgacgtcgaggacttcttcgagggagaattcttcaatttcgttctgacccaggagggcatcgacgtgtacaatgctattatcggtggattcgtgacagagtccggagaaaagattaagggccttaacgagtatatcaacctttataaccaaaagacgaagcaaaaactccccaagtttaaacctctttacaaacaagttctatcggatagagaaagcctttcgttttacggggaaggatacacctctgatgaagaggttctcgaggtgttccgtaacaccctgaacaagaactccgagatattctcgtcgattaagaaactcgaaaagttgttcaaaaacttcgacgaatactcatctgccggaatttttgtgaagaacggcccggctatttcgaccatttccaaggatatcttcggagagtggaacgttatacgagataagtggaacgcagagtatgatgatatccaccttaagaagaaggcggtcgtgacggaaaaatacgaggacgatcgtaggaagtctttcaagaagattggtagcttcagcctcgagcaactgcaggaatacgcggatgctgatctgagcgtggtcgagaagcttaaggagataatcatccaaaaggttgacgagatatacaaggtttatggttcgtcagagaagttgttcgacgccgacttcgtccttgagaagtccctgaagaagaatgacgcggtcgtggcaatcatgaaagacctcctcgactccgtcaaatcctttgagaattatattaaggcgttcttcggcgaagggaaggagacaaatagggatgagagtttttacggcgattttgtgctagcttacgacattctgctgaaagttgaccacatatacgacgctatccgaaactatgtcacccaaaagccttactcaaaagacaagttcaagctgtactttcaaaacccgcagttcatgggaggatgggataaggacaaggaaactgactacagagccacgattctccgctacgggtccaaatactacctcgccattatggataagaagtacgcgaagtgcctgcagaagatcgacaaagacgacgtgaacggaaactacgagaagatcaactataagctgctgccagggcccaacaagatgctgccgaaggttttctttagcaagaagtggatggcctactacaacccgtccgaggacatacagaaaatctacaaaaatggaactttcaaaaagggcgacatgttcaacttgaacgattgccacaagttaattgacttcttcaaggacagcatttcgcgatatccgaagtggtctaatgcctatgacttcaatttttctgaaaccgagaagtataaggatatcgcgggtttttatagggaagttgaggagcaaggttacaaagtatcatttgaatctgcctccaaaaaggaggtcgacaaactggttgaagagggcaaactatacatgtttcagatctacaacaaagatttctcggataagtcgcacgggacgccgaacttacacaccatgtacttcaaactgctgtttgatgagaacaatcacggccagatccgtctaagcggcggtgccgagcttttcatgcgccgcgcgagcttgaaaaaggaggagttggtggtccaccctgctaattcaccgattgctaacaagaaccccgataaccccaaaaagaccaccactcttagctacgatgtctataaggataagcgcttcagcgaagatcagtatgagttgcatattccgattgccatcaacaaatgccccaaaaatattttcaagatcaacactgaggtccgcgtgctgctcaaacatgacgataacccgtacgtaatcggcatcgatagaggcgaacggaacttactatacatcgtggtagtagacgggaagggaaatatcgtcgaacagtacagtctgaatgaaattattaacaatttcaacgggatccggatcaagacagactaccactccttgctcgacaagaaggaaaaggagcggttcgaggcccgacaaaactggacttcgattgagaacattaaggagctcaaagcggggtacatctcccaagtggtgcataaaatctgtgaactggttgagaaatatgatgcagtgatagctctcgaggacctcaattctggcttcaagaactccagggttaaggtagaaaaacaggtctaccaaaaatttgaaaagatgcttattgataagttaaattacatggtcgacaaaaagtcgaatccgtgtgccacaggaggcgccctcaagggataccagattacgaataagtttgaatccttcaagtctatgagcacacagaacggcttcattttctatatccccgcgtggctcacttctaaaatcgacccatccaccggcttcgtgaatttgcttaagacaaagtacactagcatcgcggactcgaagaaattcatttcgtcgtttgaccggattatgtatgtgccagaagaagatctattcgagtttgctctcgactataaaaacttctcccgcaccgacgccgactacataaagaagtggaagttgtatagctacgggaaccgcatcaggatattccggaatccgaagaagaacaatgtgtttgattgggaggaggtctgcctcacgtcagcttacaaggagctgttcaacaaatacggtataaactatcagcagggcgacatccgggcccttctgtgtgaacagagcgacaaagcattttactcttcttttatggctctgatgtccttgatgctgcaaatgcgcaattcaatcacggggagaaccgatgtagactttctgattagtccggtcaagaatagcgacggcatattctacgattcaaggaattacgaagcccaggagaacgcgatcctgccaaaaaatgcagatgcgaatggtgcatacaatattgcaaggaaagtgttatgggccatcggccagttcaagaaagctgaggacgagaagcttgacaaggtcaagatcgcaatctcaaacaaggaatggcttgaatatgcgcagactagtgtgaaacataagcgcccagctgccaccaagaaggccggccaggccaagaaaaagaagtga

SEQ ID NO: 77 - DNA, 24 bp, Triticum aestivum
  source 1..24: mol_type = genomic DNA
cagcatggcatggagggtgacgat

SEQ ID NO: 78 - DNA, 24 bp, Triticum aestivum
  source 1..24: mol_type = genomic DNA
agcatggcatggagggtgacgatg

SEQ ID NO: 79 - DNA, 24 bp, Triticum aestivum
  source 1..24: mol_type = genomic DNA
cgcaggaggaggaggagctcatcg

SEQ ID NO: 80 - DNA, 24 bp, Triticum aestivum
  source 1..24: mol_type = genomic DNA
cgcaccgcttcagccctgcagcac

SEQ ID NO: 81 - DNA, 24 bp, Triticum aestivum
  source 1..24: mol_type = genomic DNA
gcaccgcttcagccctgcagcacg

SEQ ID NO: 82 - DNA, 21 bp, Beta vulgaris
  source 1..21: mol_type = genomic DNA
gctgctaaacaatcaacattt

SEQ ID NO: 83 - DNA, 21 bp, Beta vulgaris
  source 1..21: mol_type = genomic DNA
taaacaatcaacatttaggta

SEQ ID NO: 84 - DNA, 20 bp, Beta vulgaris
  source 1..20: mol_type = genomic DNA
atttaggtatggttgtccaa

SEQ ID NO: 85 - DNA, 20 bp, Beta vulgaris
  source 1..20: mol_type = genomic DNA
tttagcagcattatcttaac

SEQ ID NO: 86 - DNA, 20 bp, Beta vulgaris
  source 1..20: mol_type = genomic DNA
tatagaacctatcttcccat

SEQ ID NO: 87 - RNA, 86 nt, Helianthus annuus; identical to SEQ ID NO: 24
  source 1..86: mol_type = other RNA

SEQ ID NO: 88 - DNA, 24 bp, synthetic construct
  misc_feature 1..24: note = crALS1 protospacer
  source 1..24: mol_type = other DNA
caccctaattgtagccaactcttg

SEQ ID NO: 89 - DNA, 24 bp, synthetic construct
  misc_feature 1..24: note = crALS2 protospacer
  source 1..24: mol_type = other DNA
gcagcattatcttaactgggagat

SEQ ID NO: 90 - DNA, 24 bp, synthetic construct
  misc_feature 1..24: note = crALS3 protospacer
  source 1..24: mol_type = other DNA
ggtatggttgtccaatgggaagat

SEQ ID NO: 91 - DNA, 24 bp, synthetic construct
  misc_feature 1..24: note = crALS4 protospacer
  source 1..24: mol_type = other DNA
caaggtatgtatgtgcccggttag

SEQ ID NO: 92 - DNA, 24 bp, synthetic construct
  misc_feature 1..24: note = crALS5 protospacer
  source 1..24: mol_type = other DNA
gaagggtttccaaggtatgtatgt

SEQ ID NO: 93 - DNA, 8828 bp, synthetic construct
  misc_feature 1..8828: note = expression plasmid
  source 1..8828: mol_type = other DNA
gattgaaagaaatatagtttaaatatttattgataaaataacaagtcaggtattatagtccaagcaaaaacataaatttattgatgcaagtttaaattcagaaatatttcaataactgattatatcagctggtacattgccgtagatgaaagactgagtgcgatattatgtgtaatacataaattgatgatatagctagcttagctcatcgggtcagaagaactcgtcaagaaggcgatagaaggcgatgcgctgcgaatcgggagcggcgataccgtaaagcacgaggaagcggtcagcccattcgccgccaagctcttcagcaatatcacgggtagccaacgctatgtcctgatagcggtccgccacacccagccggccacagtcgatgaatccagaaaagcggccattttccaccatgatattcggcaagcaggcatcgccatgagtcacgacgagatcctcgccgtcgggcatgcgcgccttgagcctggcgaacagttcggctggcgcgagcccctgatgctcttcgtccagatcatcctgatcgacaagaccggcttccatccgagtacgtgctcgctcgatgcgatgtttcgcttggtggtcgaatgggcaggtagccggatcaagcgtatgcagccgccgcattgcatcagccatgatggatactttctcggcaggagcaaggtgagatgacaggagatcctgccccggcacttcgcccaatagcagccagtcccttcccgcttcagtgacaacgtcgagcacagctgcgcaaggaacgcccgtcgtggccagccacgatagccgcgctgcctcgtcctgaagttcattcagggcaccggacaggtcggtcttgacaaaaagaaccgggcgcccctgcgctgacagccggaacacggcggcatcagagcagccgattgtctgttgtgcccagtcatagccgaatagcctctccacccaagcggccggagaacctgcgtgcaatccatcttgttcaatccaagctcccattttctgtgattttggatgtgtttttgtatggattgagagtgaatatgagactctaattggataccgaggggaatttatggaacgtcagtggagcatttttgacaagaaatatttgctagctgatagtgaccttaggcgacttttgaacgcgcaataatggtttctgacgtatgtgcttagctcattaaactccagaaacccgcggctgagtggctccttcaacgttgcggttctgtcagttccaaacgtaaaacggcttgtcccgcgtcatcggcgggggtcattccggactgtggggccatatcccagaactggttgagtcggtccaacacctgggtgccaatcatgtcgatggtggggtatggccaattttttttcaattcaaaaatgtagatgtccgcagcgttattataaaatgaaagtacattttgataaaacgacaaattacgatccgtcgtatttataggcgaaagcaataaacaaattattctaattcggaaatctttatttcgacgtgtctacattcacgtccaaatgggggcttagatgagaaacttcacgatcggctctagaggccatggcggccgctcgagcgatctagtaacatagatgacaccgcgcgcgataatttatcctagtttgcgcgctatattttgttttctatcgcgtattaaatgtataattgcgggactctaatcataaaaacccatctcataaataacgtcatgcattacatgttaattattacatgcttaacgtaattcaacagaaattatatgataatcatcgcaagaccggcaacaggattcaatcttaagaaactttattgccaaatgtttgaacgatcggggaaattcgatctacacttagtagaaattacaagagttggctacaattagggtgatctacacttagtagaaattatcaggtacctctagacttgtacagctcgtccatgccgtacaggaacaggtggtggcggccctcggagcgctcgtactgttccacgatggtgtagtcctcgttgtgggaggtgatgtccagcttggtgtccacgtagtagtagccgggcagttgcacgggcttcttggccatgtagatggtcttgaactccaccaggtagtggccgccgtccttcagcttcagggcctggtggatctcgcccttcagcacgccgtcgcgggggtacaggcgctcggtggaggcctcccagcccatggtcttcttctgcattacggggccgtcgggggggaagttggtgccgcgcatcttcaccttgtagatcagcgtgccgtcctgcagggaggagtcctgggtcacggtcaccagaccgccgtcctcgaagttcatcacgcgctcccacttgaagccctcggggaaggacagcttcttgtaatcggggatgtcggcggggtgcttcacgtacgccttggagccgtacatgaactggggggacaggatgtcccaggcgaagggcagggggccgcccttggtcaccttcagcttggcggtctgggtgccctcgtaggggcggccctcgccctcgccctcgatctcgaactcgtggccgttcatggagccctccatgcgcaccttgaagcgcatgaactctttgatgacctcctcgcccttgctcaccatggatcccctctccaaatgaaatgaacttccttatatagaggaagggtcttgcgaaggatagtgggattgtgcgtcatcccttacgtcagtggagatatcacatcaatccacttgctttgaagacgtggttggaacgtcttctttttccacgatgttcctcgtgggtgggggtccatctttgggaccactgtcggtagaggcatcttgaacgatagcctttcctttatcgcaatgatggcatttgtagaagccatcttccttttctactgtcctttcgatgaagtgacagatagctgggcaatggaatccgaggaggtttcccgatattaccctttgttgaaaagtctcaatagccctctggtcttctgagactgtatctttgatattcttggagtagacgagagtgtcgtgctccaccatgtatcacatcaatccacttgctttgaagacgtggttggaacgtcttctttttccacgatgttcctcgtgggtgggggtccatctttgggaccactgtcggtagaggcatcttgaacgatagcctttcctttatcgcaatgatggcatttgtagaagccatcttccttttctactgtcctttcgatgaagtgacagatagctgggcaatggaatccgaggaggtttcccgatattaccctttgttgaaaagtctcaatagccctctggtcttctgaacactagtaaggccttaagggccagatcccccgggctgcaggaattcgatctggcacgacaggtttcccgactggaaagcgggcagtgagcgcaacgcaattaatgtgagttagctcactcattaggcaccccaggctttacactttatgcttccggctcgtatgttgtgtggaattgtgagcggataacaatttcacacaggaaacagctatgacatgattacgaattcaaaaattacggatatgaatataggcatatccgtatccgaattatccgtttgacagctagcaacgattgtacaattgcttctttaaaaaaggaagaaagaaagaaagaaaagaatcaacatcagcgttaacaaacggccccgttacggcccaaacggtcatatagagtaacggcgttaagcgttgaaagactcctatcgaaatacgtaaccgcaaacgtgtcatagtcagatcccctcttccttcaccgcctcaaacacaaaaataatcttctacagcctatatatacaacccccccttctatctctcctttctcacaattcatcatctttctttctctacccccaattttaagaaatcctctcttctcctcttcattttcaaggtaaatctctctctctctctctctctctgttattccttgttttaattaggtatgtattattgctagtttgttaatctgcttatcttatgtatgccttatgtgaatatctttatcttgttcatctcatccgtttagaagctataaatttgttgatttgactgtgtatctacacgtggttatgtttatatctaatcagatatgaatttcttcatattgttgcgtttgtgtgtaccaatccgaaatcgttgatttttttcatttaatcgtgtagctaattgtacgtatacatatggatctacgtatcaattgttcatctgtttgtgtttgtatgtatacagatctgaaaacatcacttctctcatctgattgtgttgttacatacatagatatagatctgttatatcattttttttattaattgtgtatatatatatgtgcatagatctggattacatgattgtgattatttacatgattttgttatttacgtatgtatatatgtagatctggactttttggagttgttgacttgattgtatttgtgtgtgtatatgtgtgttctgatcttgatatgttatgtatgtgcagcgaattcggcgcgccaaacaatggcttcctccatggctcctaagaagaagaggaaggttagcaagctcgagaagtttaccaactgctacagcctctctaagaccctcaggttcaaggctatccctgtgggaaagacccaagagaatatcgacaacaagaggctcctcgtcgaggatgagaagagagctgaagattacaagggcgtgaagaagctcctcgacaggtactacctcagcttcatcaacgatgtgctccacagcatcaagctcaagaacctcaacaactacatcagcctcttccgtaagaaaaccaggaccgagaaagagaacaaagagcttgagaacctcgagatcaacctccgtaaagagatcgccaaggctttcaagggaaacgagggatacaagagcctcttcaagaaggatattatcgagacaatcctgcctgagttcctggacgataaggatgagatcgctctcgtgaacagcttcaacggattcactactgccttcaccggattcttcgacaacagggaaaacatgttcagcgaagaggccaagagcacctctatcgctttcagatgcatcaacgagaacctcacgcgttacatcagcaacatggacatcttcgagaaggtggacgccatcttcgataagcacgaggtgcaagaaatcaaagagaagatcctcaacagcgactacgacgtcgaggacttttttgaaggggagttcttcaacttcgttctcacccaagagggcatcgacgtgtacaacgctattatcggaggattcgtgaccgagtctggggagaagattaagggactcaacgagtacatcaacctgtacaaccagaaaacgaagcagaagctcccgaagttcaagccgctctacaagcaggttctctctgatcgtgagagcctctcattttacggtgagggttacacctctgacgaggaagtgcttgaggttttccgtaacaccctcaacaagaacagcgagatcttctcgtccatcaagaagttggagaaacttttcaagaacttcgacgagtacagcagcgctgggatcttcgttaagaacggacctgctatcagcaccatcagcaaggatattttcggcgagtggaacgtgatcagggacaagtggaatgctgagtacgatgacatccacctcaagaagaaggctgtcgtcactgagaagtacgaggatgacaggcgtaagtcgttcaagaagatcggctctttcagcctcgagcagcttcaagaatacgctgatgctgatctcagcgtggtcgagaagctcaaagagatcatcatccagaaggtcgacgagatctacaaggtgtacgggtcctctgagaagttgttcgatgctgatttcgtcctcgagaagagtctgaagaagaacgacgctgtcgtcgcgatcatgaaggatttgctcgacagcgtgaagtccttcgagaactatatcaaggccttcttcggagagggcaaagagactaatagggacgagtctttctacggggatttcgtgctcgcttacgatatcctcctcaaggtggaccatatctacgacgccatcagaaactacgtgacccagaagccttacagcaaggacaagttcaagttgtactttcagaacccgcagttcatgggcggatgggacaaagacaaagagacagattacagggccaccatcctcaggtacgggtctaagtactacctggccatcatggacaagaaatacgccaagtgcctccaaaagatcgacaaggatgacgtgaacgggaactatgagaagatcaactacaagctccttccgggaccgaacaagatgcttcctaaggtgttcttcagcaagaaatggatggcctactacaacccgtctgaggacatccagaaaatctacaagaacgggaccttcaagaaaggcgacatgttcaacctcaacgactgccacaagctcatcgatttcttcaaggacagcatctcgcgttacccgaagtggtctaacgcttacgactttaacttcagcgagacagaaaagtacaaggatatcgccgggttctaccgtgaggttgaggaacagggttacaaggttagcttcgagagcgcctccaagaaagaggttgacaagttggtcgaagagggcaagctctacatgttccagatctataacaaggacttctccgacaagagccacggaactcctaacctccatacgatgtacttcaagctgcttttcgacgagaacaaccacgggcagatcagactttctggtggtgctgaactcttcatgcgtagggcctcactcaagaaagaagagttggttgttcacccggccaactctccaatcgctaacaagaatcctgacaacccgaaaaagaccaccacgctgtcttacgacgtctacaaggacaaaaggttcagcgaggaccagtacgagcttcatatcccgatcgctatcaacaagtgcccgaagaacatcttcaagatcaataccgaggtgagggtgctgctcaagcacgatgataacccttacgtgatcggaatcgatcgtggtgagagaaacctcctctacatcgttgtggtggacggaaagggaaacatcgtcgagcagtacagcctgaacgagattatcaacaatttcaacggcatcaggatcaagaccgactaccactcactcctcgataagaaagaaaaagagcgtttcgaggccaggcagaactggacttctatcgaaaacatcaaagagttgaaggccggctacatctctcaggtggtgcataagatctgcgagctggtggaaaagtacgatgctgtgatcgctcttgaggacctcaactctgggttcaagaacagtagagtgaaggttgagaagcaggtctaccaaaagttcgagaagatgctcatcgacaagctcaactacatggtggacaaaaagagcaacccttgcgctaccggtggtgctcttaagggataccagatcacgaacaagttcgagtccttcaagagcatgagcacccagaacggcttcatcttctatatccctgcttggctcaccagcaagatcgatccttctactggtttcgtgaacctgctcaagaccaagtacacctcgatcgccgacagcaagaagttcatctcgtctttcgacaggatcatgtacgtgccggaagaggatcttttcgagttcgctctcgactataagaacttcagcaggaccgacgccgactacattaagaagtggaagctctactcctacgggaaccgtatcaggatcttccgaaatccgaagaaaaacaacgtgttcgactgggaagaagtgtgcctcacctctgcctacaaagaactgttcaacaagtacggcatcaactaccagcagggtgatatcagggctcttttgtgcgagcagagcgacaaggcattctacagctcattcatggccctcatgtctctcatgctccagatgaggaactctatcaccggaaggaccgatgtggacttccttatctctccggtcaagaactctgacgggatcttctacgacagccgtaactatgaggctcaagagaacgctatcctgccgaagaatgctgatgcaaacggggcttacaacattgcgagaaaggttctctgggctatcgggcagtttaagaaagcggaagatgagaagctcgacaaggtgaagatcgccatctccaacaaagagtggcttgagtacgctcagacctccgttaagcacaagaggcctgctgctactaagaaagctggccaggccaaaaagaagaagtgaggcgcgccgagctccaggcctcccagctttcgtccgtatcatcggtttcgacaacgttcgtcaagttcaatgcatcagtttcattgcccacacaccagaatcctactaagtttgagtattatggcattggaaaagctgttttcttctatcatttgttctgcttgtaatttactgtgttctttcagtttttgttttcggacatcaaaatgcaaatggatggataagagttaataaatgatatggtccttttgttcattctcaaattattattatctgttgtttttactttaatgggttgaatttaagtaagaaaggaactaacagtgtgatattaaggtgcaatgttagacatataaaacagtctttcacctctctttggttatgtcttgaattggtttgtttcttcacttatctgtgtaatcaagtttactatgagtctatgatcaagtaattatgcaatcaagttaagtacagtataggctt

SEQ ID NO: 94 - DNA, 8201 bp, synthetic construct
  misc_feature 1..8201: note = expression plasmid
  source 1..8201: mol_type = other DNA
ttgaaagaaatatagtttaaatatttattgataaaataacaagtcaggtattatagtccaagcaaaaacataaatttattgatgcaagtttaaattcagaaatatttcaataactgattatatcagctggtacattgccgtagatgaaagactgagtgcgatattatgtgtaatacataaattgatgatatagctagcttagctcatcgggtcagaagaactcgtcaagaaggcgatagaaggcgatgcgctgcgaatcgggagcggcgataccgtaaagcacgaggaagcggtcagcccattcgccgccaagctcttcagcaatatcacgggtagccaacgctatgtcctgatagcggtccgccacacccagccggccacagtcgatgaatccagaaaagcggccattttccaccatgatattcggcaagcaggcatcgccatgagtcacgacgagatcctcgccgtcgggcatgcgcgccttgagcctggcgaacagttcggctggcgcgagcccctgatgctcttcgtccagatcatcctgatcgacaagaccggcttccatccgagtacgtgctcgctcgatgcgatgtttcgcttggtggtcgaatgggcaggtagccggatcaagcgtatgcagccgccgcattgcatcagccatgatggatactttctcggcaggagcaaggtgagatgacaggagatcctgccccggcacttcgcccaatagcagccagtcccttcccgcttcagtgacaacgtcgagcacagctgcgcaaggaacgcccgtcgtggccagccacgatagccgcgctgcctcgtcctgaagttcattcagggcaccggacaggtcggtcttgacaaaaagaaccgggcgcccctgcgctgacagccggaacacggcggcatcagagcagccgattgtctgttgtgcccagtcatagccgaatagcctctccacccaagcggccggagaacctgcgtgcaatccatcttgttcaatccaagctcccattttctgtgattttggatgtgtttttgtatggattgagagtgaatatgagactctaattggataccgaggggaatttatggaacgtcagtggagcatttttgacaagaaatatttgctagctgatagtgaccttaggcgacttttgaacgcgcaataatggtttctgacgtatgtgcttagctcattaaactccagaaacccgcggctgagtggctccttcaacgttgcggttctgtcagttccaaacgtaaaacggcttgtcccgcgtcatcggcgggggtcattccggactgtggggccatatcccagaactggttgagtcggtccaacacctgggtgccaatcatgtcgatggtggggtatggccaattttttttcaattcaaaaatgtagatgtccgcagcgttattataaaatgaaagtacattttgataaaacgacaaattacgatccgtcgtatttataggcgaaagcaataaacaaattattctaattcggaaatctttatttcgacgtgtctacattcacgtccaaatgggggcttagatgagaaacttcacgatcggctctagaggccatggcggccgctcgagcgatctagtaacatagatgacaccgcgcgcgataatttatcctagtttgcgcgctatattttgttttctatcgcgtattaaatgtataattgcgggactctaatcataaaaacccatctcataaataacgtcatgcattacatgttaattattacatgcttaacgtaattcaacagaaattatatgataatcatcgcaagaccggcaacaggattcaatcttaagaaactttattgccaaatgtttgaacgatcgcctctctgcttggctcctctttcttgtgaaagagggttcccaggcgacaccacgaggaggtgcagagtaggactgacgcccaagagttggctacaattagggtgatctacacttagtagaaattagacgagcttactcgtttcgtcctcacggactcatcagtaatttggatcccctctccaaatgaaatgaacttccttatatagaggaagggtcttgcgaaggatagtgggattgtgcgtcatcccttacgtcagtggagatatcacatcaatccacttgctttgaagacgtggttggaacgtcttctttttccacgatgttcctcgtgggtgggggtccatctttgggaccactgtcggtagaggcatcttgaacgatagcctttcctttatcgcaatgatggcatttgtagaagccatcttccttttctactgtcctttcgatgaagtgacagatagctgggcaatggaatccgaggaggtttcccgatattaccctttgttgaaaagtctcaatagccctctggtcttctgagactgtatctttgatattcttggagtagacgagagtgtcgtgctccaccatgtatcacatcaatccacttgctttgaagacgtggttggaacgtcttctttttccacgatgttcctcgtgggtgggggtccatctttgggaccactgtcggtagaggcatcttgaacgatagcctttcctttatcgcaatgatggcatttgtagaagccatcttccttttctactgtcctttcgatgaagtgacagatagctgggcaatggaatccgaggaggtttcccgatattaccctttgttgaaaagtctcaatagccctctggtcttctgaacactagtaaggccttaagggccagatcccccgggctgcaggaattcgatctggcacgacaggtttcccgactggaaagcgggcagtgagcgcaacgcaattaatgtgagttagctcactcattaggcaccccaggctttacactttatgcttccggctcgtatgttgtgtggaattgtgagcggataacaatttcacacaggaaacagctatgacatgattacgaattcaaaaattacggatatgaatataggcatatccgtatccgaattatccgtttgacagctagcaacgattgtacaattgcttctttaaaaaaggaagaaagaaagaaagaaaagaatcaacatcagcgttaacaaacggccccgttacggcccaaacggtcatatagagtaacggcgttaagcgttgaaagactcctatcgaaatacgtaaccgcaaacgtgtcatagtcagatcccctcttccttcaccgcctcaaacacaaaaataatcttctacagcctatatatacaacccccccttctatctctcctttctcacaattcatcatctttctttctctacccccaattttaagaaatcctctcttctcctcttcattttcaaggtaaatctctctctctctctctctctctgttattccttgttttaattaggtatgtattattgctagtttgttaatctgcttatcttatgtatgccttatgtgaatatctttatcttgttcatctcatccgtttagaagctataaatttgttgatttgactgtgtatctacacgtggttatgtttatatctaatcagatatgaatttcttcatattgttgcgtttgtgtgtaccaatccgaaatcgttgatttttttcatttaatcgtgtagctaattgtacgtatacatatggatctacgtatcaattgttcatctgtttgtgtttgtatgtatacagatctgaaaacatcacttctctcatctgattgtgttgttacatacatagatatagatctgttatatcattttttttattaattgtgtatatatatatgtgcatagatctggattacatgattgtgattatttacatgattttgttatttacgtatgtatatatgtagatctggactttttggagttgttgacttgattgtatttgtgtgtgtatatgtgtgttctgatcttgatatgttatgtatgtgcagcgaattcggcgcgccaaacaatggcttcctccatggctcctaagaagaagaggaaggttagcaagctcgagaagtttaccaactgctacagcctctctaagaccctcaggttcaaggctatccctgtgggaaagacccaagagaatatcgacaacaagaggctcctcgtcgaggatgagaagagagctgaagattacaagggcgtgaagaagctcctcgacaggtactacctcagcttcatcaacgatgtgctccacagcatcaagctcaagaacctcaacaactacatcagcctcttccgtaagaaaaccaggaccgagaaagagaacaaagagcttgagaacctcgagatcaacctccgtaaagagatcgccaaggctttcaagggaaacgagggatacaagagcctcttcaagaaggatattatcgagacaatcctgcctgagttcctggacgataaggatgagatcgctctcgtgaacagcttcaacggattcactactgccttcaccggattcttcgacaacagggaaaacatgttcagcgaagaggccaagagcacctctatcgctttcagatgcatcaacgagaacctcacgcgttacatcagcaacatggacatcttcgagaaggtggacgccatcttcgataagcacgaggtgcaagaaatcaaagagaagatcctcaacagcgactacgacgtcgaggacttttttgaaggggagttcttcaacttcgttctcacccaagagggcatcgacgtgtacaacgctattatcggaggattcgtgaccgagtctggggagaagattaagggactcaacgagtacatcaacctgtacaaccagaaaacgaagcagaagctcccgaagttcaagccgctctacaagcaggttctctctgatcgtgagagcctctcattttacggtgagggttacacctctgacgaggaagtgcttgaggttttccgtaacaccctcaacaagaacagcgagatcttctcgtccatcaagaagttggagaaacttttcaagaacttcgacgagtacagcagcgctgggatcttcgttaagaacggacctgctatcagcaccatcagcaaggatattttcggcgagtggaacgtgatcagggacaagtggaatgctgagtacgatgacatccacctcaagaagaaggctgtcgtcactgagaagtacgaggatgacaggcgtaagtcgttcaagaagatcggctctttcagcctcgagcagcttcaagaatacgctgatgctgatctcagcgtggtcgagaagctcaaagagatcatcatccagaaggtcgacgagatctacaaggtgtacgggtcctctgagaagttgttcgatgctgatttcgtcctcgagaagagtctgaagaagaacgacgctgtcgtcgcgatcatgaaggatttgctcgacagcgtgaagtccttcgagaactatatcaaggccttcttcggagagggcaaagagactaatagggacgagtctttctacggggatttcgtgctcgcttacgatatcctcctcaaggtggaccatatctacgacgccatcagaaactacgtgacccagaagccttacagcaaggacaagttcaagttgtactttcagaacccgcagttcatgggcggatgggacaaagacaaagagacagattacagggccaccatcctcaggtacgggtctaagtactacctggccatcatggacaagaaatacgccaagtgcctccaaaagatcgacaaggatgacgtgaacgggaactatgagaagatcaactacaagctccttccgggaccgaacaagatgcttcctaaggtgttcttcagcaagaaatggatggcctactacaacccgtctgaggacatccagaaaatctacaagaacgggaccttcaagaaaggcgacatgttcaacctcaacgactgccacaagctcatcgatttcttcaaggacagcatctcgcgttacccgaagtggtctaacgcttacgactttaacttcagcgagacagaaaagtacaaggatatcgccgggttctaccgtgaggttgaggaacagggttacaaggttagcttcgagagcgcctccaagaaagaggttgacaagttggtcgaagagggcaagctctacatgttccagatctataacaaggacttctccgacaagagccacggaactcctaacctccatacgatgtacttcaagctgcttttcgacgagaacaaccacgggcagatcagactttctggtggtgctgaactcttcatgcgtagggcctcactcaagaaagaagagttggttgttcacccggccaactctccaatcgctaacaagaatcctgacaacccgaaaaagaccaccacgctgtcttacgacgtctacaaggacaaaaggttcagcgaggaccagtacgagcttcatatcccgatcgctatcaacaagtgcccgaagaacatcttcaagatcaataccgaggtgagggtgctgctcaagcacgatgataacccttacgtgatcggaatcgatcgtggtgagagaaacctcctctacatcgttgtggtggacggaaagggaaacatcgtcgagcagtacagcctgaacgagattatcaacaatttcaacggcatcaggatcaagaccgactaccactcactcctcgataagaaagaaaaagagcgtttcgaggccaggcagaactggacttctatcgaaaacatcaaagagttgaaggccggctacatctctcaggtggtgcataagatctgcgagctggtggaaaagtacgatgctgtgatcgctcttgaggacctcaactctgggttcaagaacagtagagtgaaggttgagaagcaggtctaccaaaagttcgagaagatgctcatcgacaagctcaactacatggtggacaaaaagagcaacccttgcgctaccggtggtgctcttaagggataccagatcacgaacaagttcgagtccttcaagagcatgagcacccagaacggcttcatcttctatatccctgcttggctcaccagcaagatcgatccttctactggtttcgtgaacctgctcaagaccaagtacacctcgatcgccgacagcaagaagttcatctcgtctttcgacaggatcatgtacgtgccggaagaggatcttttcgagttcgctctcgactataagaacttcagcaggaccgacgccgactacattaagaagtggaagctctactcctacgggaaccgtatcaggatcttccgaaatccgaagaaaaacaacgtgttcgactgggaagaagtgtgcctcacctctgcctacaaagaactgttcaacaagtacggcatcaactaccagcagggtgatatcagggctcttttgtgcgagcagagcgacaaggcattctacagctcattcatggccctcatgtctctcatgctccagatgaggaactctatcaccggaaggaccgatgtggacttccttatctctccggtcaagaactctgacgggatcttctacgacagccgtaactatgaggctcaagagaacgctatcctgccgaagaatgctgatgcaaacggggcttacaacattgcgagaaaggttctctgggctatcgggcagtttaagaaagcggaagatgagaagctcgacaaggtgaagatcgccatctccaacaaagagtggcttgagtacgctcagacctccgttaagcacaagaggcctgctgctactaagaaagctggccaggccaaaaagaagaagtgaggcgcgccgagctccaggcctcccagctttcgtccgtatcatcggtttcgacaacgttcgtcaagttcaatgcatcagtttcattgcccacacaccagaatcctactaagtttgagtattatggcattggaaaagctgttttcttctatcatttgttctgcttgtaatttactgtgttctttcagtttttgttttcggacatcaaaatgcaaatggatggataagagttaataaatgatatggtccttttgttcattctcaaattattattatctgttgtttttactttaatgggttgaatttaagtaagaaaggaactaacagtgtgatattaaggtgcaatgttagacatataaaacagtctttcacctctctttggttatgtcttgaattggtttgtttcttcacttatctgtgtaatcaagtttactatgagtctatgatcaagtaattatgcaatcaagttaagtacagtataggctt

SEQ ID NO: 95 - DNA, 87 bp, synthetic construct
  misc_feature 1..87: note = expression casssette
  source 1..87: mol_type = other DNA
cggggaaattcgatctacacttagtagaaattacaagagttggctacaattagggtgatctacacttagtagaaattatcaggtacc

SEQ ID NO: 96 - DNA, 141 bp, Beta vulgaris
  source 1..141: mol_type = genomic DNA
ggacaaccatacctaaatgttgattgtttagcagcattatcttaactgggagattttccaccctaattgtagccaactcttgaacattcataataaaactgccatccccatcaatatcgacaaccactgcatctggtcgag

SEQ ID NO: 97 - DNA, 135 bp, synthetic construct
  misc_feature 1..135: note = InDel1
  source 1..135: mol_type = other DNA
ggacaaccatacctaaatgttgattgtttagcagcattatcttaactttttccaccctaattgtagccaactcttgaacattcataataaaactgccatccccatcaatatcgacaaccactgcatctggtcgag

SEQ ID NO: 98 - DNA, 134 bp, synthetic construct
  misc_feature 1..134: note = InDel2
  source 1..134: mol_type = other DNA
ggacaaccatacctaaatgttgattgtttagcagcattatcttagattttccaccctaattgtagccaactcttgaacattcataataaaactgccatccccatcaatatcgacaaccactgcatctggtcgag

SEQ ID NO: 99 - DNA, 126 bp, synthetic construct
  misc_feature 1..126: note = InDel3
  source 1..126: mol_type = other DNA
ggacaaccatacctaaatgttgattgtttagcagcattatttccaccctaattgtagccaactcttgaacattcataataaaactgccatccccatcaatatcgacaaccactgcatctggtcgag

SEQ ID NO: 100 - DNA, 103 bp, synthetic construct
  misc_feature 1..103: note = InDel4
  source 1..103: mol_type = other DNA
ggacaaccatacctaaatgttgattgtttagcagcattatcttgaacattcataataaaactgccatccccatcaatatcgacaaccactgcatctggtcgag

SEQ ID NO: 101 - DNA, 83 bp, synthetic construct
  misc_feature 1..83: note = InDel5
  source 1..83: mol_type = other DNA
ggacaaccatacctaaatgttgattgtttagcagcattatctgccatccccatcaatatcgacaaccactgcatctggtcgag

SEQ ID NO: 102 - DNA, 76 bp, synthetic construct
  misc_feature 1..76: note = InDel6
  source 1..76: mol_type = other DNA
ggacaaccatacctaaatgttgattgtttagcagcattatccccatcaatatcgacaaccactgcatctggtcgag

SEQ ID NO: 103 - DNA, 64 bp, synthetic construct
  misc_feature 1..64: note = InDel7
  source 1..64: mol_type = other DNA
ggacaaccatacctaaatgttgattgtttagcagcattatcgacaaccactgcatctggtcgag

SEQ ID NO: 104 - DNA, 59 bp, Zea mays
  source 1..59: mol_type = genomic DNA
tttaatttactgtcacgattcccctctcctggtcgaacttttcaggtggggaaagctgc

SEQ ID NO: 105 - DNA, 53 bp, synthetic construct
  misc_feature 1..53: note = InDel at crGEP5 target locus
  source 1..53: mol_type = other DNA
tttgatttactgtcacgattccctggtcgaacttttcaggtggggaaagctgc

SEQ ID NO: 106 - DNA, 58 bp, synthetic construct
  misc_feature 1..58: note = InDel at crGEP5 target locus
  source 1..58: mol_type = other DNA
tttgatttactgtcacgattcccctctcctgtcgaacttttcaggtggggaaagctgc

SEQ ID NO: 107-108 - skipped (2 entries)

SEQ ID NO: 109 - DNA, 39 bp, synthetic construct
  misc_feature 1..39: note = InDel at crGEP5 target locus
  source 1..39: mol_type = other DNA
tttgatttactgtctaacttttcaggtggggaaagctgc

SEQ ID NO: 110 - DNA, 58 bp, synthetic construct
  misc_feature 1..58: note = InDel at crGEP5 target locus
  source 1..58: mol_type = other DNA
tttgatttactgtcatgattcccctccctggtcgaacttttcaggtggggaaagctgc

SEQ ID NO: 111 - DNA, 60 bp, Zea mays
  source 1..60: mol_type = genomic DNA
ctgtggcactaccaagctcctgctcaccattccaagaatccttgagcttgctgaagagct

SEQ ID NO: 112 - DNA, 54 bp, synthetic construct
  misc_feature 1..54: note = InDel at crGEP75 target locus
  source 1..54: mol_type = other DNA
ctgtggcactaccaagctcctgctcaccagaatccttgagcttgctgaagagct

SEQ ID NO: 113 - DNA, 56 bp, synthetic construct
  misc_feature 1..56: note = InDel at crGEP75 target locus
  source 1..56: mol_type = other DNA
ctgtggcactaccaagctcctgctcaccttggaatccttgagcttgctgaagagct

SEQ ID NO: 114 - DNA, 51 bp, synthetic construct
  misc_feature 1..51: note = InDel at crGEP75 target locus
  source 1..51: mol_type = other DNA
ctgtggcactaccaagctcctgctcagaatccttgagcttgctgaagagct

SEQ ID NO: 115 - DNA, 36 bp, synthetic construct
  misc_feature 1..36: note = InDel at crGEP75 target locus
  source 1..36: mol_type = other DNA
ctgtggcactaccaagctcctgcttgctgaagagct

SEQ ID NO: 116 - DNA, 53 bp, synthetic construct
  misc_feature 1..53: note = InDel at crGEP75 target locus
  source 1..53: mol_type = other DNA
ctgtggcactaccaagctcctgctcaatgaatccttgagcttgctgaagagct

SEQ ID NO: 117 - DNA, 57 bp, Zea mays
  source 1..57: mol_type = genomic DNA
gcaggagctgcctggaggcgggctcctcgtgtaccagagcttctgtgctgaagacgc

SEQ ID NO: 118 - DNA, 49 bp, synthetic construct
  misc_feature 1..49: note = InDel at crGEP77 target locus
  source 1..49: mol_type = other DNA
gcaggagctgcctggaggcgggctcctcgagcttctgtgctgaagacgc

SEQ ID NO: 119 - DNA, 39 bp, synthetic construct
  misc_feature 1..39: note = InDel at crGEP77 target locus
  source 1..39: mol_type = other DNA
gcaggagctgcctggaggcgggctctgtgctgaagacgc

SEQ ID NO: 120 - DNA, 51 bp, synthetic construct
  misc_feature 1..51: note = InDel at crGEP77 target locus
  source 1..51: mol_type = other DNA
gcaggagctgcctggaggcgggctcctcgtgagcttctgtgctgaagacgc

SEQ ID NO: 121 - DNA, 48 bp, synthetic construct
  misc_feature 1..48: note = InDel at crGEP77 target locus
  source 1..48: mol_type = other DNA
gcaggagctgcctggaggcgggctcctgagcttctgtgctgaagacgc

SEQ ID NO: 122 - DNA, 51 bp, synthetic construct
  misc_feature 1..51: note = InDel at crGEP77 target locus
  source 1..51: mol_type = other DNA
gcaggagctgcctggaggcgggctcctcgggagcttctgtgctgaagacgc

SEQ ID NO: 123 - DNA, 48 bp, synthetic construct
  misc_feature 1..48: note = InDel at crGEP77 target locus
  source 1..48: mol_type = other DNA
gcaggagctgcctggaggcgggctcctcagcttctgtgctgaagacgc

SEQ ID NO: 124 - DNA, 50 bp, synthetic construct
  misc_feature 1..50: note = InDel at crGEP77 target locus
  source 1..50: mol_type = other DNA
gcaggagctgcctggaggcgggctcctcgtagcttctgtgctgaagacgc

SEQ ID NO: 125 - DNA, 60 bp, Triticum aestivum
  source 1..60: mol_type = genomic DNA
gctcttcccgcaccgcttcagccctgcagcacgcacccatccatgacgcaacacacatca

SEQ ID NO: 126 - DNA, 57 bp, synthetic construct
  misc_feature 1..57: note = InDel in A genome
  source 1..57: mol_type = other DNA
gctcttcccgcaccgcttcagccctgcacgcacccatccatgacgcaacacacatca

SEQ ID NO: 127 - DNA, 53 bp, synthetic construct
  misc_feature 1..53: note = InDel in A genome
  source 1..53: mol_type = other DNA
gctcttcccgcaccgcttcagccccgcacccatccatgacgcaacacacatca

SEQ ID NO: 128 - DNA, 55 bp, synthetic construct
  misc_feature 1..55: note = InDel in A genome
  source 1..55: mol_type = other DNA
gctcttcccgcaccgcttcagccctacgcacccatccatgacgcaacacacatca

SEQ ID NO: 129 - DNA, 56 bp, synthetic construct
  misc_feature 1..56: note = InDel in A genome
  source 1..56: mol_type = other DNA
gctcttcccgcaccgcttcagcctgcacgcacccatccatgacgcaacacacatca

SEQ ID NO: 130 - DNA, 54 bp, synthetic construct
  misc_feature 1..54: note = InDel in A genome
  source 1..54: mol_type = other DNA
gctcttcccgcaccgcttcagccctggcacccatccatgacgcaacacacatca

SEQ ID NO: 131 - DNA, 46 bp, synthetic construct
  misc_feature 1..46: note = InDel in A genome
  source 1..46: mol_type = other DNA
gctcttcccgcaccgcttcagcccatccatgacgcaacacacatca

SEQ ID NO: 132 - DNA, 48 bp, synthetic construct
  misc_feature 1..48: note = InDel in A genome
  source 1..48: mol_type = other DNA
gctcttcccgcaccgcttcagcccccatccatgacgcaacacacatca

SEQ ID NO: 133 - DNA, 48 bp, synthetic construct
  misc_feature 1..48: note = InDel in A genome
  source 1..48: mol_type = other DNA
gctcttcccgcaccgcttcagcacccatccatgacgcaacacacatca

SEQ ID NO: 134 - DNA, 60 bp, Triticum aestivum; identical to SEQ ID NO: 125
  source 1..60: mol_type = genomic DNA

SEQ ID NO: 135 - DNA, 50 bp, synthetic construct
  misc_feature 1..50: note = InDel in B genome
  source 1..50: mol_type = other DNA
gctcttcccgcaccgcttcagcccacccatccatgacgcaacacacatca

SEQ ID NO: 136 - DNA, 54 bp, synthetic construct
  misc_feature 1..54: note = InDel in B genome
  source 1..54: mol_type = other DNA
gctcttcccgcaccgcttcagcccacgcacccatccatgacgcaacacacatca

SEQ ID NO: 137 - DNA, 53 bp, synthetic construct
  misc_feature 1..53: note = InDel in B genome
  source 1..53: mol_type = other DNA
gctcttcccgcaccgcttcagccacgcacccatccatgacgcaacacacatca

SEQ ID NO: 138 - DNA, 51 bp, synthetic construct
  misc_feature 1..51: note = InDel in B genome
  source 1..51: mol_type = other DNA
gctcttcccgcaccgcttcagccgcacccatccatgacgcaacacacatca

SEQ ID NO: 139 - DNA, 50 bp, synthetic construct
  misc_feature 1..50: note = InDel in B genome
  source 1..50: mol_type = other DNA
gctcttcccgcaccgcttcagcgcacccatccatgacgcaacacacatca

SEQ ID NO: 140 - DNA, 60 bp, synthetic construct
  misc_feature 1..60: note = InDel in B genome
  source 1..60: mol_type = other DNA
catccatgacgcaccacacatcagcccagcacgcacccatccatgacgcaacacacatca

SEQ ID NO: 141 - DNA, 60 bp, Triticum aestivum; identical to SEQ ID NO: 125
  source 1..60: mol_type = genomic DNA

SEQ ID NO: 142 - DNA, 53 bp, synthetic construct; identical to SEQ ID NO: 127
  misc_feature 1..53: note = InDel in D genome
  source 1..53: mol_type = other DNA

SEQ ID NO: 143 - DNA, 47 bp, synthetic construct
  misc_feature 1..47: note = InDel in D genome
  source 1..47: mol_type = other DNA
gctcttcccgcaccgcttcagccccatccatgacgcaacacacatca

SEQ ID NO: 144 - DNA, 51 bp, synthetic construct
  misc_feature 1..51: note = InDel in D genome
  source 1..51: mol_type = other DNA
gctcttcccgcaccgcttcagccctacccatccatgacgcaacacacatca

SEQ ID NO: 145 - DNA, 96 bp, synthetic construct
  misc_feature 1..96: note = expression cassette
  source 1..96: mol_type = other DNA
aattcgatctacacttagtagaaattaatctcccagtagaaattaatctcccagttaagataatgctgcatctacacttagtagaaattatcaggt

SEQ ID NO: 146 - DNA, 24 bp, synthetic construct
  misc_feature 1..24: note = protospacer
  source 1..24: mol_type = other DNA
caccctaattgtagccaactcttg

SEQ ID NO: 147 - DNA, 24 bp, synthetic construct
  misc_feature 1..24: note = protospacer
  source 1..24: mol_type = other DNA
gcagcattatcttaactgggagat

SEQ ID NO: 148 - DNA, 24 bp, synthetic construct
  misc_feature 1..24: note = protospacer
  source 1..24: mol_type = other DNA
ggtatggttgtccaatgggaagat

SEQ ID NO: 149 - DNA, 24 bp, synthetic construct
  misc_feature 1..24: note = protospacer
  source 1..24: mol_type = other DNA
caaggtatgtatgtgcccggttag

SEQ ID NO: 150 - DNA, 24 bp, synthetic construct
  misc_feature 1..24: note = protospacer
  source 1..24: mol_type = other DNA
gaagggtttccaaggtatgtatgt

SEQ ID NO: 151 - DNA, 187 bp, synthetic construct
  misc_feature 1..187: note = expression cassettte
  source 1..187: mol_type = other DNA
cgatcgcctctctgcttggctcctctttcttgtgaaagagggttcccaggcgacaccacgaggaggtgcagagtaggactgacgcccaagagttggctacaattagggtgatctacacttagtagaaattagacgagcttactcgtttcgtcctcacggactcatcagtaatttggatcccctctcc

SEQ ID NO: 152 - protein, 1252 aa, Lachnospiraceae bacterium
MAPKKKRKVSKLEKFTNCYSLSKTLRFKAIPVGKTQENIDNKRLLVEDEKRAEDYKGVKKLLDRYYLSFINDVLHSIKLKNLNNYISLFRKKTRTEKENKELENLEINLRKEIAKAFKGNEGYKSLFKKDIIETILPEFLDDKDEIALVNSFNGFTTAFTGFFDNRENMFSEEAKSTSIAFRCINENLTRYISNMDIFEKVDAIFDKHEVQEIKEKILNSDYDVEDFFEGEFFNFVLTQEGIDVYNAIIGGFVTESGEKIKGLNEYINLYNQKTKQKLPKFKPLYKQVLSDRESLSFYGEGYTSDEEVLEVFRNTLNKNSEIFSSIKKLEKLFKNFDEYSSAGIFVKNGPAISTISKDIFGEWNVIRDKWNAEYDDIHLKKKAVVTEKYEDDRRKSFKKIGSFSLEQLQEYADADLSVVEKLKEIIIQKVDEIYKVYGSSEKLFDADFVLEKSLKKNDAVVAIMKDLLDSVKSFENYIKAFFGEGKETNRDESFYGDFVLAYDILLKVDHIYDAIRNYVTQKPYSKDKFKLYFQNPQFMGGWDKDKETDYRATILRYGSKYYLAIMDKKYAKCLQKIDKDDVNGNYEKINYKLLPGPNKMLPKVFFSKKWMAYYNPSEDIQKIYKNGTFKKGDMFNLNDCHKLIDFFKDSISRYPKWSNAYDFNFSETEKYKDIAGFYREVEEQGYKVSFESASKKEVDKLVEEGKLYMFQIYNKDFSDKSHGTPNLHTMYFKLLFDENNHGQIRLSGGAELFMRRASLKKEELVVHPANSPIANKNPDNPKKTTTLSYDVYKDKRFSEDQYELHIPIAINKCPKNIFKINTEVRVLLKHDDNPYVIGIDRGERNLLYIVVVDGKGNIVEQYSLNEIINNFNGIRIKTDYHSLLDKKEKERFEARQNWTSIENIKELKAGYISQVVHKICELVEKYDAVIALEDLNSGFKNSRVKVEKQVYQKFEKMLIDKLNYMVDKKSNPCATGGALKGYQITNKFESFKSMSTQNGFIFYIPAWLTSKIDPSTGFVNLLKTKYTSIADSKKFISSFDRIMYVPEEDLFEFALDYKNFSRTDADYIKKWKLYSYGNRIRIFRNPKKNNVFDWEEVCLTSAYKELFNKYGINYQQGDIRALLCEQSDKAFYSSFMALMSLMLQMRNSITGRTDVDFLISPVKNSDGIFYDSRNYEAQENAILPKNADANGAYNIARKVLWAIGQFKKAEDEKLDKVKIAISNKEWLEYAQTSVKHKRPAATKKAGQAKKKK

SEQ ID NO: 153 - protein, 1252 aa, Lachnospiraceae bacterium; identical to SEQ ID NO: 152

SEQ ID NO: 154 - protein, 1260 aa, Lachnospiraceae bacterium
MAPKKKRKVGIHGVPAASKLEKFTNCYSLSKTLRFKAIPVGKTQENIDNKRLLVEDEKRAEDYKGVKKLLDRYYLSFINDVLHSIKLKNLNNYISLFRKKTRTEKENKELENLEINLRKEIAKAFKGNEGYKSLFKKDIIETILPEFLDDKDEIALVNSFNGFTTAFTGFFDNRENMFSEEAKSTSIAFRCINENLTRYISNMDIFEKVDAIFDKHEVQEIKEKILNSDYDVEDFFEGEFFNFVLTQEGIDVYNAIIGGFVTESGEKIKGLNEYINLYNQKTKQKLPKFKPLYKQVLSDRESLSFYGEGYTSDEEVLEVFRNTLNKNSEIFSSIKKLEKLFKNFDEYSSAGIFVKNGPAISTISKDIFGEWNVIRDKWNAEYDDIHLKKKAVVTEKYEDDRRKSFKKIGSFSLEQLQEYADADLSVVEKLKEIIIQKVDEIYKVYGSSEKLFDADFVLEKSLKKNDAVVAIMKDLLDSVKSFENYIKAFFGEGKETNRDESFYGDFVLAYDILLKVDHIYDAIRNYVTQKPYSKDKFKLYFQNPQFMGGWDKDKETDYRATILRYGSKYYLAIMDKKYAKCLQKIDKDDVNGNYEKINYKLLPGPNKMLPKVFFSKKWMAYYNPSEDIQKIYKNGTFKKGDMFNLNDCHKLIDFFKDSISRYPKWSNAYDFNFSETEKYKDIAGFYREVEEQGYKVSFESASKKEVDKLVEEGKLYMFQIYNKDFSDKSHGTPNLHTMYFKLLFDENNHGQIRLSGGAELFMRRASLKKEELVVHPANSPIANKNPDNPKKTTTLSYDVYKDKRFSEDQYELHIPIAINKCPKNIFKINTEVRVLLKHDDNPYVIGIDRGERNLLYIVVVDGKGNIVEQYSLNEIINNFNGIRIKTDYHSLLDKKEKERFEARQNWTSIENIKELKAGYISQVVHKICELVEKYDAVIALEDLNSGFKNSRVKVEKQVYQKFEKMLIDKLNYMVDKKSNPCATGGALKGYQITNKFESFKSMSTQNGFIFYIPAWLTSKIDPSTGFVNLLKTKYTSIADSKKFISSFDRIMYVPEEDLFEFALDYKNFSRTDADYIKKWKLYSYGNRIRIFRNPKKNNVFDWEEVCLTSAYKELFNKYGINYQQGDIRALLCEQSDKAFYSSFMALMSLMLQMRNSITGRTDVDFLISPVKNSDGIFYDSRNYEAQENAILPKNADANGAYNIARKVLWAIGQFKKAEDEKLDKVKIAISNKEWLEYAQTSVKHKRPAATKKAGQAKKKK

SEQ ID NO: 155 - protein, 1252 aa, Lachnospiraceae bacterium; identical to SEQ ID NO: 152

SEQ ID NO: 156 - protein, 1252 aa, Lachnospiraceae bacterium; identical to SEQ ID NO: 152

SEQ ID NO: 157 - DNA, 3948 bp, synthetic construct
  misc_feature 1..3948: note = variant I of Cpf1 (SEQ ID NO: 72) including an intronic sequence
  misc_feature 862..1050: note = intron
  source 1..3948: mol_type = other DNA
atggcgccgaagaagaagcgcaaggtgtccaagctcgagaagttcacgaactgctactccctctccaagaccctccgcttcaaggccatccccgtgggcaagacccaggagaacatcgacaacaagcgcctcctggtcgaggacgagaagagggcggaggactacaagggcgtgaagaagctcctggaccgctactacctctccttcatcaacgacgtcctgcacagcatcaagctcaagaacctgaacaactacatctccctgttccgcaagaagacgaggaccgagaaggagaacaaggagctcgagaacctggagatcaacctccgcaaggagatcgccaaggcgttcaagggcaacgagggctacaagagcctgttcaagaaggacatcatcgagacgatcctcccggagttcctggacgacaaggacgagatcgccctcgtgaactccttcaacggcttcaccacggcgttcaccggcttcttcgacaaccgcgagaacatgttcagcgaggaggccaagtccacgagcatcgcgttccgctgcatcaacgagaacctgaccaggtacatctccaacatggacatcttcgagaaggtcgacgccatcttcgacaagcacgaggtgcaggagatcaaggagaagatcctcaacagcgactacgacgtcgaggacttcttcgagggcgagttcttcaacttcgtcctgacgcaggagggcatcgacgtgtacaacgccatcatcggtggcttcgtgaccgagtccggcgagaagatcaagggcctcaacgagtacatcaacctgtacaaccagaagaccaagcagaagctcccgaagttcaagcccctctacaagcaggtaagtttctgcttctacctttgatatatatataataattatcattaattagtagtaatataatatttcaaatatttttttcaaaataaaagaatgtagtatatagcaattgcttttctgtagtttataagtgtgtatattttaatttataacttttctaatatatgaccaaaacatggtgatgtgcaggtcctgtccgaccgcgagtccctgagcttctacggcgagggctacacgagcgacgaggaggtcctcgaggtgttcaggaacaccctgaacaagaacagcgagatcttctccagcatcaagaagctcgagaagctgttcaagaacttcgacgagtactccagcgccggcatcttcgtcaagaacggcccggcgatctccacgatcagcaaggatatcttcggcgagtggaacgtgatcagggacaagtggaacgccgagtacgacgacatccacctcaagaagaaggcggtggtcaccgagaagtacgaggacgaccgcaggaagtccttcaagaagatcggctccttcagcctcgagcagctgcaggagtacgccgacgcggacctctccgtggtcgagaagctgaaggagatcatcatccagaaggtcgacgagatctacaaggtgtacggctccagcgagaagctgttcgacgccgacttcgtcctcgagaagtccctgaagaagaacgacgccgtggtcgcgatcatgaaggacctcctggactccgtgaagagcttcgagaactacatcaaggcgttcttcggcgagggcaaggagacgaaccgcgacgagtccttctacggcgacttcgtcctcgcctacgacatcctcctgaaggtggaccacatctacgacgcgatcaggaactacgtgacccagaagccgtacagcaaggacaagttcaagctgtacttccagaacccccagttcatgggcggctgggacaaggacaaggagacggactaccgcgccaccatcctccgctacggcagcaagtactacctggccatcatggacaagaagtacgcgaagtgcctccagaagatcgacaaggacgacgtcaacggcaactacgagaagatcaactacaagctcctgccgggccccaacaagatgctgccgaaggtgttcttctccaagaagtggatggcctactacaaccccagcgaggacatccagaagatctacaagaacggcacgttcaagaagggcgacatgttcaacctcaacgactgccacaagctgatcgacttcttcaaggactccatcagccgctacccgaagtggtccaacgcctacgacttcaacttcagcgagacagagaagtacaaggacatcgcgggcttctacagggaggtcgaggagcagggctacaaggtgtccttcgagtccgccagcaagaaggaggtcgacaagctcgtggaggagggcaagctgtacatgttccagatctacaacaaggacttctccgacaagagccacggcacgcccaacctccacaccatgtacttcaagctcctgttcgacgagaacaaccacggccagatccgcctctccggcggcgccgagctgttcatgaggagggcgagcctcaagaaggaggagctggtggtccaccccgctaacagcccaatcgcgaacaagaacccggacaaccccaagaagaccacgaccctctcctacgacgtgtacaaggacaagcgcttcagcgaggaccagtacgagctgcacatcccgatcgccatcaacaagtgccccaagaacatcttcaagatcaacaccgaggtcagggtgctcctgaagcacgacgacaacccctacgtgatcggcatcgaccgcggcgagaggaacctcctgtacatcgtggtcgtggacggcaagggcaacatcgtggagcagtactccctgaacgagatcatcaacaacttcaacggcatccgcatcaagacggactaccacagcctcctggacaagaaggagaaggagcgcttcgaggccaggcagaactggacctccatcgagaacatcaaggagctcaaggcgggctacatcagccaggtcgtgcacaagatctgcgagctggtcgagaagtacgacgccgtgatcgcgctcgaggacctgaactccggcttcaagaacagcagggtcaaggtggagaagcaggtctaccagaagttcgagaagatgctcatcgacaagctgaactacatggtggacaagaagtccaacccgtgcgctacgggcggcgcgctcaagggctaccagatcaccaacaagttcgagagcttcaagtccatgagcacccagaacggcttcatcttctacatcccggcctggctgacgtccaagatcgaccccagcaccggcttcgtcaacctcctgaagacgaagtacacctccatcgcggacagcaagaagttcatctccagcttcgaccgcatcatgtatgtgccggaggaggacctcttcgagttcgccctggactacaagaacttctccaggacggacgcggattacatcaagaagtggaagctctacagctacggcaaccgcatcaggatcttccgcaaccccaagaagaacaacgtcttcgactgggaggaggtgtgcctcacctccgcctacaaggagctgttcaacaagtacggcatcaactaccagcagggcgacatcagggcgctcctgtgcgagcagagcgacaaggccttctactccagcttcatggcgctcatgtccctcatgctgcagatgcgcaacagcatcacgggcaggaccgacgtcgacttcctgatctccccggtgaagaacagcgacggcatcttctacgacagccgcaactacgaggcccaggagaacgcgatcctgccaaagaacgcggacgccaacggcgcctacaacatcgcgaggaaggtgctgtgggccatcggccagttcaagaaggcggaggacgagaagctcgacaaggtcaagatcgccatctccaacaaggagtggctggagtacgcgcagacctcggtgaagcacaagaggcccgctgccaccaagaaggcgggccaggccaagaagaagaagtga

SEQ ID NO: 158 - DNA, 3948 bp, synthetic construct
  misc_feature 1..3948: note = variant III of Cpf1 (SEQ ID NO: 75) including an intronic sequence
  misc_feature 628..816: note = intron
  source 1..3948: mol_type = other DNA
atggccccgaagaagaagaggaaggtcagcaagctcgagaagttcaccaactgctacagcctgagcaagaccctgaggttcaaggctatcccggtgggcaagacccaagagaacatcgacaacaagaggctgctggtcgaggacgagaagcgcgctgaggattacaagggcgtgaagaagctgctggacaggtactacctgagcttcatcaacgacgtgctgcacagcatcaagctgaagaacctgaacaactacatcagcctgttccgcaagaaaaccaggaccgagaaagagaacaaagagcttgagaacctcgagatcaacctgaggaaagagatcgccaaggccttcaagggcaacgagggctacaagagcctgttcaagaaggacatcatcgagactatcctgccagagttcctggacgacaaggacgagatcgccctggtgaacagcttcaacggcttcacgaccgccttcaccggtttcttcgacaaccgcgagaatatgttcagcgaggaagccaagagcacctctatcgccttccgctgcatcaacgagaacctgacgcgctacatctccaacatggatatcttcgagaaggtggacgccatcttcgataagcacgaggtaagtttctgcttctacctttgatatatatataataattatcattaattagtagtaatataatatttcaaatatttttttcaaaataaaagaatgtagtatatagcaattgcttttctgtagtttataagtgtgtatattttaatttataacttttctaatatatgaccaaaacatggtgatgtgcaggtgcaagagatcaaagaaaagatcctgaacagcgactacgacgtcgaggacttcttcgagggcgagttcttcaacttcgtgctcacccaagagggcatcgatgtgtacaacgccatcatcggcggcttcgtgactgagagcggcgagaagatcaagggcctgaacgagtacatcaacctctacaatcaaaagaccaagcagaagctgccgaagttcaagccgctgtacaagcaggttctgagcgaccgcgagagcctgtctttctacggcgagggttacaccagcgacgaagaggtgttggaggttttccgcaacaccctgaacaagaacagcgagatcttcagctccatcaagaagctggaaaagctgtttaagaacttcgacgagtacagcagcgccggcatcttcgtgaagaacggcccagctatcagcaccatcagcaaggacatcttcggcgagtggaacgtgatcagggacaagtggaacgccgagtacgacgacatccacctgaagaaaaaggccgtggtgaccgagaagtacgaggacgacaggcgcaagagcttcaagaagatcggctccttcagcctcgagcagctgcaagagtacgctgacgctgacctgagcgtggtcgagaagctcaaagagatcatcatccagaaggtcgacgagatctacaaggtgtacggcagcagcgagaagcttttcgacgccgacttcgtccttgagaagtccctcaagaaaaacgacgccgtggtggccatcatgaaggacctgctggactccgtgaagtccttcgagaactacattaaggctttcttcggtgagggcaaagagactaacagggacgagagcttctacggggatttcgtgctggcctacgacatcctgctcaaggtggaccacatctacgacgccatccgcaactacgtgacccagaagccgtactccaaggacaagtttaagctgtacttccagaatccgcagttcatgggcggctgggacaaagacaaagaaaccgactacagggccaccatcctgaggtacggctccaagtactacctcgccatcatggacaagaaatacgccaagtgcctgcagaagatcgataaggacgacgtgaacggcaactacgagaagattaactacaagctgctgccagggccgaacaagatgctcccgaaggtgttctttagcaagaaatggatggcctactacaacccgagcgaggatatccagaaaatctacaagaacggcaccttcaagaaaggcgacatgttcaacctgaacgactgccacaagctgatcgatttcttcaaggacagcatctctcgctacccgaagtggtccaacgcctacgatttcaacttcagcgagactgaaaagtacaaggatatcgccggcttctaccgcgaggtcgaggaacagggttacaaggtgagcttcgagagcgccagcaagaaagaggtggacaagctggtcgaagagggcaagctgtacatgttccagatctataacaaggacttctccgacaagagccacggcaccccaaacctgcacaccatgtacttcaagttgctgttcgacgagaacaaccacggccagatcaggctttctggcggcgctgagcttttcatgagaagggccagcctgaaaaaagaggaactggtcgttcacccggcgaacagcccaatcgccaacaagaacccggacaacccgaaaaagaccaccacgctgagctacgacgtgtacaaggacaaaaggttctccgaggaccagtacgagctgcacatcccgatcgccatcaacaagtgcccgaagaacatcttcaagatcaacaccgaggtgagggtgctgctgaagcacgacgacaacccatacgtgatcggcatcgataggggcgagcgcaacctgctctacatcgtggtggttgacggcaagggcaatatcgtcgagcagtacagccttaacgagatcattaacaacttcaatggcatcaggatcaagaccgactaccacagcctgctcgacaagaaagaaaaagagcgcttcgaggccaggcagaactggaccagcatcgagaatatcaaagagctgaaggccggctacattagccaggtggtgcacaagatctgcgagctggtggaaaagtacgacgcggtgatcgctctcgaggacctgaactccgggttcaagaactcccgcgtgaaggttgagaagcaggtctaccaaaagttcgagaagatgctgatcgacaagctcaactacatggtggacaaaaagagcaacccctgcgccacaggcggcgctcttaagggctaccagatcacgaacaagttcgagtccttcaagagcatgagcacccagaatggcttcatcttctacatcccggcctggctgaccagcaagatcgatccatctaccggcttcgtcaacctcctcaagaccaagtacaccagcattgccgacagcaagaagttcatctccagcttcgacaggatcatgtacgtgccggaagaggacctgttcgagttcgcgctcgattacaagaacttcagcaggaccgacgcggactatattaagaagtggaagctctacagctacggcaacaggatccgcatcttcagaaacccgaagaaaaacaacgtgttcgactgggaagaagtgtgcctgaccagcgcctacaaagaactgttcaacaagtacggcatcaactaccagcagggcgacatcagggctctgctgtgcgagcagtctgacaaggcgttctacagctccttcatggccctgatgagcctgatgctgcagatgaggaacagcatcaccggcaggacggacgtcgacttcctgatcagcccagtgaagaattccgacggcattttctacgactctaggaactacgaggctcaagagaacgccatcctgccgaagaacgccgatgctaacggcgcgtacaacattgcccgcaaggtgctgtgggctatcggccagtttaagaaggccgaggacgaaaaactggacaaggtgaagatcgccattagcaacaaagagtggctcgagtacgcccagaccagcgtgaagcacaaaaggccagccgccactaagaaggctggccaggccaaaaagaagaagtga